European Patent Application EP 4 796 178 A2, published August 26, 2026. Title: SELECTIVE REDUCTION OF ALLELIC VARIANTS. Applicant: Ionis Pharmaceuticals, Inc. The sequence listing filed with the application follows.

SEQUENCE LISTING (288 sequences)

SEQ ID NO: 1 - DNA, 202001 bp, Homo sapiens
  source 1..202001: mol_type = genomic DNA
gcccagcaggtgtcagcctcattttaccccgcccctattcaagatgaagttgttctggttccaacgcctctgacatattagctgcatcattttacatttcttttttttttttccttttaaatggggtcttgctctgtcacccaggctggagtgctgtggtatgatctcggctcactgcaatctccacctccgaggttccagcgattctcttgcctcagcctcccgagtagctgggactacaggcacccaccatcatactgggctaatttttgtgtttttagtagagatggggtttccccatgttgcccaggctgatctcaaactcctgggcttaagcaatacagccgcgttggcctcccaaagtgttgggattacaagcatgagctaccccacccagctcattttacatttccacttgttaaactgaaaactggcccgagaaagcttctgtactgccatccttgcgtccttgcagatgaatcgtaacctagcatagtaggtaggcagactgaaaacctaacttagcagtaggcttctgtaacaacagctgtgtctcagccagttcctgcagccagacttcaaccactcacaggccgcaaactgttcaaactgtgttcggagaaggcgaattcatctggctgttaacgtgcctcacttctgctttctgtggccactttcccttttctgtccataaatttgctttgaccacacagcatccctagagtctccctgaatctgctgtgattctgggacctgcaccatttgtgaattgttttttttttccttgatcagctaaactctgttcaattcaatttgttggaagtttttaacataccaatggtgcaccaaggttccaatttctccacttcctcataaataagtcattttaaatggcttttcagtattccaatatttggaagtattaatgtttctaccaattttctatttttggacattgaggttgtttcattttttttttctttttttgagacagagtctcgctccgtcacccaggctggagtgcagtggcctgatcccggcccactgcaacctccacctccctcctcagcctcctgagtagctgggattacaggtgcatgcaccaccacacccagctaatttttgtatttttagtagagatggggtttcaccatgttggtcaggctggtctcaaactcctgacctcaggtggtccacctgccttggcctcccaaaatgctgggattacaggcctgagccactgcgcctggcctcatcttcttgatattaatgttgctttaacatctttgtccctgtgttttttgtttttttttttgagacggagtctcattcattctgtcacccaggctggagttcagtggcgtgatctcagctcactgcaacctctgtctcctgggttccagtgattctcctgcgtcggtctcctgagtagctgtgttcctgggtctttcgatggttatttaatacttccctacagtaatgccctgtgcgtacatgctaagtgtgatgaaatggttggcacagttaaatcttttgaaagacattgccaagtcactcttcagaaaagtgataggaggtcatagcaattttaagaagtcctcatttctacatttccttactaatctcggttggtgtctcttcaatctttcctcacacttttcttgggtttttcctgaatcatgagtctactacatttacacattttaaagcatctttagaaacaggatctcattttgttgcccaggctagagtttggtggcatgattatagctcctcatactcctgggctcaagtgatccttccacctctgaaaccccaaaatttgagaaaggtctcatttaatttagaaagtttattttgccaaggttgagggtgcacacctgtgatgatatacgagttaaaaagaaattatttaggcagatactgagggtaagaaagtcctcggtaaggttttcttttcaatgaaaagcagcccccaagcattttcttttctaacaaagagcagcctgtaaaatcgagctgcagacatacacaagcaagctggaagcttgcacaggtgaatgctggcagctgtgccaataagaaaaggctacctggggccaggcagatccaacatggcggctccatcttccctttccttgtcaaccatgtgcacagtaaggagcaggcaacatagtgtcccccgagtagagaccaatttgcataataaaaggtgagggtagggtgggcagcttctttgcatgctatgtaaacattatgcctggtccaaccaatctttgggccctgtgtaaattagacaccacctcctcaagcctgtctataaaaccctgtccattctgccgcaggctggaagacccactggggcacccctctctctctataggagacagctattcatttttctctttctttcacctattaaagctccactcttaaccccactccgtgtgtatctatgttcttgatttccttggcatgaggcaatgaaccttgggtattaccccagaaccttgggtattatgccacttcagtgacacagcctcaggaaatcctgatgacatgttcccaagatggtcggggcacagcttggttttatacattttagggagacatgagacgtcaattcatatatgtaagaagtacattggttccgtccagaaaggcggggacaacttgaggcagggagagagcttctaggtcacaggtagacaaatggttgcattcttttgaatctccgataagcctttccaaaggaggcaatcagaatatgcgtctattgactgggcgcagtggctcatgcctgtaatgccagcactttgggaggcggaggtgggtggatcacctgaggtcaggagtttgagagcagcccggccaacatggtgaaaccctgtctctactaaaaatacaaaaaattagctgggcgtggtggcgggcgcctgtaatcccagctactcgggaggctgaggcaggagaatagcttgaacccagaaggaagaggttgcagtgagctgagatggtgccattgcactccagcctgggcaacaagagtgaaactccatctcagaaaaaaaaaaaaaaggcctgggcaaagtggctcacgcctgtaatcccagcactttgggaagccgaggcgggcaggtcacaaagtcaggagattgagaccatcctggctaacatgatgaaaccccatctctactaaaaaatacaaaaaactagctgggtgtggtggcgagcacctgtagtcccagctactcggcaggctgaggcaggagaatggcgtgaaccggggaggcggagcttgcagtgagccgagatcacaccactgcactccagcccggacgacagggcaagactctatctcaaattaaaaaaaaaaaaaaaaaaaaaaaaaaagagagagagaatatgcatctatctcagtgagcagaaggatgactttgaatggaatgggagcagttcctagcttgaacttcccctttagcttcagtgatttgggggctcaaggtatgttcctttcacatacctcagcctcccaagtagctgggaccacaagtgcatgccaccacacgtggctaatgttttattttttttgtaggaatagggtctcactatgtgtccaggctggtctaaaacccctgagctcaaatggtcctcccgcctcagcctcccgaaatgctgggattacaggcatgagccagcatgcccggcctagtctacatttttataaattgctaattcaaagttccctctccaaaacctcatggttttccctgttctcatcccctgcaccctcccttcccctggagtactcacctggccttggaggtctggtgtgagcccggacttcgattctaggcacagcatgtgatgagcgcccccaggtcaaacacctcccctctgcggcctgtgcttcaccgccttgacagtgagaaaggtctcccttcggctcattctcgaagtctcaaacttcacttctcctgtgcgctgattctgaattcagcccccgtccaaggtcctggcccctttctcttctgcttggcgtgttgttcatcaccactgtgcactgctgagggtaagtgcggttctctggacctctgctttatcattagaacagactcttgcggtttcccacgacattcctttcacttctcacttggaagatgagccgtgaggaaatcctgtgttgtgtggtatgtgggctgtgcttctgcttgacttgagggccaagcagcattgcaagccatggttttaaataagaaagaacatttctaaccttcatcttctagtaaggaaacaagtgggctttagagttcttgctcaggaaagacctatgtcccagtccaaccggaccttttactaaagagatcttcctgatcctcctccccaggccaggggaggggtcctccctggggttggagcctttagtagggggtcggagacacgacgtagccttcatgacattcatagtctagttacacgatccctgtaagggtcagttgaagtaagtgctacaaaggaagggaggtgctcagtggagagggctctcttttatgtattatatttctttcatggggagggatatggatcagggatcagcagaggtgtttcagtcccgagggaaagaaagtcagcgtggcttgggagttgggagcagcaagacagtggctcaagatatcttaagactagtggagtacaccttgcatgttaaaagccttgctcagggctgcctggttcttgtaggacgacagagatggcctagctctgcatactgcacccccaggggctcagaacagtgcaaatgtcagtctatctgtcagtggcagagccagccttggagcaggggtgcaaggaggtctctgcactggccaggcatgcagaacattctgttcagtagcactggacagaaggccccatctagatgagacagagctggtggggcaggacaaagactcctggcagctcaaacggcctggcagatgcttggagagagggggcttcttgagacagcaccatttctgggaagagagtcacctgggagggatgaggccacgctccggcttggaggtgaagagaggggctgctgcaagaaagaattagagacatgccagcctttgctgtgttgcccaggctggtcatgaactcttggcctcaagcaatcttcccacctcagcctccccaagcgctgggattatagacatgagcccccatgctggccaataaaagatgattttatggaggggatggtggtgaaggttgtgggtggtatgaaatagtaagaaatatatattggtctgcacccagttcctgccacagagctcctaaaatcctgagaacttcctgggtgagcatcttttgttctaatgaggtgactcttggtggctcctggataggagtgaatcaccagaaagatcaagccagagttagaagcagaaagtgctggctataacacaggaaagctgtaacacaaataataaagtttttttttttttttttgagatggagcctcactctgttgcccaggctggagtgcaatggtgcaatctcagctcactacaagctctgcctcccaggttcaagtgattctcctgcctcagcctcctgagcagttgggactacaggtgtgtgccaccacatctggctaatttttgtatttttagcagagacggggtttcaccatattaaccaggctggcctcaaactccttaccttgtgatccgcctgcctcagcctcccaaagtgctgggattacaggcatgagccaccgtgcctggccaaaagacattgttcttaaaagaatcaactaactaaccaaataaataaaaatctaacctaattaagaaactaaaaatacacaaaaattaatttcaaggggagaaaaatcatgtaaagagagaaagataatgaatactttgcagaaatttatgaacataaacataaaacttggatgaaatgcatttctaggaaaacataatttatcaaaactaaccacaagtaaaatagaagcctaaataggatattttcaagagaagaagtaaagttgtcaaagtgctacccttcaaaaaaacaccaggctcaaacaatctgacatgggaatgttagcacaccttagagagcaaataaaactttgaatgggcttgaaatattccagactctagaaaaacaaaacttcccaattctttttataaagcaagtataaattgataccaaaatcttataaagaccttatacaaaacttcataccaatctcttttatgaatacaaaacccttaataaagtattaccagacagaacccaacaatacataaaaatgtcacatcataacatagtggggtttatttcaataatgcatggatggttcaatacaaggaaattcagtaacacaatataatagatcatgtgaatatacccaaagaaaaaatagattattttcatagatgctgtaaaggcatttgaccaaattcaacacctactttttaggtggtcaataaaataaattagttactccttctttagcatgataaaatatatttatcagcccagaaggcatcattttacccgataagggcacacgctggagggaataatgttaaaattaggaataagaggatagctagtttctttcttcttttttttttttgagacggagtcttgctctgttgccaggctggagtgcagtggtgcaatgttggctcactgcacgccccccgcctcccaggttcaagcgattctcctgcctcagcctcccgagtagctgggactacaggcgcgcaccaccatgcccggctaatttttttttgtattttagtagagatggggtttcaccatgttggtcaggctggtcttgaactcccaacctcacgtactgggattaccggtgtgagccaccacgccagcccaactactttcaacattatccttaatactgatgcttattgacttactatggggttacctctagataaatccataataagttgaaaatataagtaaaaaatgcccttaatacacctaacctaccaaacatcatagctgagcccagcctgccttagctatgctcagacactgacgtcagcctacaattggcaaaatcacacagcagcacagtctactgcagagcatctgctgtttgcccttgtgactgcgtggctgcctgggagcttcccagcttcacaagacagtattacgtagcacatcactagcctggggaaagatcaaagttgaaaatttgaagtgtggtttccattgaatgtgtactgcttttgcaccatcatcaagtcaaaaaattttagttgaaccagcctaagtttgggaccatctttattttcaggaggaacttccatgtacattgatgacggacgatagaatccgtttctatcatcctaatgaacataatgaataaatccagacaaacataaacattaacagagtaagcagctttcggggctggaagccagaagagggtgggagcgcagagagagaggccaaacaccagggctgcttctgctttgcgggtatttgctgatctggacaaggtatctggaaggctgagctaagcctcctttttttttgaggtggcgtctcactctgttgccaggctggagtgcaatggtgcgatctcagctcactgcaacctccacctccctggttcaagcgattctcctgcctcagcctcccgagtagctgggattacaggctcccgccactacacccagctgatttttgtaattttagtagagacggggtttcaccatgttggccaggatggtctcgatctcttgacgtcatgatctgtccacctcggcctcccaaagtgctgggattataggcgtgacccaccgtgccccgtctgagctaagcctcttgagcataggggactaaaaatgaaatctagcgcatgccaagtttagggtcccaggcaattcctttccactttggggtccactttggggtccaccccacccaagaagaaggatgacttggaagtaaaccagctctgaaatatggatggtcctctgggaccataccaatcccttcatatcaaccacatccagttcctcaaaactggaacttggattaagatggcctaggacttctagtgtcccaggagcctggcattgcaaacaaaaatcctctccggaagaagataataccttaagcttcaaatgactctctaataaatttcaaatacaatgtccagcacacaaacacaaattaccaggaacgtgatatgaggcctgatggatgggaattagcagaaacttcaggcatgagaaacataccctcagaggcctagaatctatctagtgtctagataatggagatatgaaatacagacacttaaacaactatgtttcccatgttcaaagaggaaatttgcaaaacttgaaagtgttggcaggaaatcagaaactataaaatgtgacaacagcatactttagagtcagtataaattacggtcccgaaaactgcagaattccagaacttaatggtaaagcaagggtttaacagcagaatagaaatagccagagagaactaggaagtaagtcagatgacactacccagaataaggcactgagaggccaaggaatggaaaatgcagaagaaaggatatggtgagaggatctaatatacatttatttggagtaccagggagagagagaaggagaagaacagaagccgtgtttcaaggacggtgactgagaggcttcgaaactgatgaaagccatcagttcacaaattcaaagcccagtgaattccaaggagaaaaaaagaaatccatactgtgaaagcaagtccagacaatgacaaacaccatcaacaatacacaggacaggcataagatgcatttaatggggacactcagaggcagagggttatcagaaggaggcacttctctcccaagttctcatcatcccagggccagggacagctggtcacaccttagggagttcactaggagagggatctggcttcttgtcattctgggtatttgtagggaaattggaagggaaccgagagcacctagccaatcgcatagcaatgggagatttcaggctgtggggaatgtctttgctggtgaaaagaacatcctgaccttagaaatctttcaccgagggggatctgcgttccagaacttctggagctggtataggtaaggctttgagctttcctactgagccagcctgttgctaggttaccaaaggggacctcgagggccatctggccaacaagcagacttgtctctccttacacccccagacgtatcactgcaaaactacagaaaaccaaagacagagaaaatcttaaaagcagccagatttaaaaaatggcatattagtttcaaagcagcagccatgaaattgacagctgatgtctcaacagcaagaatgaaaagtggaagacaggccaggtgtggtggctcaggcctgtaatcccagcactttgggaggccgaggcgggtggatcacgaggtcaggagaccaagaccatcctggctaacatggtgaaaccccgtctctactaaaaatacaaaaaaattagtcgggcatggtggtgggtgcctgtagtcccagctactcgggaggctgaggcaggagaatggcgtgaacccgggaggcggagcttgcagtgagccgagattgtgccactgcactccagcctgggtgacagagcaagactctgtctcaaaaaaaaaaaaaaaaaaaaaaaaaaaagggtgacgaagcttcaatctcctgaaaggaagcaactgccgcctttgattcgatacccaccaaaatccgtgaagaaggaaggcaaaataaaaacacttcctgattgaactggaaagatttccgcaatagaagacccactgtccaaggaattctaaaggatgctttccaggcagaagaaaatgaccccagaggaagatcagagattcaggaaagaaatggagagtgataaaaatggaaaattcgggggccaatttaaacaaaagctgactgctctacaactgttgtgtctctatcttttgtaacatatatgtgtgtgtagcttttttttttttttttgtcaagatggattctcactctgtcgcccaggctacagtgaaatggcacggtctcggctcactgcaacctctgccccttgggctcaaatgattctcttgcctcagcctcctgagtagctgagattacaggtgcctggcacaatgcctggctaatttttgtatttttactagagatgggatttctccatgttggccaggctggtcttgaacacctgacctcaggtgatccacctgcctgggcctcccaaagtgctaggattacaggcgcgagccactgcatctggcctatgtgtgtgtttatatggaattaaaacacatggcaataataccctccaaattgggagaaaccaaaaatagcatttaaatgttgtaagctccctgcataatcaagaagagaatagatttacgttagattttgatacctggaggatgaatgttgtaatttctagggtgaccatgaaaagaggagacaacggtgtatgtttttttttttttgagatggagtctcactttgtcacccaggctggagtgttgtggtgtgatcttggctcactgcaacctcctcctcttgggttcaggccatcctcccacctaggcctccagagtaggtgggatcacaggcacctgccaccacacctggctaatttttttttttttttaaatatttagtagagatggggtttcaccatgttggccaggctggtcttgaactcctgacctcaggcgatctgcctacctctgcctctcaaagtgctgggattacaggtgtgagccatcgcgcccggccaacagtgatcactttcaaactaacagaggttcaaaaataaaatcagacttaaccaaaaaccaggtaacagagctggtaggatatacagaaagactgacctcacgtatatcaacgattacagttaatattaatgaaggaaatgctctagtttaaaaacgagggttgtcaaagaccccacataagaagctccttaccagcggtgcacctagaacctaaggaaacaggacagatgaaggaggacgcgcccccgccgctgtcctgcgcctcagccatcctatgagacgggaaaggtttctgtctgcagctgggcccgtgctctttaccagctcctggctttcttctctggaaggttcctgcctgttttgccctcacacctgctcctctctcagccctctcaggggtggggctggaggccaccaaagagcctcctctgctctccagttgctcgactgctcctcatttccccctggggtctgcgtcagggtttccttcttttccagccccaccccgcgtgcatcccacctggtctcgggtcggggctgctcccgcttactgccccctgcccaggctggtgtgcaccccctctggctgctttcaaggcctcttctctcttctcggcaggacaggcacaggcaggtggccaggtgtcatgcttagctccccgcccagtgagattctttcatttaacaatcttcccctgaatagttcatgttcattgctgaaaatttgaaaaatatggaaaagcacaaagattaagatataaaccgccctcaattcccctgcccagagagagtcactgctatgacttggtgactaggaaccttatttctctctcgctcttttttttttttttgagacagagtcttgctctgtcacccaggctggagtgcagtggctcgatctcagctcactgcaacctccgcctcctgggttcaagcgattctcctgcctcagcctcttgagtagctgggattacaggcacctgccaccatgcccggctaatttttgtatttttagttgagagagggtttcatcttgttggtcaggcggacttgaactcctgacctcaggtgatcagcccacctcggcctcccaaagtgctgggattacaggtgtgagccactgcgccttcatctctcttctgtgtatgtgtacgctgttttttctttagaatgggggacgttatcaggctctacatggtgtgtagtcggctagcatgttgtaagcctttccctgtgtcacaagtgctcatctggaacaggattctaatgactgcctgtggctatgttgggattcctttaactcagctccttctgcccagcatctatcttttttccatcttttgtcctaagtgttgctataataaatcattgatcacacatgcctgactgtttgcataggataaattacgggaaatgtttttgctgttcagggactgtgcccatttttaggcctcagagacaccatgccagactgcccagtattgatctttactctttttagatgatgccaaacttttctgtgaactttaaaaacctgtgtcttgacagtccatttctgtaagtctttcacattagatttcctgtcaggatgatagtcaattctaggcagatgatgttttctcagccatggctgaagcagttgtgatttgttgtggccatgtaaagtcccgatgatccattgcctccctggatgggttggaataatttggtttgggagcatataacagaatgacctggagtcacagcagctcagacggaagtgtatttctcccttacagatgaaagaattccaggccaggctggaatgacaactgcacacagtcatctgggccccctccttccagctcccatcaccccaggatgtggcttttatgcagatgatccaaaatggctgctcaagtcccagccaacacatcccattccagggagcaggaaaaaggtgtgtctttcccttcattttatgtgattcctttctagaagtactactcattacttctgcttgcatctccctggctagcacttacttagttatatggccatagctagctgaaggaaggacagggactgtcatacactagctaagaggcaaactgcttagataaaaaggtctctaaagaaggtcagagcggctgctagggtgcaactctattacttattgttatgggacgaactgtgtccctcattcaggttgatgtcctaagccccagaacctcagaatgggattgtatttggagacaggttctttaaggaggtaaggaggctaaaatgagatcattagggtgggccataatccgactgatgtcttacaagaagagattaggacacggacatgctcagagggacggccacgtgaggacaccaagaaaggcagctgtctgcaagtcaaggacagggctcaggggaaaccaaccttgccaacaccttcatctcggacttctagcctctaggaccatgagaagatacatttctgttgtttaagctgcccggtctgtggtactttgttatggcagcccaagtaaacaaatacagtcatctgctgctggaacaaatcaccccagcactgtggcttggcagcacacatgtctagtcatagagttatatgtagttacgtgtagagccatatgtatcgtcacacgttctgtgggtcaggaatttggacccagcttaaccagctccacttctcgccagggttcagtcaaataccagctgcctcccacctgagagctcagccggggaagggtccctttccaatctcacgtggtgttggcaggatccagttcctcatggcctgctggactgagaacctcagttctcactgcctgttggccagaggccgcctttatgtcctcgccatgtgggcctctccaacatggcagctgacttcatcagagcatccatgccaagaaggcaacagagagggccagggagactgaagtcatacccttttgcgacctagtcatggggtgacattccatcacctttgcccattggttagaagcaggccaccaggtacagcccaagctcacggggaggggtcatacaagggtgtcaataccaggaggtgaggggtgctggggccatcttatgagtctgcccactgaggtaactaacaaccttgaggcctgacacagtggacaaaggcccttattaacagcagagaactgggaactttatttatttatttatttttgagacagagtctcactcttgtcacccaggctggagtgcaatggcatgatcttggctcactgcaacctccacctcccaggttcaagcaattctgcctcagcctccggaatagctgggactacaggcatgcaccactacacccggctaatttttgtatttttagtagagacagggtttcgccatgttggccaggctggtctcgaactcctgacctctggtgatctgcctgccttggcctcccaaagtgctgggattacaggcgtgagccaccgcacctcgctggaacttaatttttttagagacagtgtcgctctatcacccaagctggagtgcagtggtgcaatcctagctcacttgcagcctcaaattcctgggttcaggtgatcctcccacatcagcctcccaagaactgggaactaacagctgtttctctgctgtccttctcaagaaaagggaggctactgctaccccactggggacaatgctgggtttccctttaggacaggctctgagacaaggcggaggtgctgtttgtggccacagagcaggggactctgggttgcaggtgtggcctggctaaagtaggctttactgggctcctctctgcctgcatcaccccccggctgggcggttgtctctgaggccaaccttactccctgctgggcaggctggacagctgccctctccgtttgcccctctaccacccaaaaggcaggaggctctggagaccaggaccctgcccgccacggcctgtgtcccaggcgtgagggggtgccccacagacctctgctgagctgctgctgaatgacgccccttgggggtcctgccggaaggtcagagcaggggtgcactcccataaagaaacgcccccaggtcgggactcattcctgtgggcggcatcttgtggccatagctgcttctcgctgcactaatcacagtgcctctgtgggcagcaggcgctgaccacccaggcctgccccagaccctctcctcccttccggggcgctgcgctgggaccgatggggggcgccaggcctgtggacaccgccctgcaggggcctctccagctcactgggggtggggtgggggtcacacttggggtcctcaggtcgtgccgaccacgcgcattctctgcgctctgcgcaggagctcgcccaccctctccccgtgcagagagccccgcagctggctccccgcagggctgtccgggtgagtatggctctggccacgggccagtgtggcgggagggcaaaccccaaggccacctcggctcagagtccacggccggctgtcgccccgctccaggcgtcggcgggggatcctttccgcatgggcctgcgcccgcgctcggcgccccctccacggccccgccccgtccatggccccgtccttcatgggcgagcccctccatggccctgcccctccgcgccccacccctccctcgccccacctctcaccttcctgccccgcccccagcctccccacccctcaccggccagtcccctcccctatcccgctccgcccctcagccgccccgcccctcagccggcctgcctaatgtccccgtccccagcatcgccccgccccgcccccgtctcgccccgcccctcaggcggcctccctgctgtgccccgccccggcctcgccacgcccctacctcaccacgccccccgcatcgccacgccccccgcatcgccacgcctcccttaccatgcagtcccgccccgtcccttcctcgtcccgcctcgccgcgacacttcacacacagcttcgcctcaccccattacagtctcaccacgccccgtcccctctccgttgagccccgcgccttcgcccgggtggggcgctgcgctgtcagcggccttgctgtgtgaggcagaacctgcgggggcaggggcgggctggttccctggccagccattggcagagtccgcaggctagggctgtcaatcatgctggccggcgtggccccgcctccgccggcgcggccccgcctccgccggcgcagcgtctgggacgcaaggcgccgtgggggctgccgggacgggtccaagatggacggccgctcaggttctgcttttacctgcggcccagagccccattcattgccccggtgctgagcggcgccgcgagtcggcccgaggcctccggggactgccgtgccgggcgggagaccgccatggcgaccctggaaaagctgatgaaggccttcgagtccctcaagtccttccagcagcagcagcagcagcagcagcagcagcagcagcagcagcagcagcagcagcagcaacagccgccaccgccgccgccgccgccgccgcctcctcagcttcctcagccgccgccgcaggcacagccgctgctgcctcagccgcagccgcccccgccgccgcccccgccgccacccggcccggctgtggctgaggagccgctgcaccgaccgtgagtttgggcccgctgcagctccctgtcccggcgggtcccaggctacggcggggatggcggtaaccctgcagcctgcgggccggcgacacgaacccccggccccgcagagacagagtgacccagcaacccagagcccatgagggacacccgccccctcctggggcgaggccttcccccacttcagccccgctccctcacttgggtcttcccttgtcctctcgcgaggggaggcagagccttgttggggcctgtcctgaattcaccgaggggagtcacggcctcagccctctcgcccttcgcaggatgcgaagagttggggcgagaacttgtttctttttatttgcgagaaaccagggcgggggttcttttaactgcgttgtgaagagaacttggaggagccgagatttgctcagtgccacttccctcttctagtctgagagggaagagggctgggggcgcgggacacttcgagaggaggcggggtttggagctggagagatgtgggggcagtggatgacataatgcttttaggacgcctcggcgggagtggcggggcagggggggggcggggagtgagggcgcgtccaatgggagatttcttttcctagtggcacttaaaacagcctgagatttgaggctcttcctacattgtcaggacatttcatttagttcatgatcacggtggtagtaacacgattttaagcaccacctaagagatctgctcatctaagcctaagttggtctgcaggcgtttgaatgagttgtggttgccaagtaaagtggtgaacttacgtggtgattaatgaaattatcttaaatattaggaagagttgattgaagttttttgcctatgtgtgttgggaataaaaccaacacgttgctgatggggaggttaattgccgagggatgaatgaggtgtacattttaccagtattccagtcaggcttgccagaatacggggggtccgcagactccgtgggcatctcagatgtgccagtgaaagggtttctgtttgcttcattgctgacagcttgttactttttggaagctaggggtttctgttgcttgttcttggggagaatttttgaaacaggaaaagagagaccattaaaacatctagcggaaccccaggactttccctggaagtctgtgtgtcgagtgtacagtaggagttaggaagtactctggtgcagttcaggcctttctcttacctctcagtattctatttccgatctggatgtgtcccagatggcatttggtaagaatatctctgttaagactgattaatttttagtaatatttcttgttctttgtttctgttatgatccttgtctcgtcttcaaagtttaattagaaaatgattcggagagcagtgttagcttatttgttggaataaaatttaggaataaattattctaaaggatggaaaaactttttggatatttggagaaattttaaaacaatttggcttatctcttcagtaagtaatttctcatccagaaatttactgtagtgcttttctaggaggtaggtgtcataaaagttcacacattgcatgtatcttgtgtaaacactaaacagggctcctgatgggaaggaagacctttctgctgggctgcttcagacacttgatcattctaaaaatatgccttctctttcttatgctgatttgacagaacctgcatttgcttatcttcaaaatatgggtatcaagaaatttcctttgctgccttgacaaaggagatagattttgtttcattactttaaggtaatatatgattaccttatttaaaaaatttaatcaggactggcaaggtggcttacacctttaatccgagcactttgggaggcctaggtggacgaatcacctgaggtcaggagtttgagaccagcctggctaacatggtgaaaccctgtctctactaaaaatacaaaaattagctggtcatggtggcacgtgcctgtaatccaagctacctgggaggctgaggcaggaaaatcgcttgaacccgggaggcagagtctgcagtgagttgagatcacgccactgcactccagcctgggtgacagagcgagactctatctcaaaaaaaattttttttaatgtattatttttgcataagtaatacattgacatgatacaaattctgtaattacaaaagggcaataattaaaatatcttccttccacccctttcctctgagtacctaactttgtccccaagaacaagcactatttcagttcctcatgtatcctgccagatataacctgttcatattgtaagatagatttaaaatgctctaaaaacaaaagtagtttagaataatatatatctatatattttttgagatgtagtctcacattgtcacccaggctggagtgcagtgatacaatctcggctcactgcagtctctgcctcccaggttcaaatgcttctcctgcctcagccttctgagtagctgggattacaggcgcccaccaccatgtccagctaatttttgtatttttagtagagatggggtttcaccatgttggccaggctggtcttgaactcctgaccttgtgatctgtccacctcggcctcccaaagtgctgggattacaggtgtgagccaccatgcctggctagaataataacttttaaaggttcttagcatgctctgaaatcaactgcattaggtttatttatagttttatagttattttaaataaaatgcatatttgtcatatttctctgtattttgctgttgagaaaggaggtattcactaattttgagtaacaaacactgctcacaaagtttggattttggcagttctgttcacgtgcttcagccaaaaaatcctcttctcaaagtaagattgatgaaagcaatttagaaagtatctgttctgtttttatggctcttgctctttggtgtggaactgtggtgtcacgccatgcatgggcctcagtttatgagtgtttgtgctctgctcagcatacaggatgcaggagttccttatggggctggctgcaggctcagcaaatctagcatgcttgggagggtcctcacagtaattaggaggcaattaatacttgcttctggcagtttcttattctccttcagattcctatctggtgtttccctgactttattcattcatcagtaaatatttactaaacatgtactatgtgcctggcactgttataggtgcagggctcagcagtgagcagacaaagctctgccctcgtgaagctttcattctaatgaaggacatagacagtaagcaagatagataagtaaaatatacagtacgttaatacgtggaggaacttcaaagcagggaaggggatagggaaatgtcagggttaatcgagtgttaacttatttttatttttaaaaaaattgttaagggctttccagcaaaacccagaaagcctgctagacaaattccaaaagagctgtagcactaagtgttgacatttttattttattttgttttgttttgttttttttgagacagttcttgctctatcagccaggctggagtgcactagtgtgatcttggctcactgcaacctctgcctcttgggttcaagtgattctcatgcctcagcctcctgtttagctgggattatagacatgcactgccatgcctgggtaattttttttttttcccccgagacggagtcttgctctgtcgcccaggctggagtgcagtggcgcgatctcagctcactgcaagctccgcttcccgagttcacgccattctcctgcctcagtctcccaagtagctgggactacaggcgcctgccaccacgtccagctaatttttttgtatttttaatagagacggggtttcaccgtgttagccaggatgatcttgatctcctgacctcgtcatccgccgaccttgtgatccgcccacctcggcctcccaaagtgctgggattacaggcatgagccactgtgcccggccacgcctgggtaatttttgtatttttagtagagatggggttttgccatgatgagcaggctggtctcgaactcccggcctcatgtgatctgcctgccttggcctcccaaagtgctaggattacaggcatgagccaccatacctggccagtgttgatattttaaatacggtgttcagggaaggtccactgagaagacagctttttttttttttttttttggggttggggggcaaggtcttgctctttaacccaggctggaatgcagtatcactatcgtagctcacttcagccttgaactcctgggctcaagtgatcctcccacctcaacctcacaatgtgttgggactataggtgtgagccatcacacctggccagatgatggcttttgagtaaagacctcaagcgagttaagagtctagtgtaagggtgtatgaagtagtggtattccagatggggggaacaggtccaaaatcttcctgtttcaggaatagcaaggatgtcattttagttgggtgaattgagtgagggggacatttgtagtaagaagtaaggtccaagaggtcaagggagtgccatatcagaccaatactacttgccttgtagatggaataaagatattggcatttatgtgagtgagatgggatgtcactggaggattagagcagaggagtagcatgatctgaatttcaatcttaagtgaactctggctgacaacagagtgaaggggaacaccggcaaaagcagaaaccagttaggaagccactgcagtgctcagataagcatggtgggttctgtcagggtaccggctgtcggctgtgggcagtgtgaggaatgactgactggattttgaatgcggaaccaactgcacttgttgaactctgctaagtataacaatttagcagtagcttgcgttatcaggtttgtattcagctgcaagtaacagaaaatcctgctgcaatagcttaaactggtaacaagcaagagcttatcagaagacaaaaataagtctggggaaattcaacaataagttaaggaacccaggctctttcttttttttttttttgaaacggagtttcgctcttgtcacccgggctggagtgcaatgatgtgatctcagctcactaaaacctctacctcctgggttcaagtgattcttctgcctcagcctcccaagtaactgggattacaggcgtataccaccatgcccagctaatttttgtgtttttagtagagatggggtttcaccatgttggccaggctggtctcgaacttctgacctcaggtgatccactcgcctcagcctgccaaagtgctgggattacaggtttgggccactgcacccggtcagaacccaggctctttcttatacttaccttgcaaacccttgttctcattttttccctttgtatttttattgttgaattgtaatagttctttatatattctggatactggattcttatcagatagatgatttgtaaaaactctcccttcctttggattgtctttttactttcttgatagtgtcttttgaagtgtaaaagtttttaattttgatgaagtcgagtttatctattttgtctttggttgctgtgcttcaagtgtcatatctaagaaatcattgtctaatccaaagtcaaaaaggtttactcctatgttttcttctaagaattttagagttttacatttaagtctgatccattttgagttaatttttatatatggttcaggtagaagtccaactttattcttttccatgtggttattcagttgtcccagcactgtttgttgaagagactattctttccccatggaattatcttagtacccttgttgaaaattaatcgtccttaattgtataaatttatttctagactgtcagttctacctgttggtctttatgtcgatcctgtgccagtaccatacagtcttgattactgaagtttgtgtcacagtttaaattcatgaaatgtgagttctccaactttgttccttttcaagattgatttggccatgctgggtcccttgcatttccgtacgaattgtaggatcagcttgtcagtttcaacaaagaagccaagtaggattctgagagggattgtgttgaatctgtagatcaacttggggagtattcgcatcttaacaatattgtcttccacctatgaacatgggcaaactttgtgtaaatggtcagattgtaagtatttcgggctgtgtgggcacagtgtctctgtcacagctacgcggctctgccattgtagcatgaaagtagccataagcaatatgtatgagtgtctgtgttccaatagaattttattaatgacaaggaagtttgaatttcatataattttcacctgtcatgagatagtatttgattattttggtcaaccatttaaaaatgtaaaaacatttcttagcttgtgaactagccaaaaatatgcaggttatagttttcccactcctaggttaaaatatgataggaccacatttggaaagcatttctttttttttttttttttttttttttgagacggagtttcactcttgttgcccaggctggagtgcagtggcgcgatctcggctcactgcaacctctgcctcccaggttcaagacattctcctgcacggcctccctagtagctgggattacaggcatgcgccaccacacccagctaattttgtatttttagtagagacggggtttctccatgttggtcaggctggtcttgaactcctgacctcaggtgatccacccgcctcagcctcccaaagtgctgggattacagggtgtgagccaccacaccctgctggaaagcatttcttttttggctgtttttgttttttttttaaactagttttgaaaattataaaagttacacatatacattataaaaatatcttcaagcagcacagatgaaaaacaaagcccttcttgcaagtctgtcatctttgtctaacttcctaagaacaaaagtgtttcttgtgtcttcttcccagattttaatatgcatatacaagcatttaaatgtgtcattttttgtttgcttgactgagatcacattacatatgtatttttttacttaacaatgtgtcatagatattgttccatagcagtacctgtaattcttattaattgctatgtaatattttagaatttctttttaaaagaggacttttggagatgtaaaggcaaaggtctcacatttttgtggctgtagaatgtgctggtgacatattctctctaccttgagaagtccccatccccatcacctccatttcctgtaaataagtcaaccacttgataaactacctttgaatggatccacactcaaaacatttagtcttattcagacaacaaggaggaaaaataaaataccttataaagcactgtttaatattgtattaaattggatcaatttgggggctagaatgtatgttagagacatgatatgtccataggtccttgctatcacagtgaggtctcagggacagtcgtttggtatcatttgggatctcataagcagactctctctgcttgacctgacaaatcagagtctgtgttttaacaggttcagtgagtgacttacatgcacattggagtttgggaagctccactgtaggtgcttagaccttacctttgttgttgctaataacaatgcaagcatttgggaggaagacctgtgttgctcatatgtgtccaggtgtagctgaggtggccttgcttatctgctgtagggccgttgagcatttctgtagctgtgatgagtgagctgaggtgagcctgcggagagctcccagccattggtagtgggactcgcttagatgaactggaaggaccctttcatctgagcagccactatggagaaaaacaaccgaatgaggggagagacaatgtgcaattttatttagggcacaaaggagagctgtggttagaaggtgacatttgagtggaaagggggcaagccatgtgtatagcgggagaagagaggtccaggcagagttaacagaaggcagaaatgctttccatgtttgagaaccagtaaggaggccagtggctgaagtaaggtgaagggcagaaataaggatgaggctgcgagagatgagaggttagagacgagcgtcttgtgcaccaagataagcttgtgtggtcaaaacaagtagtttaatttatgtttttaaaagatcattttggctgggcacaatggttcatgcctgtaataccagtagtttgagacggtgtggtgggaggattgcctgaggccagacgaccagcatagccaacatagcagcacctataaggtctctacaaaaaactttaaaaaattagctgggcatagtggtgtgtgcctgtagtcccagctactcaggaggctgaggaggctggaggattgcttgagtccaggagtttgaggctgcagtgagctatgattatgccactacactacaacctgggcaagagagtgagaccctgtctctaaatatacacacacacacacacacacacacacacacacacacacacacacacacacacacacatatatatgtatatatatgcatttagatgaaaagatcactttgacaataccacatgctggtgaggatttagaaaaactaggtcacttattgctggtgggaatataatatagtacggccactctggaaaacagtttggcagtttgtcataaaactgaacataccgttagtatacagcccagcagcaactacaatcctgggcattaatcctagagaaatgaaaccttaatgttcacataaaaacctatactcaagtatgcatagcagctttacccataatatctaagaactggaatcagctcagatgtccttcaacaggtgaatggttaaactactcagtaataaaaaggaatgagctactgatagcatgcaacagtttaggtgaagttatgctaatgaaaaaagccaatcccaaaaggttatacatactgtatgattctatgtttttttgcaatggcacagttttagggatggagaatagattagtggttgcctggggttagagatggggtagtagagtaggttagtggtggcagaggagagaaaagagagggaggtgaatgtggttataaaaggacaacacaggggaatacttgtaatggaaatgctttgtctttttttttttttttttttttttggcgacagagtcttgctctgttgcccaggctggagtgcagtggcatgatcttttctcactgcaacctctgcctcctgggttcaagtgatacttgtgtctcagtctcccatgttcagagtgaaacaaaccagaggtaatgttcatccaaataatccaacacacatgacattaaaacatcaagatcaggtcggacgtggtggctcatgcctgtaatcccagcacttttgggaggccaaggtgggcagatcacttgaggtcaggagttcgagaccagccgggccaacatgatgaaaccccatcttgactaaaaatacaaaaattagccgggcatggtggtgtgcacctgtagtcccagctacttgggaggctgaggcaagagaactgcttgaacccgaggggcagaggttgcagtgagctgagagtgcgccattgcacttcagcctgtgtgacagagtaagactccatctccaaaaaaaaaaaaccaagatcaattaaaatacagcattactgggccgggtgtggtggctcacacctgtaatcccagcactttgggaggccgagatgggcagatcacgaggtcaggagatccagaccatcccggctaacacggtgaaaccccgtctctactaaaaaatacaaaaaattagccgggtatagtggtgggtgcctgtagtcccagctacttgggaggctgaagcaggagaatggtgtgaacccgggaggcagagctggcagtgagctgagatcgcgccactgcactccagcctgggcgacagagcaagactccgtctcgggggaaaaaaaaaaataaataaatagaatgctgtagtgtccttgagtttacatgcccctccttacgcttgtgtgcccgtgcagattgcttgattacacaattagaggaggctggcggaggattgttttaatttttttttttttgagacagtctggctctgttccccaggctagagtgcaatggcgcaatcttggtgcactgcaacctctgcctcctgggttcaagcagttcttctgccgcagcctcccgagtagctgggattataggcgcccgccaccacgcccaactattttttgtatttttagtagagcagcgtttcaccatgctggccaggctggtctcgaactcctgacctcagatgatctgctgccccagcctcccaaagtgctgggattacaggcgtgagccacacctggccgtttgttttaattttgaaggtgaagtgaaagtgactacatttaccaaaagtgattgaaaagccaggactgttcttaccctgtttttccagttcttgctcagagcaaggtggtttctttttcacttaatcaccatacttacttttcatgtagaacaagtcagtttgagttatcagttcatcatcttaactaaattccatgggggaaggaattagttttagtttcttaaacttccaggtttgcttattggacaaaatgagatagcaaggcagtgtttttaagttagattttttatttctttggtaatacaattttctcagaaacttagtagtcttttagtttagttgtttttagttggtcctatgttttggatcacccctctctactttattttgatagtgccaactgtgaagacatctgaagccataggtttggatgggaaggaggcatctttagcctgatcatcttcgccaggctgtttatctccttttgcttggctgagaagtcttaataggaggcttattcccagctatttggggacatagaagcagttagccattgcttatattttactgaggtctgtgtggtatgttgattgtagtcagttaacgattttgagaactgaaggcagcctggtatatatagagtaggtattagactgtgtttcttctaattgaatttcccatctcttgtaatctatgccatcatcttctgtactgctgagaaagaaagaaagtttctaatcaaactataccactggttgtaagatgcagtttggctttagtgatgttaacacatgattcaaacgtgaaattgattgagtattggtgaaatacagaggagatttaaagccagaagacctgggtttaaatgctggctgtatgacttcatatctgtgtgatcttgggcatgtcatggttggcacttcaatttcttctctctataatgggggaagtgaggccagtcatggtggctcatacctataatcccagtgctttgggaggccaagatgggaagatcgcttgaggccaggagtttgagcaattgggcaacatcgtgaggccccgtctctacaaaatattttgaaaaaattagccaggcccagtggtgcgtgcctgtggtccgcgccactcaggaggctgagacgggaggatcctttcagcctaggagtttaaggctaaagtgagccatgattgtgctatcgtactccagcctgggcagcagagcaagatcctgactctaaaaaaaagtaaaataaagtaaaatgggggaaatgaactgctttagtaacatcatctgttttttctgtgagcagcgtagcttgacagccattggtgaactcgtgccctgtgcttccctgtccagatccccattctgcccgcaacatggagtataacggtttattcatagtagtcgagaaacactcactgaatgaatgaatgaggtgtagaactaagtggagtgggtaattcaacacatattaatttccttcttttttttatttttagaaagaaagaactttcagctaccaagaaagaccgtgtgaatcattgtctgacaatatgtgaaaacatagtggcacagtctgtcaggtaattgcactttgaactgtctagagaaaataagaactttgtatattttcagtcttaatgggctagaatattctttgtgtcccagctattttaaatggattcagaaatccatttaagatgaagaaggacccttttcccatatttctggctatatacaaggatatccagacactgaaatgaataatgttccctttttgtaatcttttatgcaaaaattaaaaccattatggtaattgaacaacatgtttatgtttagttaacacccttagcaactatagttattttaaaaccatctatggtttgatatttttgcatttgttgcaatagtaggaacagcacaagacagttcagtttgtctctcttatttgctttttcttggcagtttgctgtcctattgtacctctgctcctagcagtggctggagcccactcctctgtgcttcgggattagtggggatcgtggggcattgactgtaggtcagctttccttgcttgatctttctcactgggatgaactagcagcaccttcttttgtagctgctttgcttttgactatctttctgaccgttgttcctagtagctgtagatggtaaatatatttaggcctgtttccaatggctcagtaggagacatattcacctatgatatctgaattctgttacccacatgggcatgcgtgaaatagttgccttgccttactttcccttggaataaataattcatgttattctcctggtagaagctagaaaaagcctttatagtcagtcagaaaaaaatttttagacaaataatcttgattttagtactgacaaaaacgtgtggtgattctttttttaatttttttttgagacggagtttcactcttgttgcccaggctggagtgcaatggcgtgatctcggctcactgcaacctctgcctcctgggttcaagtgattctcctgcctcagcctcccaagtagctggagttacaggcatgtgctactgtgcccagctaattttgtatttttagtagagatgttggtcaggctgatctcgaactcccaaccttaggtgatctgcccgcctcagcctcccaaagtgctgggattacaggcgtgagccagggcgcccggtgattcatttgttttttcaaaaaatttcctcttggccattgcttttcacttttgttttttttttttttttgagacggagtcacgatctgtcacccaggctggagtgcagtggcatgatcttggcttactgcaagctctgcctcccaggttcacgccattctcctgcttcagcctggcgagtagctgggactacaggtgctcgccaccacacccggctaattttttgtatttttagtagagatggggtttcaccgtggtcttgatctcctgacctcatgacccgctcaactcagcctcccaaagtgctgggattacaggcgtgagccaccgcgcccggccctctcttgtctttttattgtggtaaaatgcacataaaattgactgtcttaaccatttttaggggtacagttcagtatatatattcgtaatgttgtacagccatcactgccatctacttcataagtttttcttctgtcaaaactgaacatctgtcttcattaaactccctatcatccattctttcctgtagtccctttctactttctgtctgtatgagtgtaactgctctggagacctcatgtaagtggattcctacaggatttgtgttttttttttggtgatctgcttatttttaatgcctctgtgcatttgtattatatactttcaaagtgatttcacaaaaccgtttcattttaggttaactcatttctgttgtttgtgaaatactgtgtatgattctgttctgtttctgtctaatttgtggaaatgttgtgggaagaaaatgaaataacaaatgagcatatgtcctgaaaataaaaatataaaaattctaagttagcatgctattgtagaatacaacgctatgataaaagtaggaaaaaaaaaggtttgaattctatctctgctacctgtgtaagctgggtgactttagataagctgtaacgtgtttgagccttactggctcatttttgaaatgtaatccctagttacacagttcttgtgggatcagatggtacatgtgaaacactgtgaaaaagcaactgcatagatatgttcattagccacctgagcgggaagcgtatcccattgcgatgcccatcatccaaagctatatgttatctttacttttttttttttgagacagagtcttgctctgttgcccaggctagagtgcagtggtgcaatctcagctcactgcaagctccacctcccgggttcacgctattctcctgccccagcctcccaagtagctgggactacaggcacccgccaccatgcctggctaaatttttgtatttttagtagagatggggtttcaccgtgttagccaggatggtcttgatctcctgacctcgtgatccgcccgcctcggcctcccaaagtgctgggattacaggcgtgagccactgcccctggccatctttactttttttgtgaaatgactttaaatacttggcaaacatttggtcattgttcatctgatctccaccatccaggtctcagagaacataatttctctctgaaagcttattgacccaggaaataagatctctttcaatctgagtgcgtcaggctttattcttgtcattttgtcttttgataattttcaaatggaattcatggaatgttggcttatattcatatattagtaaagtatgttgagacatcttaagattgatttgtggttctatatgccatattaaatcaaaataatagctgttaatggttttcacattagtctgtctcttgtttttatggagtaatgctgagagttcattatgcttgttctacagaagagcatgttaaaaggagtttttggagtcagagaggttattcttggtttcataggatacactctatactttttagggatttcagagtatatagctgaaggtgatattttatgtaaatatgttttatggaaacttattgctcatcgctgtttcctgttaactctcctaaaatataattaaacttttggaacttttttatagcttttgtgctagactaatttttgtctctaatgaggttatataaatggcagcttctgacgttttcaatgtaggaagtcatttaaaacttcatgtatattgtgaaaatgtagtctgctttaagctctctaaagtggtctaagttactggttcctaagtatggatgagcatcaaaatcatctggaaaatttgttaaaaatacagtaatgaaggcacctcactgtcctttttcccaaacatacttctgcattctgtttgagtaggtagggactacacatttttcacaagtatcctcttgggaatacccaggaatgcttacttgagcaacctcttactaatatgtaccttgataaggtggctaggtaaacataaatatacaaaaatccatagatctcccatatattagcataaatcagctagaaaatataacgtttaaagatctagttcacagtagcaccaatatatcgaactctaaggaatcgataaatatgcaaaaactttataaaaacttctgttaatgtttctgaaagatataggtgaccactttctagataggaagattttatattactaagttgaattttctctaaattaacacagaaatttaaaataatcttgatcaaaattctagtagaggtatttttgaacttgttcactgcaagaataaatacataattgcaaagaatatctcaaaatcatcaccaggcctggtgtggtggcccatgcctgtaatcccagcactttgggaggctgaggcaggcagatcacctgaggtcaagagtttgagaccagctggaccagtgcggtgaaacactgcctctactaaaaatacaaaaattagctgggtgtggtggtgcatgcctgtagtcccagctacttgggaggctgaggcaggagaattgcttgaacccaggaggtacaggttgcggtgagcctagatcgcaccactgcattccagcctgggcgacaagagcaaaattctgtctcaagaaaaaagagaaaaaagaaaaagaaatcaacactaatatggtgagacttaatgtatgtgacattaaaatagtgattggatgttaaaacaggtatagaacagaaagaagagtgtatgtgtgtatctgtatgaatttatgatgggtgtaacatatatgtattagggaaatgagggaaatgatacatttctctgactttgggagaacattatatctctacctcatattgcaaacaaacataaagttcagattaattacctaaatgtgaaaaaatgaaataatttctttaaaaaatgtaatcttagtttgaggaaggttaacattataaaggaaaaaactgttttgagtggaatatagttcaatatgtcaaaatccaccttcaacaaaattgaaagtaaattgaacttggggaaagtattgacagcatatagatcaaaggttactagcctgtgtaaagagcagttataaatatcgttaagaaaaacactgtcgacctgtcggcaccttgttctccgactcccagcctccagaactgtgacgagtaagtgcttattgtttaaaccacccagtctgtatgtggtattttgttatagaaactcaagctgattaggacactagtaatcagtagactgaaactgaaacaaaaataagaaccttttttacctgtcaaattggcaaacattaagaatattcagatttttgtcagaggtgatacaaccttctaagaaggcaatttgggaaaatataaagctttagattattatatgtctgacctagcagttttacctctagggtgcttacccctaggaaagtgtgtaatgatattggtgcagtgcccttcatcccattagaaaattaaaaataaccttaatggcctaccactaaaaggggattgaaaatttaagatatatttatttatgtgtttattgagatggagtcttgcactgtccgcctgggccagagtgcaatggtgcgatctcggctcactgcaacctctgcttcccgggttcatgtgattctcctgcctcagcctcctgagtagctgggattacaggctcacaccaccgcacccggctaattttttgtatttttagtagagatggggtttcactgtgttggccagactggtctcgaactcctgacctcatgatccgcgcccctcggcctcccagtgttgggattacaggtgtgagccactgcgcctggccagatacatttatacaagagaatgttagttaacattcatagatatttatattttgtttactttttattaaaaaaattttttttagagacaggatcttactctgtcacccaggcaggatgcagttgcacaatcatagcccactgcagcctgaactcctgggcttaagtgatccttctgcctcagccttttgagtacctgggggactttaggcagtgctactatacctggctaatttttaaatgttttatagatgagatcttgctgtattgcccaggctggtctagaattcctgggcccaagtgatcctcccaccttggcctcccaaagcgctgagattacaggcatgagccaccacttctgaccaatagatatttatatttgtgactggaaaatatattaacaatgtgttaaaaaattcagttaaaaaataatgaaagatttttgcttctggctaagatagaataacaaggacagcatttatcttcttgccttgaaatagttgaaaacggaagaaatatatgtaacagtggttttcaagttattgggcatcaggcaaagaagaatagttatcccaggaaaatgaatgtggagagccctacaatttccttacattactgcctggtcatggcaagaggaaaaactgagaggagactgaggctgagccagtggtttgctgggttgaggaggcagagctgggagtgcagagatgcaaggtggtgagagcccatatggaagaataccagggaagagagctgcagagggagctccggagacctgcaccctgccctctcagtaccctgtcatgtgtgtagctgagtactgacgagcacttgcttgtgcggaaatgacccagggctggaggtagagccacctgaaaggattagaaggaacagttgctgaaagtcacacagggccaggaagaatttctaatcacaccagttggagtggaaaacctcagctctcatagagcaggtagggtactcagaagggtttgcccacctagccccagactaagtttcgttactctgaccctacctaatattaaaaagagattaattaaattgttcgcaacaaaaataatatatttcagtgtttgtaacacgtagaagtgaattgtatgacaatagcataaaggctggaagagcagaaattgacatgtatttgcgctgggcagaataatgctcccctctttccccaaaagatatcaagtcctaatccctggagcctgtaaatattactttatatggaaaattgttttatgatgtgattaaattcaggatcttgagatgagggggctatcttggatgatctgggtaggcactaaatgcaatcacatatatataaaaaggaggcagagggagattttacacacagagagaaggccctgtgaagatggaacagaaagatttgaaggtgctggccttgaaaattggagtgatgaagctataagccaaggaatgcagcagccaccaaagctggaagaggcacggagcagttctcatttagagcctactccagagggaatgtggtgctgccaattccttttttttttttttttttaagatatcatttacccctttaagttggttttttttttttttttttttttttagtatttattgatcattcttgggtgtttcttggagagggggatttggcagggtcataggacaatagtggagggaaggtcagcagataaacatgtaaacaaaggtctctggttttcctaggcagagggccctgccacgttctgcagtgtttgtgtccctgggtacttgagattagggagtggtgatgactcttaacgagtatgctgccttcaagcatctgtttaacaaagcacatcttgcaccgcccttaatccatttaacccttagtggacacagcacatgtttcagagagcacggggttgggggtaaggttatagattaacagcatcccaaggcagaagaatttttcttagtacagaacaaaatggagtgtcctatgtctacttctttctacgcagacacagtaacaatctgatctctctttcttttcccacatttcctccttttctattcgacaaaactgccaccgtcatcatggactgttctcaatgagctattgggtacacctcccagatggggtggcggccgggcagaggggctcctcacttcccagatggggcggccgggcagaggcgccccccaacctcccagacggggcggcggctgggcgggggctgccccccacctcccggacggggcgggtggccgggcgggggctgcccaccacctcccggacggggcggctggccgggcgggggctgccccccacctcccggacggggcgggtggccgggcgggggctgccccccacctcccggacggggcggctggccgggcgggggctgccccccacctcccggacggagcggctgccgggcggaggggctcctcacttcccggacggggcggctgctgggcggaggggctcctcacttctcagacggggcggctggtcagagacgctcctcacctcccagacggggtggcagtggggcagagacattcttaagttcccagacggagtcacggccgggcagaggtgctcttcacatctcagacggggcggcggggcagaggtgctccccacttcccagacgatgggcggccgggcagagatgctcctcacttcctagatgggatgacagccgggaagaggcgctcctcacttcccagactgggcagccaggcagaggggctcctcacatcccagacgatgggcggccaggcagaaacgctcctcacttcctagacggggtggcggctgggcagaggccgcaatcttggcactttgggaggccaaggcaggcggctgggaggtgaaggttgtagtgacccgagatcacgccactgcactccagcctgggcaacactgagcactgagtgagcgagactccgtctgcaatcccggcacctcgggaggccgaggctggcagatcacttgcagtcaggagctggagaccagcccggccaacacggcgaaaccccgtctccaccaaaaaacacgaaaaccagtcagacatggcggtgcgtgcctgcaatcccaggcacttggcaggctgaggcaggagaatcaggtagggaggttgcagtgagtagagatggtggcagtacagtccagccttggctcggcatcagagggagactgtgcgagggcgagggcgagggcgagggaattccttaatttcagtttagtgatactaattttggactctggcctctaaaactgtgaaagaaaaaattttttgtttgtttgtttcttttaagccacatagtttgtggtaatttgttacagcagctgcaggaaactaatttatgctgcatgtgaaatggtgtaataaggtagattgtgatgaagatacatagtataaacaattaagcaacaactaaaagcacaacaaggaattatagctaatgaaccaaaaaaggagattagaataataaaaatggtgaatcccaaagaagccagaaataggggaagaggcaaataaaggaaagaaagagcttgatggtagatttcaacctaactatgtcaaaaaggacattacatgtaaaaggcagcgatttttcagattgaatggaaaagtaagactcggtatatgctgctgcctgcaagaaacacattctaaatataaaggcaaaaataacctacaggtaacagaacggaaagaagttcactgtgcttacaagaattagatgcaagctagactggttctgttaatatcagacaaagtggatttcaaagcaaaggctcttgcccaggatgagatggtcatttcataatgatgaaggggattcgttcatcagcctggcatagcaagctgaaatgtttatgcaccggactacagagctaaaatacatgaagcaaagcctgacagaactacaagtagaaacagacaaatccacagtgatagagatttcagtagccgctctcaatgatttgtagaacacgtagccataatatctggatctagaacacttgaccaacactgtcccctgtgcaacctcattggcatttacaggacactccacccagcaccagcagaagagacactctctcaagtgctcacagaatgtttgccaagatagagcagatgctgggccataaaacaagtctctaaattaaaagcattcaaattattcagagtatgttttctgacctcagtatcattaagttggaatatattataggaagataacctggaaaagcctcagatatgtggaaaaacccatttccacatggcccatgggtcagaagtgaagtcaaaagggaaatttgaaagtcttttggattgactgatataaaaacaatagatttctaaacttgtggggtgctgttacagcatagtaaatggaaatttctagcattaaatgcctgttttaggaaagaaagatttcaaatcaatgacctcagcttctacctttggaaacttgaaaatgacaagcaaatggaatccagagttaccagaagggccaggtacggtggcttatgcctgcagttctgccactttgggaggccgaggcaggtggattgtttgagactggcagttgaagaccagcctgggcagcctagggagaccccatatctacaaaaaacaaaaaaattagccaggtgtggtggcatgtgcctgtagtcccagctaaccaggagtctaaggtgggaggattgcttgagtctgggaggttgaggctgcagtgaactgtgattgtgccactgtgttccatcctgggcaacagaatgagaccctgtctcaaaaacaaaaacagttactagaagaatggacatcataaagataggagcagaagtcagtaaaatagaaaacaaaaatacataggaaatcaataaaaccaaaagctggttcatcaagaacatcaataaattggtaaagctgataggaaaaacagtgaagtcacaaattagcaatatcaggaatgagggagatgacagtagtatagattatatagatattaaaaggactgtatgaggcaggtgtggtggttcacgcctgtaatcccagcaccttgggaggccgaggtggacagatcacctgaggtcaggagtttgggaccagcctggccaacatggtgaaactctgtctctactaaaaatacaaaaattagttggtcgtggtgctgtgtgcctgtaatcccagctacttgggaggctgaggcaggagaattgcttgaacctgggaggcggaggttgcagtgagctgagattgtgccgttgcactccagcctgggtgacagagcaagactccatctcaaaacaaataaataaataaaaaggactatatggtaatattatgaacaactttatgccaataaatttgacaacttatagatgaaatggatgagttccttgaaagacacagaaactattaaagctctctcaagaagatatagataagctgattagccctatatctattttattgaatttaaatgtaaaaatcaatatttagttactggaaaacttttaagtgtggttggaaatggtatacgaactttttcaactgaattttatgaagtctaatcacaggtaaaggttttctgatgaaaatttagtgtctgaattgagatatactgtaaaaaatgttatatatcttaattatttcttcacattaattacatgttgaaataatactttgggtgtattgggttaaattaaatattatgaaaatcttgcctgttttctttttacttttgatgcgtcagctaggaaatataaaagtgtagctcacattctgtttctgttgacagtactgctttggagcacagtgtttgaatgatctatcatttcaaagacctttcctcagttcgttattcatggctgtctgtattccacatagataaggtctgaaatactgctaagtggcatgttttgttttatgcttttataagtttgttgatcattactgatgtggacttttggtgcctcttaggctcattgctatcttccaaccattgtttgcaatttttacctagagataaagagaaagagacatttggtttcagagtagttagattgggatcatgaaagagcaacctcattttgatgcttcaaaaatagcacatcccccgtattactgggatttgctattcttgggattacttcaagaacatccttgtgttactggtttggatgcttctgaatgctgtgaagtcagtttcatgtacatggctcatcagtttagctctctcttggctttgtttagacagttggagcatgatggcctaaacagcttctttcaattaaacattttaaaatagtttacaaatagtaaacaaactccagtttttgtgactctttgtctcgcacaacaaaaacacaatctgaccatgatcatctggcatcttagggtgaaatatggttatactttggcccataccgaaagcaagattaaaaaggggcaggagagatagactgctgaactgattttcaaggttccaagaatattgtaggttaagagtaaaagtaaacttttggtagaaagcagtgggttgtctaggattgaagtatctgaagtttttaaacgaaaatttaaaaagaaaaatgagaattgccttacaagtacaatctcttcttttttaaaaaataaactttattttgaaatagttttagatttatagaaaaaaattagatagggtaggaagttttcatataccctacatccagttaccccagttattatcatcctaatttagtgtgagacattttcatgtttaatgaatcaatattgatatgctattaacttaagtccagactttattcagattttcttaatttctatgtaatgtcctttttctgttccagaattccatgcaggacaccggatacctcattacatttcattgtcatgtcaccttaggctcctcttgacagtttctcttctttttttgcttagaaattctccagaatttcagaaacttctgggcatcgctatggaactttttctgctgtgcagtgatgacgcagagtcagatgtcaggatggtggctgacgaatgcctcaacaaagttatcaaagtaagaaccgtgtggatgatgttctcctcagagctatcattgttgtaggctgagagaagaagcgatcattgagtgttcttctgttttgagtccctgaggatgtctgcacttttttcctttctgatgtatggtttggaggtgctctgttgtatggtttggaggtgctctgttgtatggtttggaggtgctctattgtatggtttggaggtgctctgttgtatggtttggaggtgctcttgtatggtttggaggtgctcttgtatggtttggaggtgctctgttgtatggtttggaggtggtcttgtatggtttgcaggtgctctattgcatggtttgcaggtgctctattgtatggtttggaagtgctcttgtatggtttggaggtgctcttgtatggtttggagatgctctattgtatggtttgcaggtgctctattgtatggtttggaagtgctcttgtatggtttggaggtgctcttgtatggtttggaggtgctctgttgtatggtttggaggtgctctgttgtatggtttggaggtgctcttgtatggtttggaggtgctctattgtatggtttggagatgctctggtatctgcctgcattgcttgccacacctgcccggtcagaaggcgctatgttgacaattgtgcctgcacggtgcctaggtcaatgaagggaaccgatggtagccactggatgctcctgggaaaatgtcactacaggcaccagagaagccagagctatgcccaaatttctatgagtctcagttttcttaaccataaaatgggatcaatgtttttgtggcatgtgtatgagtgtgtgtctgtgtatgtgtgaggattaaattgtgtatgtgtgaggactaattgccactactggatcctcaaagtggtaagaagtgttcttattaataatgacatccttacactcttacccagcaagattgatgggtgtggcactgcttctctttttccatcacatggtttccatggtatccttttgcccagggaatctttgctttgtggctagcactttgttgtttggctaatcacgctttctgtggtcaggacgctggcttctctggagccatgggattctagctccctgtcttgtccctagagtggtcactgtcttctctctccgcttgcaattcctgctttgctcgcatctcacttatgcagtgacgtatatcagtttcaccttgttctccgtgcctgctgatcattggcaccacttgcatggtgccatttagggcctgcttccagttaagcttgcttctccacaggcctaaatatccttgcttgcttcttttattctcactggcaggaccagggcggtctgtctttgcatgagacagggtctcgctcagtcacccaggctggagtgcagtggctgatcacggctcattgcagccttgagctaccgggctcaagctatcctcctggcttggccccttgagtagctgggactacaggcgtgcaccaccatgcccagctaatttttaaaattatttgtagagatgggatctcgccaggttgcccaggctggtcttgaacgcctgggctcaagtgatcctccctccttggtttcccaaagtgctgggatcacaggtgtgagccactgtgcctggcccttgatgtttcagttcttgatatttgatcctcagagtcagaaaatctaaaaagagggctatcccaggttgccttggttcatggcaaatgggacgttaagagggcagagagaatatgaacagaaactgttctaatattggtcatttaatgtgtaagtattgttcttttttaaacctccttcattttttttccaggaattgctggacacagtggcttggtgtgtgtctgaggactgtaggccatggccctaggttgtggttttaggtctcaggtgctcttcctggctgtctccttgcttctttcccatgtcctcttctttgtttccagccatttctcccttatgcttaagtttggtgcagcagggtttggctgctctcagattcctgcttcctcagatgctgtagttgtcaggcccagcgggctggcagcgggatcaggatctggctaggtttgctctcactgtggcagagtagggggaggcgtgggagagcacgtgtgaccccaggccagctgtagggagcataggcatggtcacgtagccttcaggtcctagactttgtcttctcatgagtatggctgtgtgtgtatggtgaaaactaggttctacttagcccaagaaaatgggcacattttgcatgtggtttctgtagagaaatgcactgggtatctgacatagcctggcagcatgcctccctcaggtaggttagtctcaggcggtgaagcacgtgtgtccagcaagaacttcatatgtggcataaagtctccgttctgtgaggtgctggcaaatcaccaccaccgtcaagaggctgaagtgatttttgtctagggaggcaggaaaggcttcctggagtcagcagccagtaggtgaaagagtagattggagaccttcttaatcatcaccgcctcttgtctcaaggggtgccaggaagctgtggaggctgaacccatcttatgctgccagagagtgggacaccatgagggtcaggtcaaggggttgtaccttgtttggtagagaattaggggctcttgaagactttggatgtggtcaggggagtgtatcatttaggaagagtgacccggtgaggacgtggggtagaggaggacaggtgggagggagtccaggtgggagtgagtagacccagcaggagtgcagggcctcgagccaggatggtggcagggctgtgaggagaggcagccacctgtgtgtctgcggaagcaggggcaagagggaagaggccagcagcgtgctgccatcacccagcgactggcgtagattgtgagagaccattccctgctcttaggaggggctgagttttagttttctcttgttatacaataagcttggtatttgtttacaaaacatttgtaaagctaaatcaaggtttgataaggcttctagttttatttaagaagtaatgttgaaataaatgtttgtccaattcgctttgctcatttaaggactttcagtacaaactgcaacaacaggattaggatttaaacgtttctgagatgtttttactcctcagaatttcccagaatgtgatctggttttgattttcaagcttgctgacccaataggttaacccacaagttttacgaagaccatctcagtccacttacatcaactgcccatgccacggttaaagagatcatcgactgatgtttggcacagcttcctccctcttgggtgggcaagcatttggaagagaaggctcctatgggtgagagtggggcaccaaagtcttccctgtcccatcccctagcttgagaagcccttctctaatgtggactttgtgccgttagcatcgttactagcttgaagttgaccatctggacgtactttctggtttagcctcacaagtgagcaaggagggttgagagatgtgctgtgaggaatgtggggccccagctggcagcaggctctgggtcaggggggcagggaccacgggcatacctgacagtgaggaggggccacacctgcagaaaaggatgcaggactccgccttgggaagtgttctaggccagagcgagggtctgtggtttataagtacacccacagtgctcgggaccctgcagatgtccagggtgccgtctgagcccgtatcatccaacagaatgttctgctagtgaagattaaagatttactccaggggctttaggatttattatatatatataaatcctatatatataattttttttttttttttttttgagatggagtttcgctcttgttgcccaggctggagtgcaatggcgtgatcttggctcactgcaacctccgcctcccgggttcaaactattctcctgcctcagcctctcgagtagctgggattacaggcgcccaccaccacacccggctaatttttgtattttttagtagagacggagtttctccatgttggtcaggctggtcttgaactcctgacctcaggtgatctgcccgccttggcctcccaaagtgctgggattacaggcatgagccaccccacctggccaggatttattgtatttgaaccatctaccattttaattttgatgttatgtagtatttgatgataatgaaagttaaattgtttttctttccatttttctgtttaagtgaatgacctgtatctagtttattcagtaacttcctgcatatatttgtttctttcattcttaatgaatatattcttaatttagttgctattatgttttgctttgccccaaaattgaaatcttagtttccttttagctcgttttagaactagtgatgggatgtgtcttccataaatctcttgtgatttgttgtaggctttgatggattctaatcttccaaggttacagctcgagctctataaggaaattaaaaaggtgggccttgcttttcttttttaaaaatgttttaaattttaaatttttataggtacacgtattttgtaggtacatgtaaatgtatatatttatggggtacatgagatattttgatacaggtatacaatacataataatcacaccatggaaagttggatatccatgccctcaagcatttatcctttgtgttacaaacaatccagttacatgctttacttattttattttatttttgagacagagtcttgctttcacccatgctagagtacagtggcatgaccttggctcactgcaacctccgcctcccgggttcaaccgaactttgggctggtctcaaactcctgacctcaggtgatccgcccgcctcggcctcccaaagtgttgggattacaggcgtgagccactgtgccgggcctgattgtacattttaaaataactaaaacagtcagggcacagtggctcatgcctgtaatcccagcattttgggaggctgaggcaggtgatcacctgagatcaggagttcgagaccagcctggccaacatggagaaaccctgtctctactaaaaatacaaaaattagccaagtgtggtggcgggcgcctgtaatcctggctactcgggaggctgaggtaggggaatcgcttgaacctgggggtggaggttgcagtgagccgagatcacgccactgcattccagcctgagcgacagagtgagactttgtctcaaaaaataaaaatgaaataaaattgggccgggtgtggtggctcacaccttagtcccagcactttgggaacctgaggcaggtggatgcttgagaccaggagtttgagaccagcatgggcaacatggcaaaacgctgtctgtacagaaattagctgggtgtggtggtgcacaactatagtctcagctacttgggagattgaggtgggaggattaattgagcctggaaggttgaatctataggtagctgagattgtgccactgcccttcagcctgggcgaccaagtgagaccctgtctcaaaagaaaaacaaaaaaacaaaaaacaaaccactattatcgactatatattattgtctatgatccctctgctgtgctgtcgaataccaggtcttgggcccttatttccatcactgagcaaacttcactctgttaagcagcaggtgtgggatttcatcgttattcagtaattcacaatgttagaaggaaatgctgtttggtagacgattgctttacttttcttcaaaaggttactctttattagatgagatgagaattaaaaatggtaacttactttatatctttataattgaagcccactagaccttaaagtagttaccagatgttttatgcatttaaatggccttttctctaaaattagaaagtaacaaggaaagaaaatgcttcgtttctatgcaaccctcttggtgactagtatgtgactcttaatgcaaccctcattgcaccccctcagaatggtgcccctcggagtttgcgtgctgccctgtggaggtttgctgagctggctcacctggttcggcctcagaaatgcaggtaagttgtacactctggatgttggtttttgtcgggggccagctgctactgatcctttatgtctcagctcagatgtcatttcaaaagtctgctctgccctctccaaattgcagtcgaccttgccctgtttatgtttccctcatagcactaatccatgtcagaaattgtcacgtacagtctatctgtgtgcttgtttattttctatcccacccttccgcaagagacttatgggatgtgtgccccaggacagcaggggtcttactgtcttatgctctgttgcagcccagcagcgataacagtgtctgcacatagtacttgcttaaaagatacttgccaaattgttgaaggttgaggtaccaatttcattattgctgactataggagttatagcaaaatatccatttgtctgttacatgagttaaaaatatggttgttgcactgtgaatagtttggtttagtcaaaacagttgtatcttaacggattgagaaacaaaagcaggaccacttttcatcagctccctccttctccttaaccagcaatacatgctgatgctgatatcccatagaccctcagctccatcctgagtcactgggaatgtggtctaaaccctcactattaatatgaactgagtttcaataagaatcttatatgggtcgggcatagtggctcatacctttgatcccagcacttcaggaggccaaggcaggtggattgcttgacccagactaggcaacatggtgaaacgccgcctctacaaaaaatacaaaacttagccaggcatggtggtgcgtgcctgtggtcacagccactcgagaggctgaggtgggaggatcacttgagcctgggaggtggaggtcgtgttgagccaagatcgcaccactgcactccagcctgggcaacagagtgagacctgtctcaaaaaaaccaaaatccagaaaagaacttatatggctgcagaggtataatcactaaggaaatttccttttgtataatcttttttcttttactatcatttaaaaaaatgtgttatatttctgaagcaacacatccaggttctgcacatagcagccaaagtgaccttaaagaatataactgggtcttgtcattcccttatttaaactcttgtacccatttcccagtgccgtttagatagagattccagactcgtcaatggctctgtcacctcagacaccctgcattgactcattagtctgattagagtcaggtttttcttcctcctgatggtttttttttcccccttagttctcagcggaacagtcacttccttagggaggtttccccagccaccctctgaggccgtgcttgttgccagactctgccactagagggcagggctgcaccactcctggcacctcgcacccggcctgccctgtcactctgtgtgttgggtgaattcctgtgatctgtgactcactgctctgtgtcctacacattcggcttttcttctctccccacaaccccattttataattctcctttttcaggaaagctttattcccatttaaaaatttttgtttttaaaatggtattttcttacacttattttctaattaaaaatgagtgttttaagaagtattatgatttactgcaaataatttttaaacccagccttttagatcctctgtgatcataagagaaatgaaggatgtctcccaacacttgagcttcatccacatttcatcctcctgttctttcagctgagttttccccatcccattagggactgttggaatataaaactggcttttccctaacagggaatgaattgcttctgtttctcctgaaggagagctggaagaatgacttgcgttcttttgcatacacaggccttacctggtgaaccttctgccgtgcctgactcgaacaagcaagagacccgaagaatcagtccaggagaccttggctgcagctgttcccaaaattatggcttcttttggcaattttgcaaatgacaatgaaattaaggtatgattgttgcctcaggtcacaaacatgcgagtgatgctgtgagtgagtctgtggagggtgagggcttctgaacagggagtcctgtgggagtgcttcttggggtatgttgtatgtcgtaatttagactaccatcatttgtgttatttttgaggcacctaaggacttctttccacttctcatttcttactgtggggtgaagagttgaattgggagatggtttctagatgcaaattgaaaaggcatttttccagagcagatttgttttcggcgtactagagtgactctttaacctagctgcgggaagatgactgtgccaagactgcaggtaggagaaagctcactgacgaggccttgtgggtctgaacgtcctgcagctatcagagcctgttggcttcctgttgtgcattccaacaaatcatcttcaaacccactttagtgttttgtttataatgtccagaaatagtgaccctgtcacatgctctacagattacaggattcttagcctcttcctttttggtaggtcagtcctgggtttgagcccaagtgaccctcctgggaggtgatgatacacactgggtagagtggaatcagatggacttggattagaattctgtcctctttactagttattttcctctaggcaaactgcccaacagctctaagctatttccttcgtattctgaaaaataagccttaatgggacccatatagggcaactctgagagtaaaataaaggaatatgtgttagagtgtagcatagtcacccacgggaagggcttagatgttagctgctactgctcttattagctgaatgatttggaataaactgttagcctctctcatgttttttctcttgagcttcgaagttttcttgttaatactaaggagatattcaaactagtcatggggttttggaatgacgaagggagatgatgaatctaaagaatttagtgtaatatttcttcatgctcagtaaatggtagtttctgctgctgttatttttattaccatctctttggaatgggagtaggtgctcctttgtggtcagaggctgtgagagctccacagcgccagtttgcccatctgtacactggggtctgttgaaggcagtcccctctgtgatatctctggctgtcagagctcagatgatagatggtatttttgtactcttagttctcatcattttcatgatttcgatcaccatttgagtatgatgatgctaacactttgttgaacgtagaatccgttaattacttccttcctgaacctttggcattaaaaaaaatctattctgctacctctctgctcatttatggttattcaaatttattatcaagagcctggtacagtggcttgtgcctataattgtagctacttgggaggctgaggtaggaggattgcttgaggccaggagtttgagaccagcctgggcaagatagtgagaccctatctctaaaaaaactgaaaaaaaattagctggacatgatggcatgtgcctgtggtcctagctactcaggaggctgagacaggaggctcggttgagcccaggagttggagttcgaggctacactgagctgtgattgtgccaccacactccagcatgggtggtaaaacaagatgccatttcttaaaaaaaaaaaatatatatatatatattatcaatgaaattcagtagtaccaacaggattataaacaaagatagtagttcccttcctactttttctcttaatccttgtgtctcacaggcaaacataactcttagtatttcttccaatatttactttcatgtttctttctttctttctttttttttctttgagatggagttttgctcttgttgccaaggctggagtgcaatgacgcaatcttggctcaccacaacctctgtctcccgggttcaagcgattctcctgcctcagcctcctagtagctgggattacaggcatgcatcaccacgctcggctaattttgtacttttagtagagatggggtttctccgggttggtcaggctggtctcgaactcctgacctcaggtgatcctcccacctcagcctcccaaagtgctgggattacaggcgtgagccactgcgcccagcaacttccacatttctaaataacatgcttctactgctattttttttttcaattttagacatttttttactttcactatagttctatcagaattcagtgtgtacgttattatgcctaagtaaatagtcatggttgcttacgtattatatttctttgattgtgtttcttatttgatgagaaagctgtgttttttgctctgggttgaaactggagagaggacctggggaggaggaggaggacagatgaagttggtgactgtaccttcatggccatagctgggttctcagcacccggggatctgctgatcacctactcataggccaggcccctatcgaagttctaggtgacccagtgctggggacgggggggccacctgcaaggtctaatcatggaggtgggggctacagtgttggcttgtgctggggccagcatccttaggaaggcatcttggaggtggaggagacagccgcccacttcttgattggggccttcagcagcaccagcttcttgggcaggctggtgctggctttcatcaccatgtcgtgttcaatcttcttccagatcctgacttctaggttcagctttcctcagaccctggttcctttcagaggccattgctgctgccttgctctttgctggcttgtgccttgattatatgtctttgtacaactttttgttttcctggagttaatcttcacatctgttttcttggagttaatcgttacctctatatcgcttgcttattattctttggcctttttgtcttctcacaccttccaacttctttgtaatatgtgtttagtacaatttttcatgacaggtagtttactgaatcagtttttccccagtgtggtcatccaacttgagttatccagctctctgccccagtctgggcaggttgatcttcaggtctgtagtacacttgtatcctaggacttctctttgccattagcctggaatttcctttgcagttctcccgttggatgcccagttcctagatgccatatgtttttctatcgtctagtagcttcctgagagaagatgaatgggagggaaattgtatgaggttttgcattcataaaaatgccattttttttcctgtacacttggctgggtatggtgttctggggtagaaatcattttccctcagaaatgcaaagtctttgccctgttgtcttaaaatctccaacgtgacccgattccttaacctatgaatgtacttttctttggaagctttccatttttggggaggtgaagtgctaggtacttagtaggccttttaatttggaaacttacatcccttcagttctgggaaaattttcttaacatttctctgagaagttcttgccttttattttctgtgttctctcctgaaattggttagttggatgttggtcctcctagattgactcacatcttacctttttcttttctttttctggtactttttagatatccatctcaaactcttctattcattgttatgtttttaacttctttcttttctttgtctcttgatggggtcttgccctgttgcccaggttgtggtgcagtggtgcgatcatagctcactgcagcctcaaattcctgggctcaagcagctgttctgcctcaccctcccaagtagttgggactacaggtatgcaccaccacgtccagctattttctttacttttttttttttttttttgagatggagtcctactctgtcgcccaggctagagtgcggtggtgggattttggctcacttaagcctctgcctcccaggttcaagcagttctcctgcctcagcctctcaagtagctgggattacaggtgtgcaccaccatgcccggctaatttttgtatttttagtagagccagagtttcaccatgttggccaggctggtctcgaacgcctgacctcaggtgatccgcctgccttggcctccgaaagtgccgggattacaggcgtgagcccatcattagatctttaaataccagtatctataagtcttttcctcttgagtcagctagtatccctggaaggaaattactcattttcctgcttggaggctataagcttggctatgtttatcctgcaaccggggactggaagggaggggactgacagtgttgctggtcagggtgccctcttactttttgttttctgtgtgcatctcacgtctgtcctcagcctatgtaaacacctcttgagattatccctctcaatctttgccggaggtgggggaggggctgcttcctgggctgccttggattggagggaagacctcaggtgagtgggtgggaatttgcccaaggagccatgagaccagccactatttcaccctctccatccctccactttcagatgtatgtggcgcctccaaagcccgagctcttcttggcgtctgtggcttcaataagcttgctttttgctggtatccctcctaccctcccctgtccccagcaaagcttgcatttgaacttcttcctacgggctaacaaatcagtcagttatgtagctcttgttactttttagcttccgaagttttgttgacacccgtagtctgctaatgtccctgttctgttctttctgttcgtgtaaatatatgctttatacaacttctttacatgatttttgtggggtttctgggtagcagagcttcacaagttcaatccagcgtgttggattagaaatctcccaccctctggtttattcttattctcaaaattacctgccaaacactgatactcccttgtttttccttttcctgacaggaaatgtacataccatacaggacagaaatcattagtgtatcccttggtgaataaccacaaagtgaacttaacccttgtaaccgccacccaggtcaagacagaatattaccaagcactcagaagcctctcccctattcccccgtcactgctcctgccttcctccccaaggtcatgactgctggcttctaattccagagtctgtttttaaattctgtgtacatagaccatggattaagtgttctttttgtctggtttattttggtcgacattaagttcatgagagtcttctatattatcgtgtgtattagtattcctgtagttttaggagcttcatagcattccattgtagggatataccacagtttattcattgtattatcactgggttgtttctagttcttggctattgcgagcagtgctactgtgaccactcttaggtgtgtcttttggagtacatgtgcaggtttccatcttgcacagctagaggtggagttgttgggtgatagggtgtgtgcatctcagctgcagtagaaactgccaaatagctttccttgagtgcttgtaccagctcacccttttgccactgtgtatggggattccaggagctctggtcctcgctagcacttggaattgctgatgcttttactcttagccttcctgatgggtgttttctggaatcacattatgattttaatttccattccttaaagtacccttggctctgaagtttaatgattcatgcatctcttcccttttgaagtactcttacaggtatgttgtgcatgtgttgaaaagtggcactatctattctaaaatacagtatgcctcctctgtgtttgaacagttgtagcgtggccttggggcctcctgttagctggcttggagaagggattcttgggattgtagagattagacctgaggaggccccttggagctctctgactaaattttattctttattattccaaactatttaagctcaccgtgtgctgactcatcataataatgagtagctctcattgtgcttgtctatttggactcatacaatgattttttttttttctttgagacagagtcttgctctgttgcctaggctggagtgcagtggcacaatctcggctcactgcagcctccacctcccaggttcaagtgattcttgtgcctcagcttctcaagtagctgagactgcaggtgcgtaccaccatgcctggctaatgtttgtatttttagtagagacggggtttcaccatgttggccaggttggtctcaaactcctgacctcaagtgatctgccttcttcagcctcccaaagtgctgggattacaggtgtgagccactgagcttggccaaagtagttttttaagatgttagtatcttttcttgcagctaaaaaagtttgtcagagatgattctactttgttctccaggtgttttctcagggagaaattggaggcagtaagccactgggggagtcctgtggctggggggtggggtagtcctgtggctccttgtcagggagtcctgtggctggcaaggagagaagtcctgtggctgggttgggagggagtcctgtggctggggtctcatcctgtgcctaacagtgtccagaggtgccgagaccagctcagtcggggagaccctaacccagcagcgctagaggaattaaagacacacacacagaaatatagaggtgtgaagtgggaaatcaggggtctcacagcctttagagctgagagccctgaacagagatttacccacatatttattaatagcaaaccagtcattagcattgtttctatagatgttaaattaactaaaagtatcccttatgggaaacgaggggatgggccgaattaaaagaagaggttgggctagttaaccgcagcaggagcatgtccttaaggcacagatcgctcatgctattgtttgtggcttaagaatgcctttaagcggttttccaccctgggtgggccaggtgttccttgccctcattcctgtcaacccacaaccttccagtgtgggcattagggccattatgaacatgttacagtgcttcagagattttgtttatggccagttttggggccagtttatggccagattttggggggcctgctcccaatacagaggtctcgtgtaaattccctgggaggcgataagcctctgagaaacagactatgctaaccacgccatgaaagagaaacttatttataaatcagatgccagttactagtttactgcttatttgcccaggcgtagctctgacagagtccccgactcatagtgcttgctcagtgcatgctgaacaatgattggaatcaagtcatggctcagagcatagttttgaataatgggaaatggatgttcttaagtaacatagtcaccaagataatgcgactagctgggtcaccccttttcaattttaggatatttttatcaagatttaaatggccatcattagagttatagcactttctcctttggattgtcctagaggcccatgagaaagtattccctaatttcttaggagaacagtttgtgggtagtatgcggtcatgtccagttaaattgcagatatttccgatcgaagatgttccagtcctgagaacttcgtgacattagcaggacttctacaagccatctcttagggtggggcatttactgcagttggctagtactcttttctccttaactttgtcatttgttgatttttttttaactgtccccaaatactgtgggcagagtgtatctagaattgaggcctccaccattgcggagaggacatggatgctgagcagtcccctgagtgaaggttataaagaagcaaatagactacacatgtctgtaaactgctcttgagtgtcccaaatttggggtacttcagttcagctgtaggaaaagcctcaaactgtttatactttgcaagaattggaaacttctaattcacgttaagttttatgtaatacatgataagcttcataggagcttcatcttttatctacttggacttttgcttccgtaggttttgttaaaggccttcatagcgaacctgaagtcaagctcccccaccattcggcggacagcggctggatcagcagtgagcatctgccagcactcaagaaggacacaatatttctatagttggctactaaatgtgctcttaggtaaggtggaggcatatgagtggaagagtctccagcatgtactcaagatagacctttgaaataaataaaaccagatgatccctcagcttctagaccaggctatttggcactggttgattgaatgtgaactgcactggggctgctgtgagcccgcatgggtctctgtgaccctgcagatgcagccgtgcccagggactgggcagtgggtgtgggctggtgtgagccctgtctgccacccagggcctggccctctgtctgtgtcggccatgactatggtgagtcttgtaggcttgagactgtgcctcgggttcctgcgggttctctgtaggtcagttgacagtttctcctgttgtttgggtaactgtggaaacgaacactggcaagtgctgaagcgagcatgtggacgtgcgatatgaaataacgacctggctttcaaaggcagtgaggctctctggaaaggaccttgctgagctagggatgtgggtgtgtagccattcccagtgggcctcatggcgtactcgttcatgatcatgtttgtgccatcttgatctctcaggatctcttcttttttaacagattaagccgggaatctccaaacagtgagtcagatgttaagatgtcttgcttccacccccacaggcttactcgttcctgtcgaggatgaacactccactctgctgattcttggcgtgctgctcaccctgaggtatttggtgcccttgctgcagcagcaggtcaaggacacaagcctgaaaggcagcttcggagtgacaaggaaagaaatggaagtctctccttctgcagagcagcttgtccaggtaggagcacagggtttactctaggccctgcatgtgaatgactgacattcaaagaaccgattaatttggaagagaagcggcagaaccgagagttagaggtgtggactctggagctgcgctgctcgtttccaaccctaggtgctgacctctagctgtcttccctctgtatgtccctgtcaccgtgagtcaaatgcgggtgatgcctcctcaggtgccgtgttacctaagcctctcagagaccactgctaccctgtttctaaaaccagaggtcacgatatgtgttcatccacccagtaaatactgattgagcacccactgtgtgctaggctctgggataggggctgggtatacaatggtgagtatttcagctgcagcttctgccccgtggaggctgtggcctagcacactggtctaggcacggtggtatatgctcactcaaggagatagggacgtggtcgtttggggtgtcggaacaaaatgtcggaacttctctttccaatgcagagaaaccttgcagtaattctaatgtactgtgattggcagttgacttcagttctttgtagcacgcttactcaggttatttcactaactatgtaaccatgcagcctcattttaagcaattggattttttgaactttacttaaaatgttatgtcagggtttttattgtgcttaatgtgtgccatttagctaagttttgtaggatacgaaattgtaagtggcttaaaatgattcttaatagaatcatgaattgaagataatgctaataatttaagcactgagttaggtagtgtttgtaaaatgcttagaatgcttcctggcacatgttaaggccatgtaagtgctgcgtgttgataaacagctgagcaaaagtggactcttaagaaagtattggggctgagagttctgttccaaccagctgccctttggttatttttcagaataaaagcagagtctcatgggatatgacatttatatttccttcacaaaaaacactgctgagtgttttgttgagtaaaaagggtgtagccatggtaataatacatttaaaatatagtttatttcatctttaccttgccttgttttttttttaagctagctttttattgagaattccacacatacaaaagtatcaactcatgaccagttatatttcatttataatcctacttctccctttttttattatttgaaagcaaaccccaattatcctcttatttcatctataagtatttcagtatctctatagatgaggactcttctttatttttaaaactttatttttaaaatgatggtcagatgcagtgttcatgcctgtaatcccagaactttgggaggccaagctgggcggatcacttgaacctgggagtttgagaccagcccgggaaacatggcgaaaccccatgtcttaaagaaaaaaatcagccaagtgtggtgatgcatgcctgtagtcccagctacttgggaggctgagatgggagggtcacatgagcctggaagatcaaggctgcagtgatccatgattgtaccactgcactccatcctgggtgatggagcaagattctgtctcaaaaaaacaaaactgcaaaacaacgtcacaaaacagtgccattgttagacctgaaaatattaaacatttcctacatcaaatacccaccaactcattatcaatttttctctctactcttttggaatcagcatctaaataaaattggtcgataaggattgtaaatctctttgatgaactggttcccctccatcccagtttttttcccttagagttcatttattgagaaaccagattgtttgtcttctaagttttcctgtggtctgatatactgcttccatctccactgtgtaaattaacacctttttctcttctctgtatttcctgtaaatcaataattggaggaaaagccttgtcagatttagtgtatattttatatctgagtccagtatttcttatataatattttaagataagtgtactcttttaaaaagtattgaaactatatgctcaattttttttaactgatgcttttaagaaggctgcttgatcataaaagtttagagatcattggtctgatgggaaaagcaaataattactaaaccgtttagcaaggttgaggtgcacatggtggggcctggagaagttcagtcatgagccgtcacttatgggcacgtggaatctgacccggcacagagttgggagaagacaggagctttatagacagaaaatgtggtctttgctaagtcccaggagtgaaagggtgagacagtgctcacagcacacgagtgtgggtgcgtagacagagcaagggtgggtcctgaaaaggcctgcaggctttctcatagattagcaagagtgctggttacggaggtttctaacatttgtgaacagatcgaaactgtgttaaattgggattgcagtaatcctggaaggacagggatagagggtgaaggggaaaaaagggtatggatgtgagacttaattgctgattttcttaagacctttctccaaagtaaataaatgatgtggcacatttttgaactggcaaattctaaactctagatatgattatctctataacatatcttactccatcttcttttgactaaaaactgttcttaattaaattaccatgagacgttcaattcagcaaatgtagtttggctaaccatatttaattagaatttaatataatcctaggcctggccaaactattaagcaagtgtgggcaaaatattgataattttagatatgcaggaacttagtttgctttccatgtgtgcttttcgaaaaaggaataaattgaaaaatagaggaagccctgaaatccaagaagcaaactctctcacctaggcatgcagtaaaagcaattctaggatgattgctgtttggcgcgtagttcgtattagaaaccattcttcttgaataaatagtatgtttaagaagctgggcagagggaaggcatatgcatatattatcaacaaggagggagaaaaaggcaattagtaaccatccataggagggtcagcaagatttataaaggaaatttgtgatccaagtatgaagcaaaataaggtgcagaataaattttaagcaagtaatagattagagtaagagaacccatttgaccattaaccttgggacattctctttcaaatgacatggagtagtactgaaatctttctttctttctgagtctaggttattgtgactggactcagaaagaaatatttcattattgcagtgaataacatttgtgaacattattgttcataaattatgcagtgaataacatttatgaacacgtgatgtgtaagatacatactgtttatttttagttaagttttttggctcaacttctaggcagagaacattaaatgtaaatagtgttacctaggagcatgtaaatggaaatctccatagtatgaaagcagtgctgttgctaacagaatttaggagggggcagatgaggtgaaggaaatgtgggtgctgatttccttattacattgagaggagccaggagattctttgttcaaaatggatggcttaagaagtcaaagtataagctgattacgtagagcaggtacccaaaaatgttttgtgtaaggggccagatagtaaatattttcagtcttgcaggccatcccaagtctgtggcagctactcaacactacctttgtagcatgaaagcagccacaggcagcccataaatgtggctctgttccggtgaaactttaggtacaaaagcaggtgcaggccagacctgacctgtgcactgtggtttgctgacctgggattcaggggtatagaagttaccatcagaagagctaaaagtgagactttttactttatactcttctacactgtctgattttgaaaaaaagaaacatgtattttataatattaaagatagggttggcaaatagcaaataaaaatacagaataccagtgaaatttgaacttcagatacattatgagtaattttatggtgtaagtatattccaaatcatgtgggacatacttacactacaaaattatttgttgtttgtttacagtttaaatttgagtgccttgtattttatctggcaactgtaattaaagggaaaaagaataaattcattatgttcatataatgtgatatagcaggggtccccaacccccaggctgcagagtggtactggtccatgggtccccaacccccaggctgcagagcggtattggtccatggcctgttaggaaccaggctgcccagcaggaagtgagcagcaggtgagctggcattcccacctgagcaccgcctcctgtcagatcagtggcagcattagattcccataggagtgcaaaccctattgtgaactgcacatgtgaggggtctaggttgtgcgctccttatgagaatctaatgcctgatgatctgaggtggaacagtctcgtcttgaaaccatcccctggccctgtggaaaaattgtctcccatgaaaccagtctctggtgccagaaaggttgggtagcactgtgatatagtattaaaagtgctaataaatatggcatactgcctttaaaatgtctggtagctctttctcagtggcactcataatagtgttttttgatttttaaatgtgtgtcaagctgactctcccctccgtgtatgctgggctttattttccctttcctagtcaccagttttgggaaatagagatcttcattctcatgctgctcctctagtgcaagtgctccatttatttttaaggaattaatataacaaaaaatcatgggaatttagaaaacaacatggaagctaatgatcacattggtggaagtgatagggaaatatttagggggagaagttaaggtataaactttgtcaatgaagtcctattaaaaacaacaaaaaagtgaagcttaggatgcattttataaactctgaccagaacacctgtgtttctctgtttctaggtttatgaactgacgttacatcatacacagcaccaagaccacaatgttgtgaccggagccctggagctgttgcagcagctcttcagaacgcctccacccgagcttctgcaaaccctgaccgcagtcgggggcattgggcagctcaccgctgctaaggaggagtctggtggccgaagccgtagtgggagtattgtggaacttataggcaagttattagcaaggtctactcttacaattaactttgcagtaatactagttacactctattgattatgggcctgccctgtgctaagcagtctgcattccatcttccttgccaaaacttataatacaaatttcatctttattttataaataggggagttgggctgggtgtggtggctcacgcctgtaatttcagcactttggaaggatcgcttcagcccaggagtttgagacaacctggccaagtgagaccctgtctctacaaaaaaaaaaaaaaaaaaaaaattagctgggcatggtggcacatgcctgtagtcccagctgctttggaggctgaggtggtaggattgcttaagcccaagaggttgaggctgcagtgaatcttgatggcagctgcactgagcctggtgacagagcaagatgctgtctcaaaataaatttaaaaataaaataagagaattaaagtttagcaggttgggtggcaaaatgaggccacacatttaaagcccctcctcctgattcttttctctgccttggctgcctcctgtggcattttaggtgctgagaaatgaaaacagtagggaaaatagttccaggatcctcatgttaatttgccagaaatggcatcttcaagtcgtcagagggatctgagagttccttcctggcctgacttgagaaaatccgtctgtccccagctctgcgtctgcctccactgcccagtcacctcctctccatgctcttggggctgggccctaccccaccatgcagtgctgccctggagcagtgagcttggtgggtcctgtctggcatgagagctgcctttgggagctggatcccagcctctaccactgggtctggtgcctagcaggctatggataaacttctgctgactccggcctctcctaagccactgcaacgtggtcggtgtagtgcacagtgtgtgtgcagcgtggccttactcacagcctccacattagagagaatctgactgaagtcttactgctgcctcgtgtgaacataaatgtttgccagaaccatgagcaggaaatgttaatctgccttgtttcctgtcctttacacggaagaatttttttctgtatggaatgcgtgccttacaaataatgagtggaaatacccatcgctaatgaaaagttatacttgactgttagtcagctaaataatctgagatttctaatacttttaatttggcttttacaatgcaatttatcttagcttttttgatttcttaggtcatatctttagaactatatatttgaatgttaatgtaattttcatattgaaattaaaatgttgaactgcgatgttaagtgtttcctgtggaaaaacgttcacattttctctagttttaaagttgaatcaagctgtttgaagattttcacatttcttctagattttatcagcttgttactttatctgtcactttctgtgatttgcagctggagggggttcctcatgcagccctgtcctttcaagaaaacaaaaaggtgattatttcagaaatcagagtcttgtgttgaatcttactgattttcttgtatttctgtaatgtaatgtatcttgtatttcttgtaatactgtattggactctgtgtatatctcttctcagatgagtgattatatgtgtgaatgttgctggaatctgataaccaggcctgaatagttttgtagggtggcttttaaaaattactttcatatcagaattgctttgtcataaattttgaacgcatcataaatttctaatgttcggggtcagcagactttttttgtaaagggacagagtgtaaacatcttagctttatgggccatatggtctcttttgcaacattcagctctgccctgtgacaggaatgcagttgtaaagacatgagctactggccagctatgttccagtagaactttacttacagaaacagacaggctgtagtttgccaatacctgccttagggaatgtgttgttatattttgtgagttaccttctcagtaaattttatttagtattagtcaggaatattattaagtagcttcttttccagcctggtcaacatagtgagacccggtctctaccaaaacaaaacaaaacaaaaaaacagccacgcatgtggcatgtgcctgtagcctcagctgctgctcagggggctgaggcaagaggattgtttgagcccaggagtttgaggtcacagtgagctgtagtcatgccactgcactccagcctaggcaacagaatgagaccttgtgtcttaaaaaaaaaaagtttcctttgttgggttattttaatttggacctggttatcatttttcagccatatttaactttgtacatatcagaatgttctgataaaacttaacttttattaaagtgtttgtgatataatctgctagttttggtacacattatcttttgcaatgccagttattttcttttccagtgtgggtttgcataggaaaagaattgctgtcactttctattttgaaatcttaaaagactgatccttttttgtgtcatgatttgagtatttaattgagagcctaatgcctaatattatttgcagtattaaatgggatcttaacaggaatagcattctagccttcattgaattaagtaaacatttcttaagagaacttggaatctataatatttgcgtcatcatagtatgagatacttaatcaagtttgagattttagtgaaacattgtttagaagccaaaaggattctaggaaaaattaatgtctatattcttgaattaggagagattttgggacgtgtgactaagttacgctgacacttgtttgtttcttagtcgctttttccagtggcggtgagaacgaagatgactgattcacattgctcagatgagtttatcctcttctggctgggacatgggatatatcctgtctcttttaagcctttttggtatttttcccccattgagagctgtgtcttcaaactcttctgttatagctggaaaatcctttttaagtgaaatctgcccaaattataagacagatgaaggtagagttgtgttggatataggattagggtgaaagtagtgggggtgtcctggagcctctcttctggtggcagcctagctcttgtgcctttgaggaaattaccctggggacggctctgtggaacatatttgcaaaccactgatttggaagatagagatggcttttgttaagatctgaattcacctttttggcattttatttgatttctcaaggtaaagaacttattttgtaataaagtttcctattatttagtagataggccaagttgctgtgttaattccatgtagattttgggtttcctttgctcattttttcactcttaatctcacatcattgtaagtttatggaagttatcatacttctgactttttctttgaagagcagaaattagaaattcccaataattattttgatagtgtcatttaatgacactcacatgtgatgtagccacaaagatttaatgagttcagttttaaatcatattaagactgttggtttcatttgttctcattaatgtaattctgaagatgaacaataaaatgtatttttagaactttcaaatgaaatattatttcatccttccagatcatataatgcttaagttctgattgttaatcataaagtctagaaaattaaaagataataaaatgaaagtgacttttaggtattagagttttattataaattctggtgtgtcattggagctatgacatgaatatttcaaaggccaatagcattggatctttacagttataacttaccatttttaagtttaagtagtaatatagattatttaataatcaaaatcaataaatattaattattaaaatgttttgtggtatagtttgagaatcattgcttttaactttttccatataggtttattgactttaatagcattctaaacataacatctctacattctttgtgtttaatactgtggaggtataaaaatacttatatatgatgataaactatattagagtaaattaaatattcttatgagtttcattttagagtgcatttacttaattttgaagtccttatttttagcaaactaaaaggaatgttggtacattatttactaggcaaagtgctcttaggagaagaagaagccttggaggatgactctgaatcgagatcggatgtcagcagctctgccttaacaggtagttctcactagttagccgctggtgtggaccttcactgtctgccttccaccccttgcccttcctgctcgtccccctgcacctggtggacagcacgactgggggcagcagtggagccaggttgcttaaatggggcatattcgggcttcttttataatacttactctgaagcttgtgtgtctgtggtgtttgcatcatatatttgttgttttccatggtttaggctgttttaaaattaggtttatggcttgagcatagggctttgtgagtaggggatggcaggtcgaaacatctcatgagttggatgggttatgctgggggttgggaaatgggatgaaaaattatgggatgaaaaattgcctatggatagtttaacttgaaagaatctgcctttgtttacagatagttatcttttttcttttttgagatagagtctcacactgtcacccagtgcagatacccagtgtcactggagtgcagtggtgtgctcttggtgcactgcagcctccgccttctgggttccagcgattctcctgcctcagcctcccaagtagctgggactacaggtgcccgccaccacgcttggctaatttttgtatttttttgtggagacgggtttttgccatgttggtcaggctggtcttgaactcctgacctcaagtgatctgcctgcctcagcctcccacagtgccgggattacaggagtgagccactgtgcccggccagttacagatacttatctaatgaaattctctgtgtactttataaaagatgaggattaactgaaggtactaataactggattatatgagggtggttttggttgtataatcctatctaaaagaatattttagctataactgaaagtaagacttaaatatttagagaggaaaatctgaataattctagtagtaattatttatttacaaaataaaaatagatttttttttgattacacaaattaaacaacaataaaacatcacagcaatccggatactataaagctcacatgcttaccgacccaactgccccaggagtgaccactgccaacagcttcatgtcgacctttttgccataatttttatatagccttttttgtttttaaatggtaatttagaaagtcaactaggaaaatgtgttacaggtttatcttccaggagaataggactggagtcgagatcttgaatgtggcttggaagaaggcaagcccaccccagagagatgagttgacagttgtttctgaccactgcttgcttagagggcctgcgtgtctgtgaccgcctagctttgcgcccctgactaggctgccccttaattacaaatgtctttatatattgctccagctaaggcttggagtagtcggttaagaacttgaacttcggtttttgcagtgaaacagcatttgagaatatcaccttctgataagccttattttataaggtgggtactgtagtgggaggcagtgtgagagatgcttgaaggatgcactgctgtcctgcatttcagcatcttcaggatgctgtgcagctgaaacatttgataacggtggaactgttcgttattttgcaagcctgtgattccctattgaatgttttctctcgccatttgacaaatgagtgtttctctgtcttcagcctcagtgaaggatgagatcagtggagagctggctgcttcttcaggggtttccactccagggtcagcaggtcatgacatcatcacagaacagccacggtcacagcacacactgcaggcggactcagtggatctggccagctgtgacttgacaagctctgccactgatggggatgaggaggatatcttgagccacagctccagccaggtcagcgccgtcccatctgaccctgccatggacctgaatgatgggacccaggcctcgtcgcccatcagcgacagctcccagaccaccaccgaagggcctgattcagctgttaccccttcagacagttctgaaattgtaagtgggcagaggggcctgacatctttttttttattttttatttgagacagagtctcactccatagtgcagtggaggccgggcacaggggctcatgcctgtaatcccagcactttgggagactgaggcaggcggatcacttgaggtcaggagttcgagaccagcctggccaacatggtgaaaccctgtctctactaaaaatacaaaaattagttgggcgtggtggcacatgtctgtagtcccagctgttagggaggctgaggcaggagaattgcttgagcctgggaggcagaggttgcaatgagccgagatcgtgacactgcactccagcccgggcaacagagcaagactccatttcaaaaaaaataaaaaaataaagtgcagtggctcgttctcagcccactgcaacttctgcctcccaggctcgagcgattctcccgcctcagcctcctgagtaggtgggattacaggtgggcaccaccacactcagctaatgtttgtattttcagtagagacagggtttcaccatgttggccaggctggtctcaaactcctgaccttagatgatccacccaccttggcctcctaaagtattgggattatagttgtgagccaccatgcccggccctgccacctgccatcttttgagttcttccctggagacctagacctgaaccctcctgcttgttctcttgttatctaatacccctattgacagcgcagcttagatcattaatggagagcttgacctcatctgataccttcactgaaggaaacaacttagtgtcttttgtgttgaacactgaggtaaaaaattggaatagttgattatatgaactctgctaaaattgagtgcattttacattttttaaggccttgttgggccctggttaaataattatttttaaaaatccttaaggagcctattataaacagatctgtggtcttaatgaaatgtgattaatactgtgcattattttaagaacttttgacttttcaaaaaacttttacaacatttcccatttgatagcggcataggtttaagcacttctcatctctaagttagtggacaaaaaaccctcatggatagtctaataatgtttgctacaagtccatgttgagttttatactccattttattttcagttttaaaaactgtggttaaatatgtgtaacataaaatttatgttcttaaccattttttgcgtatacagttcgctggtattaaatacatttaaataatgtcatggaatcattgctaccacccatctctgtaaccttttgatcatgtaacactgaagctctgttcccattgaactctattcctcctttcccgccaagtccctggcaaccacgattcttctttctgtcttctgaatttgactactttgggttctcatatactttaggagtcacacagtatttgttttacttagcataatgtccccaaagctcatgcatgttgtagcctatgttagaacttcctaatgtttcaggccaaatactattccattgtatggataggccacattttgcttttccattcctctgtccatggacacttgtattgcttcatgttttagccattgtgaatcatgctgttatgaacgtgggtgtacagatagctcctggagactctgctttccatttttttggctaaatacccagaaatggagttgcttttacattccaattttaatttaaaacattcatatcattgagtgttttacttaatagtatagtagttaacaaacttaataaaatagtattttggtaataatttgctggtagtccattgttcagtttttttaggtaaattacacaggacatttcaagtggacatgaaacatcttgtgatgtggaatcatgccccaagctgatggctaaacatatgaaataccataccctaaatttagtagatttagtctttgcaatttaggagataacctgttatattgttaggtttttgtcgaaaagctttgtcctcatatttccaacttgctgtaaaatttgtttgtgaagacaaatatttttgtatgggttttttctttttcatattaaaaagaaatgtccacattggaatttttttggagtttttagagctaatagagcttttcataatgtagtgggaatgagtgatcagtaagctcttagcagtttccatgcgtgcatttctgtgccttgaaataaatgacagatgagtacatttgtgttctgtgtgtaaaatgtgctctttcctcattgcacttccatgttggagggcttgtctcttggtgatcacacttcaaaattctcacagccccccttgaaccgtttaggtgttagacggtaccgacaaccagtatttgggcctgcagattggacagccccaggatgaagatgaggaagccacaggtattcttcctgatgaagcctcggaggccttcaggaactcttccatgggtatgtggactacaggtgatgcgctacaaagtggtttgtattcagacctggacatcttaattatatctttgcttccaagaagaagtcctttgatactgttttctgagttctgaatagctgatgaaaatgaccaattgaggaataatcatactttttcttgatctaaatcttatacttttgagttatcttagcataaatgtataattgtattttaagtggaaatttgtcacttaatcttgatttctctgtttttaaagcccttcaacaggcacatttattgaaaaacatgagtcactgcaggcagccttctgacagcagtgttgataaatttgtgttgagagatgaagctactgaaccgggtgatcaagaaaacaaggtgagggacataggcttgagacgacttggtgtttctgagcttgtgtgaggatttaaaatcgccctggctactgtctactttattgctttcccatccctgggcctttaaatttcccctttaaataccagctcttcccaggcctgttgttttctgcctttccaggtactacccacagccttgagaattgcctgagttctgcctcctttgagagtgtgccccagacaaatctattctgtactgaatgtttccttgtctgatttcttggatcattcatttgatggttgcgtatggcctgcaacgtttcttgttttggttctactgaactgttctaaaagtctctcttcatattatctttttacatgtaaatgtaactgtcttcacttttaattcctcaaggacaaggaatagcgtttcacagttcgtcccatcaatcagaattatagcctttggcatctccctatctaccaggcccacttcctcttagatttgggcttccccaggctgttgcctttccccaagtagcttctgcttgtcctgtagaagacctttcatgctttgcttctgcagcagccgttcctgaatgcctagtgtcaactgccttcttaccacgcccaccctccctgcatgctgcatttatcccctgccacagccctgtgaccctgtgtcctgctgcctctgacttgtctgtttctgcttggccatggtctctgtgaggtcaggtgtgcatatgggcacaaaccagggcatctctttatccccagcacctggcttaagtgctgctctggaactatctgttgaatgaactaatgcatgaatgtattgttgagtatgagacaaacaagtgtcattgtctcctttctagccttgccgcatcaaaggtgacattggacagtccactgatgatgactctgcacctcttgtccattgtgtccgccttttatctgcttcgtttttgctaacagggggaaaaaatggtgagtacaaaaggggatgtgcacagttgaaggaaataactaggtttcagaggtcagcttggtggcctgtttttgccttgcgtgcagcagaggaagtagaatctgaggatgagtttggttttcactagccgaggggagggaggaaatgatgggagcaggtaggttattgggtctggttttgttcatttgaaaacaatctgttgtttgaggctgaaggtggcttgggtgatttcttggcagtgctggttccggacagggatgtgagggtcagcgtgaaggccctggccctcagctgtgtgggagcagctgtggccctccacccggaatctttcttcagcaaactctataaagttcctcttgacaccacggaataccctggtatgttaaaagttcacatcttattttctcagatttaatcattattgtaaaaactatttcagtattgactattttagttttagagcagtaagtgttttgagttcatttgggatatttgacctgcgttgtagctcttcagaaaacacatgaatagtgaagttctttgtttcatgggttccctttagatgaaacccatagaggagaaaagtagaaacctcagcacgtaagagccaacatatatacacatcggatttaaacctaaagcacaaattgtgcctggtcgcagtggcgctgagtcgcactcagccaggccaggcattcacactcagggtgagtgggaaccaggactggctgaggcagcagtggacccaagtctccatcgcgcccatgcttactatggagccttctcgttctctctttttctttgggtgagagggtacacttgtgtttttgaatttatatgaggtaagtgtgtaatagggttttttctaatcttttttaagtggaatctggaattttaatcagatttattatctgacaacctagaattataatccagaaagtctgtggtattgaggacatattggcaatatgatgaatctctaattcttaaatcctgaaacttttttttttttaatcacttagggttattatagtgaagtcatttctgaatttggatcttctcttcacacctctttttctctttcctgagaattaagcttttgtttcgagttagaaagttgatagtagggaattgttccatggctgagcaatttatctccacagaggaacagtatgtctcagacatcttgaactacatcgatcatggagacccacaggttcgaggagccactgccattctctgtgggaccctcatctgctccatcctcagcaggtcccgcttccacgtgggagattggatgggcaccattagaaccctcacaggtaacggccagtttttcagctgtgttttttctagttatgcttactaaggtttaagtttagatgatgatgtttgttgcttgttcttctggttaggaaatacattttctttggcggattgcattcctttgctgcggaaaacactgaaggatgagtcttctgttacttgcaagttagcttgtacagctgtgagggtgagcataatcttctgtggaaccatttcttcacttagtggacattttatcattgctacaattaaaattggagcttaataggaaatatttccatgcactctaaagctgtaaccagtaatacccaccatgtatccatctctcagctttagaaagaaaacgttgccagtaaagttaatgcttcataaacttcagtttaagttctaattctcagaatatttgtttgaaatagacctcttcctaaaggatatatttagaaataacctatcattaagtgtaaagtctgttgaatatgctgggcacggtgactcacacctgtaatctgaccactttgggaggccaaggtggaaggattgcttgagcccaggagttcaagactatgggcaacatagttgaccctgtccctacagaaaattaaaaaaaaaaaaaaaaaaagtagctgggtatggtggtgcatacctgtagtctcagctactcgggaagctgaggtggaggggggattgcttgagccccagagatcaaggctgcagtaaggcgtggttacaccactgccctctagcctgggcaacagagtgagactgtctcaaaaataatagtaataataatcagttgaattaaaaaaaaaaaaaaaaaaaccactgtgctaggcccatagtatggtaagagttaaagtgagccttagggattatttactcaacctctgtttctgtataaagtggaataggctcaattctttaagtgatagcatgttgaacctttccataccaactggctcataagtcacaactggccagtcaacaagagtaaaaattaactggtaaaaatcaaagcaaaaaacctacaattgtcaaatttgtgggataactcccccttttaaaatgtcatgcctgacagtaatttctctctagtttccaggttttcagtcagttgtgtcttttttgagcagaaggaagcatgctaagagctcaatcttgtggctagctgggggtctttgtgtcagccatgcatgtgatggtgcccctgggtgcttggggctgcaggggaggggtacagcagtaggggcctgttctgttctctcgtgctgtggagtacatagtgacatagtggggtggtccttggtgtaggtcccttgttcctacccctgggtctgagatttatttagaagtggtgttggggctgtgcggcaggcccctctgtaactgatcaatgtttgtgaagttgctgtttgagagttgaaaccatgacataagcagaaatggaaggaagaaagaaccagttatgtgaaagggacacatttacttttaagcttgtatttactgagataaagtattcttaatcaatgttcttgagaggtgtgggaaaaatgcaacatcctggttgcagttaaacccagaacattgtgtgttgaagagtgacggttctcaaaccgtcaagacgcgggtactgagtgggactaacctgctgtcctcttgccttggaccttgtgttccagaactgtgtcatgagtctctgcagcagcagctacagtgagttaggactgcagctgatcatcgatgtgctgactctgaggaacagttcctattggctggtgaggacagagcttctggaaacccttgcagagattgacttcaggtaagtgagtcacatccattagatttcatgaactaagctcaattgaaagttctgggatcacttgatgcaaggaatgatgttatcaagtaccctgtccatcagaaatccgagtggtttaggtagatgacagtgattttctcctcccagtggctttttgctgaactttgccctatgcttggaattttattttattttattatttatttagagacaagatcttgctctgtcgcccaggcttgaatgcagtagcacaatcatagctcactgaagctttgaactctaggactcaagtggtcctcctgcctcagcctcccgattagctaggagaataggtgtgtgccgtcacactggctaatattttttgtagaaatggggtcttgctatgttgcccaggctggtctcaaactcctgggcttgattgatcctccatcttggcctcccaaagtgctgggattacaggcatgagccactgtgcctggcctagaattttaaaatataagtagaagagtagatttttttttttggtagtcctcgtcatttaagtattctggatagtgggaataaaagagcttagaatttttcatctttgtcttaaacttttaaaaaaatgtagcttatattaattctgcttgtttaaaaagaatatactcttcattatactgaacctaggtaagacagctggtttatattttgttgcaattaaaaaacgtgagctgtggttgcagtgagccaagattgtggccattgcacttcagcctggcaacagagtgagacttggcctcaaaaaaaaaaaaataacatgagctgtgttggcactttcattttctaagagtagttttggctggagaagttttctttcagtactttcttttagaagggaaattttcctttataatttagggtttgttttttttttttccaagccaccttttatagagcccttgtgggttatttcatttaatccttagaatgtttataaatctgggcttgttctcggctccacccacagatagggacgctgagcgtgcatgagtgggcagcaagatagcaggttatggagggcccagctcaccccttctgtggcttgagccaattttatagggcacttacagagtcttttgaaatagtatttattttgaagaaaaagaaaaacagtttactgagtactgtcttattgagtctggaattgtgagaggaatgccacctctatttatttaaagccattggccttttttgttgttttgagtaagtgctgcccaaggtccttccagggcacctggatgagcctgctctggagcaagctggcggtaagtgtttactgagtaactaaatgatttcattgttaaatgtgctcttttgttaggctggtgagctttttggaggcaaaagcagaaaacttacacagaggggctcatcattatacaggggtaagcggtttatttttgtgagatgctgttttaccttcaagaaggtgaaagtgaggctttccttgtggaatttctctaaatgcattcgtcatgttttagatgtttatttcacagtttatatcatgaaagttataatcttgtcatatggatttaagtctagtaatgttgagttctttctcactagctttccaaaatatcttacctaaaatttagtcaaatacaagattatgtttatttttattatccttctctctaaagcttttaaaactgcaagaacgagtgctcaataatgttgtcatccatttgcttggagatgaagaccccagggtgcgacatgttgccgcagcatcactaattaggtatttaccaatattttatctcttttccttttttggttgaagtactaaaagatacgagaatggaaagagagggaagaattcaaaggatgtagagcagtattcctgaatctgagctcatttcagccattctattcttaaactataatgaaaaaaaaatccaaaaaagtctaaaattataattaaaaaaacaacaaaatactaactgtccattgtaaaaagtaatgcactttcattgtaaaaattttggactatagagaatagtactaagaagaaaaaaaaaatcaccttcaattctgctgccacctggaggtaatcactgttaatattttgctatatactctatgagtttcttgttcaaaatcaggtcaaaattacatgcaattttgtaatctgacaatttccacttaatattttattagcattttcctgttatgaaacagtaattttagttatgggtcgttgttttgctatgcggttgggataaaattttatatactttttttggcaattacttattatacataaatgtttgtgtatagttttctttttctgagaattcctggaagttgagttaccaggcccggctttgaatttttttttttattttttttttgagacagagtcctgctctattgtccaggtgctatctcggctcactgcaacctctgtctccctggttcaagcgattctcctgcctcagcctcccgagtagctgggattacaggggcacaccaccacgcccaattaatttttgtatttttagtagagacagggtttcacgatattggccaggctggtctcgaacttctgaccccgtgatccacctgcattggcctcccaaagtgctgggattacaggcgtgagccatggcgcctggccaggctttaaatttaaaacaaatcttctaatagctttatggaggttataatttacatttcttgaaatgtactcactttgagtgtatagtaaactccaattttatcacatttctgtcaccccaaatgtatccttgtgcccatttgctgtaacctccggttcctgccccaactcctaggcagccactcatctattttctgtcccttaagatttgtgttttcgccaggcgctcatgcctgtaatcccagcactttgggaggccgaggttggtggatcacttgaggtcaggagttcgagaccagcctggccaacatggtgaaaccttgtctctactaaaaatacaaaaattagtcggatgtggtggcacacgcctgtaatcccagctactcgggaggctgaggcaggagaatcacttgaacctgggaggcggaggttgcagtgagcagagatcgcgccactgccttccaacctgggcaacagagagagactgtctcaaaacaaacaaagatttgtattttctggacattttatagtactggggtcatagtatagatggacttttgcatttggcttcttttacttaattgtgagattggttcttgttgtagcatgtatcagtagtttgttcatttttattggcgaaagtattctattatatgaataataccatattttatctatccatcagatggatattatagagttcatgttttggctaatttatgaattatggtactgtgaacatttgcctgcaagattttgtgtagacatgtcttcatttctcttgagtagatcacctagaagtggatttttaaataattttggtacttactgtgaaactgctcttcaaaaacataccattgttccttccttccttccttccttccttccttccttctttccttcctcccttcctccctcccttccctacttccctctccctttccctttcccttccccttttcccttccccttcccgcctgcctgcctgcctgccttccttccttccttccttcgtttctttctacatatacacatttttttaaatttcaatggtttttggggtacaagtggtttttggttacatggctgaattttggttacatggtgaagtctgagattttagtacacctgtcacccgagtagtgtaccttgtacccaatatgtagttttttgtccctcaccttccagccttccgccttgtgagtctccaatgtccattataccacactgtatgcccttgcgtacccacagctcagctcccacttctgagaacatatagcagaaacatgccaaagtatactcccactaccagaatgtgattgtgcctgattcttctcaccagtacaaatatttcaaaaaaagttaaatatgtatcagttttttgggcagaagttgatacttctctttatttatttattttttttgagatagggtctcattctatgatgcccaggctggagtgtggtggtgcgatctcggctcactgcagtctctgcctcccaggttcaagtgattcccacgtcagcctcccaggaagctggaattacaggcgagggccaccactgccagctaatttttgtattttttggtagagatggggtttcaccatgttggccagactggtctcaagctcctgacctcaagtgatccacctgccttggccttccaaagtgctgggattacaggcgtgagctaccacacccggctgatatttctttttaaaataacttaccttcttttgaaagtaatacatgtttaatgaacagaatttaaggaaaatataaaaaaacgaaataatctttgtaatcaaactactgaaaagaaaaccaaagttacattttggtgcatattctttttcattttcatcattgtaatttgcatttctttgattacttgtgagacactcctttcatttacttaataggtttatatgacttgcctattcagagattttgcagctttaccattttctgcaaatgatagcaacttctttttgtttgtttgtttgtggagacagagtctcgctctgtcactcaggcaggaatgcagtggtggaatcttggctcattgcaactattgcctcctgggttcaagcgattttcctgcctcagcctcccaagtagctgggattacaggagtgtgccaccatgcccggctaatttttgtatctttagtagagatggggttttgccatgttggccgggctgatcttgaactcctggcctcaagcggtccccctgtctcggcctcccaaagtgctgggattacaggcgtgagccaccgtacccagccagtagttacttcttatattctagaaaaaattctactcatgatcaagtctccatgaggaaagagactttaattgaagatcatggggcttgcagaccaatatgataaaatagttcattgtttctaaaagtattactgagtgttgatggcagatatgaacccttttgtttttgtaggaaaatgttacccgtattctccatttgaattcagtttagatttgttaggaatcgcagcttaagctttgccatctgggagtgtttgggacagttttgcagacaaaattgcaaaagtgcctaaggaatgcagctggcattcagacctgctctgtgctcagtactctgtggacagacactgttcagcacttgttgatcagaaggtttagaaagagaactttcaaagttggtttttaattaaagcatttaatagtgtaaatagaaagggattaaattttatgacagacaaaagaaagtacagcacccagctgggcgtgggggctcacgcctgtaatccagcactatggggggctgaggtgggtggatcacgaggtcaggagttcaagagttcaagaacagcctggccaaggtgatgaaaccctgtctctactaaaactacaaaaattagccgggcgcggtggcaggcgcctgtaatcccagctactcaggaggctgaggcaggagaatcacttgaacctggacggcagaggttgcagtgagccaagattgcaccattgtactccggcctgggccacagagtgacattctgtctcaaaaaaaaaaaaaaaagaaaaaaagaaagtacagcacccagttatgtccgagtgggtgcatgagagtgaccctgagattggagacaacgctgtcacgtgcttgaagaacgccacctgagaaagggggcgagaagtggtgtccgctggtaaccagaggtgttggcttagccatctgcagggaggagggtggtctatcacaggtgagtttcatctactttcttaagcaaattaaccttacttttgtgttaggcttgtcccaaagctgttttataaatgtgaccaaggacaagctgatccagtagtggccgtggcaagagatcaaagcagtgtttacctgaaacttctcatgcatgagacgcagcctccatctcatttctccgtcagcacaataaccaggtatgctgacccagtggcatcttcacattgtcgggaaaatgccctttcctgatgcctttctttaggctttaattgaaaacattttattttctagaaaaaagcttcagctcaggatgtttgagtgtaggtcagtcctttgataggatattatcattttgaggattgaccacaccacctctgtatttaagctctgccacaatcactcagctgtgacactgtaaatctcttaatagtttattacattccatgtgctgacagttgtatttttgtttgtgacacttacgtattatctgttaaaacattttcactttagttgtgttacctttaaagaggattgtattctatcatgcctgttgattttttggtgagcgggctattaaagtcagtgttatttagggttatccactagttcagtgatttgcgagattatcattcacatttattgtggagcttttgaatatcgtgtcaaatggccacatatatcccattcttatctgcttcttaggtgagtgggacacagtgctttaatgaagctataatcttcagaattctagcttgcagagaagattgcagaagtgataagacttgtgctttttaattttgtcttttaaatgttattttaaaaattggctttatatgatactctttttttctgctgagtaacagtgttttacaaaacttggactaaatgacttctaagcttaaatgatcacttgatgctttttttctgaattaggaactcagcttatcaaatatcaaagtcataattcctgaataaataacgtcttttttcatgtaaagactgctttaaaaaacacatggaaggctgggtgcggtggctcacgcctgtaatcctaacactttgggaggcccaggtgggcaggtcgcttgagctcaggggttcaagaccacccagggcaacatggcaaaacccacctctactcaaatacaaaaaattagccaggcgtggtggcgggcccctgtaatcccagctactcgggaggctgagggatgagaatcacttgagccccggaggcagaggttgcagtgagccaagattgtgccattgcactcccagcttgggctacagagtgagactctgtctcaaaaaaagacacacacacaaacaaaaaaaacatggagacatttttttggccaccttaatatttcccctcagataatttcctttgtttaaactcagaactggcattttctctcttggagaagattcaggacaaatactcctttaagataagtagaagcagtgaaagaggatttgattatcaggaatttgataagcttagaataaattgttgcttcttaatgtcatttcagaagatgaatatttattaatagatgccaactgagatatcattaaaattgattactaactactacttggaaaagtctcccagttccaaacttcagcaggcctcttgacaattcagctgtggtcaattgggtcttgcgtgatagatacaatgaccaattgtgcagcagagtgtgctgcttagctgcctattctgttagcattcatgtgttaacttaaaatcataatctccttagttttgttgagtgtctccgtggacaagacactgtgagggatacaaaatcagattggctttattcaaaccactggggtattataattcatttataatttattttattttttgccttttttccatgtgttctaaaggaattagagtttgtatataactataatgggggatagaaattgacatgtgccatgaagggaatgcaaaaaagtgccgtgggagatgagaagtggagaaaggaatttcttttttcttggaagcaggaataacttcatgaagcatgtatttcaacttaaacagatagtaggcaacgctgtaaggggagtatggctgcagcaaaagtgttcggggcagactgggaggaagggagggaataaattcagccattgttatggaataatgatcaaaatttattttcagcccgtttcacttaaaagttgagactgcttaactttttttaatctttaatcttaaacttttaaatgccatttgatctttaaaaatatatgttttaatagtgtattttaagtctctatatttttgttattagaatatatagaggctataacctactaccaagcataacagacgtcactatggaaaataacctttcaagagttattgcagcagtttctcatgaactaatcacatcaaccaccagagcactcacagtaagtctctttcttgatcggtcttactgacattgtaatagtttttggtagcttgtatggccagttagttgtatggtcatcttacggtgaggtgcttgtcttacagctcttacttatccatgaggcttgctaagaaattgtgcttctgtgaaaagaatctcagcttactccaggaatgtaaatgactatgttttttctgattattaaagtaatacacgcccaaaataaaaaaattcagccaatttaggaagacacaacaattaaaataagccaggcatggtggctcatgcctgtaatcccagcactttgggaggccaaggttgggggctcacttgaggtcaggagtcggataccagcctggccaacgtggtgaaaccccatctctactaaaaatacaaaaattagctgggcgtggtggcgggcgcctgtaatcccagctactcaggaggctgaggcaggagaatcgcttgaacctgggaggtagaggttgcagtgagctgaggtcaagccactgcactccagcctgtgcaatagagcgagactctgtctcaaaaaaaaaaaaaaaaaaagaaaagaaaaaagtaaactactgtcacctgcattggtaatgtatcagaagtttaaaatgtctagattataattaactcagtgacctggtaatatatactaagggaaaaatatttataatttacatttttacatttttatttttttaattttattattttttttttgagacagagttttgctcttgttgcccaggctggagtgcaatggcatgatctcagctcaccacaacctccacctcccgggttcaagcaattctcctgcctcagcctcctgagtagctgggattacaggcatgcaccaccatgcccggctaattttgtatttttagtagagacagggtttctccatgttggtcaggctggtctcaaactcccaacctcaggtgatccgccctcctcgaccccccaaagtgctgggattacaggtgtgagccaccatgcctggccttacatttttataataagaatttatgttgctgacattagaaaagaaccataatatccaagaatccaagaataattaaattatgtacatatgctagtatatagtgtgatgctttggagaatttttaacaatatggagatgtataatctggattgtaatattgagtgaaaaaaggcagaatacaaacctggtgggggtatagtcggatttcagttaagaaaaataatatttacatatatacatttctcacactggcagataatcaccaagataaattttgggattgtggatgatttttttcttctttatatttttcagatattctcaaattttctaaaatgagcaagtataacttttgttatcagaaaaaaataatatacaaaagtaatgttaatttgctggtgaccaggttaaacctttttatttttattttttgagatggaatctcactctgttgcccaggctagagcacagtggcatgatcttggctcactgcagcctccgcttcctgggttcaaatgattctctggccccagcctcctgagtggctggaattacaggcgtgtggcaccacacctggctaatttttgtatttttagtagaggtagggtttcaccaggttggtcaggctggtctcgaactcctgacctcgtgatccacccacctcggcctcccaaagtgctgggattacaggcgtgagctactgcgcccagccagacctttttattttatttgacaaaagaaatacttccatgttatagaagactaaatattgtttgggctgtctgcagtatggtcttcccttgatttgttcaaaatatcgtaaactttgcttatttatttttattgtggccgactgtgtcgggcactgttgtaggcttgggatggaaaaacaggattcctgcccttagggtttctgcaggctggtcagggagacgatgtggtaagctggagctcagctcctaaggatgtgcaggggcagttgagaggcggaagggtgggagatcattccagggtgtgggcagcacaggaacctctcttcattgggatataattgccattctgataacacgtgtttgaggtgtctaaagtaggaagttgtaccatggtgggacagatatcctgtggttatcatacacagatctcagttttcttctcattgtttgtactttttataaagggtaacaggagatataattcaataaacctttgtggtgtttgggtgtgattttattgtttctttcttctcagtttggatgctgtgaagctttgtgtcttctttccactgccttcccagtttgcatttggagtttaggttggcactgtgggtatgtattttcctcagtatatattaatagttgtctacaacagtatgacataaacatagttattaggatgccctttttctttctttttaagtcttttatcaatttggctttttggaaaaatatctgatggaatacttgtttctgctatattagctgtgtgagactagtgacaggagctgtgggaaatgaatgccaaatgttcttaggcattgatgggaatttcagggtgtggtcttcaagttcatttaagggaattttcatatgctggcaaaaggcttttctcattagcttgactctttccaaaattatttgctgtgaattagaagtttaggaaccttttttcacttaattgtgacctagcatacgaaatggtgatgatttaggaactactgttcttgtattaacagcttttatttaaaaatgattttcctccagtagatggccctactagcatctgggaaataatttcaagtcttctccagcattcaggaataggctttcattttgtgtatcaattactgagaatgattttggtgactcacatcacatttgagaagtaaacctgcagatttcttgtgtgtgtcagcaaatgaccaactgatatttgcttgaagtggattacattatctgctctagaatgattgctttcccaccttcctcacatacagactgagcagctacggtttctaatcataggtctggcactagacttcacttctgggcaactttggcattggagtaaaatgtattaatttaaagaaagttaaaaatccgttcaagtaaacatacagttctaatactttttacaatttaaaatatagatttaaatgataaaataaaaaagaaaatatgggtagacaccataatcctcgtttctgcatctgttcacaaggggttgatatttatgagttctattctccatatccattctatgttctcttaatgctcagtcagcacctcaggtggttggagttcaatgcttggtagtttgacttacactgtcttttctaggggattgagccctgggtagtcctgcttatttgaggttgcaatttgtctttcaataacttttactacaagatatggcgtgttaaaggataccattggggaaccaacataataatatcaggaaaactaaccacgtcagacctgccccattgtgtatcaagtacactatttttccatagtaataaagagttcaccccagccaattctcttttattttgtgcctgtttactcaatggcattaacatgcccaaatgtctgggtagctgtctcatctccagttcagcagaaccattgtcatatgccctagtaaaagcattccttcattggacacttaggccccaatactttcattcagatctactacctgatttcatttctcaaatgatttttatggagctctgatttataggaaagatgttagttgattaaaaataaaacaatttctgagctggtataaaatgtattgtgacatgccttcctcttggaattgcaagagaaaggaagactgttgtttgcttaaaaattgtctataatttgactttgcaaatgtctgcttccagagtgcctccactgagtgcctcagatgagtctaggaagagctgtaccgttgggatggccacaatgattctgaccctgctctcgtcagcttggttcccattggatctctcagcccatcaagatgctttgattttggccggaaacttgcttgcaggtactggtactgagttgaaacagggactccaggacttggattttgatttccttagggggaatgggggtggtgagcatatgaggggaaaatactataaggtcattgccagtgatggcttgtccctttagtcaaatttcagatgttacctatatgcataaacacatgcagttggcagctgttctgtgctgagtattttaaagtagcctcttcccaatatagcccctcagttaactacaagtaaactcattttgaatttcattttaatgggcaccatatgccagtactccctcgggcactgggatgttaagaaagtataatgtatggacttcattctcaagttagttttagattagagggggatacacgtaaacaaaagtgcagtggtcacacagagtggccctaatcactctccttgggcagatttatgggctggtaggaaagagcacaacacggagagggtgtagcaccttggcgatgataatggaggatgtggccagcaaggaagacggagtccattgaaattgattttgggagaagttgccaatctccatgaaagaattggggcctgtgctatttgcttcagggggctataggagagtttcgtgaaagggactaaaagatgagtattttaataagatcattcatccaacttgaacatgggctggaggagaaggtagggagactcaggagattaatgttgatgctaaggcaagataatggctttgggactgtagggaagacactgattgtaagagaatgaaggaggcagaattgccaggcctggttcaccaactgaacttcggttgtgaagacaaagaaacctgggatgacttcacatcctgggcaggtgtgtggtggtgacagtcatggaaattgggaacacagatttgtgcgggaaacatcagtttcagtttgagtttggcttatcagttgaatatcaggcacagatgtctggccaactctcaacatagggtcttaaatgacttcagttccccaagcaatttgtccttcccatgctattggggtggagaggtaatgtctgtgcccatatcacagccagtgctcccaaatctctgagaagttcatgggcctctgaagaagaagccaacccagcagccaccaagcaagaggaggtctggccagccctgggggaccgggccctggtgcccatggtggagcagctcttctctcacctgctgaaggtgattaacatttgtgcccacgtcctggatgacgtggctcctggacccgcaataaaggtaatgtcccacttgggtgctggattcatacagccttaatgactatgggtttccagactacctttgtttagtaatctgtcccttctttattctctttttgctttaaatgaacaaaattgctcagattgtgacactaaatttaacatcaaaatgtgaccatgtggatgggtgcagtggctcgtgcctgttattccagcactttgggagactgaggcaagtggatcacttgaggccaagagttcgagaccagcctgggcaacatcacgaaaccccctctctactaaaaatacaaaaaattagatgggttgggccgggcgtggtggctcaagcctgtaatcccagcactttgggaggccgaggtgggcggatcacgaggtcaagagatcaagaccatcctggctaacacagtgaaaccccgtctctactaaaaatacaaaaaaattatctgagcatggtggcgggcgcctgtagtcccagctgctcgggaggctgaggcaggagaatggcgtgaatccgggaggcggagcttgcagtgagccgagatcgtgccactgcactccagcctgggtgacagagcgagactccgtctcaaaaaaaaaattagatgggcatggtggtgcgtgcctgtaatcccagctacttgggaggctgaggcaagagagttgcttgaacctgggaggcggagtttgcagtaagccttgattgtgccgctgcactccagcctgggtgacagagtcagactctttccaaaagaagaaaaaaatgtgaccatgtgttttatagctcttttagtatcatcagtcactgttatccctaagagggaaatacctagctttagttttaggtttccagcattagccaagaaagctcagaattgatgttcctggccaagtacctcattgctgtctccttaaatcttggttaatggctactgtcctggctagcatagttatggagcatttccatggttgtagaatgttctgccaatctcagggacagttttgcttttctgtgaagcaataaaatcaacttcaaaacaaatgttaactatttgtacaatggatttaagatagaccagttcacatacttttttttttttttttttttgagatggagtttcattcttgttgcctgggctggagtgcaatggtgtgatctcagctcactgcaacttctgcctcctgggttcaaacgattcttctgcctcagcctctcgaggcagattacagctgggattacaggcatgcaccaccacacccagctaatttttttgtagttttagtagagacggggtttcaccatgttggtcaggttggtctcaaactcctgacctgaagtgatctatccgcttcggcctcccaaagtgttgggattacgggcatgagccaccacgcccagcctaagatagaccagttcacttactgtttatatctgattactctctctttgccttgtcttctacctttaaaaatctccctactaacttcccattctcctttagctgccatcagtcttctcccttctctgcaaacatctctggagagtcccagcctcagcccacagagcttcccactgctctgaggtggaccttgtttgcaaggcttctttggctctcttggcctggaccctgtctactacttcagccatccttccttaacccctgctggtggtttctgttgccacactccatagcagcgtttcccgcccagatcatgtctttacatctctgggcactgctctggtcctgcctgcctttccctctttgtatcctgcaggctgctacccccatcttgagtgtcctcttcagttggctttcagagggcctcctgggtgttcccttacccacttgccactccccagtcactgggttcagtccttcctgcccaccagcacatgctttctaggctctgtcctaggccgtcttctctctttgtagtctctgggccagtgctgttctagagagtggcagaattttctataaccatggcagtgctccatagctatgccaggcaagacagtagccactaaacacatatagctgttgagcccttgaaatgcagctagtgtgactgaagaactgaaccccgattcggtttaattttcattaaatttaaatttaaataaccttatgtgggtagtggctccagtattgggcagggcagcctgagagtcggggctgttctcctgtcttcagtgtctagatgagggacctcagaggacctgtctctggagctgcagttcaatgtagccagctgccccgtgacacttacatatagctgatttgtggatatgtcagacacggtgtgatgagctcagctttctgtcctcctccccacatctgcccctgccccatttaccccactttgtgtcttatcaagctagaaacaggtcaccacaagtcttcatttccactcaccaagtcttttgtttcccctactaaatattttgcgagaagaaagtgtgtacctttgtattcacatacatgtacatgcacatatacatgcacatatgcaggggtccccaacctctgttaaaaaccggactgcaggccgtgcgtggtggctcacgcctgtaattccagaactttgggaggccgagaccagtgcatcacaaggtcaggagatcgagaccattccggctcacacggtgaaaccccgtctctactaaaaatacaaaaaaaaattagccgggtgtggtggcgggcgcccatagtcccagctacctgggaggctgatgcaggagaacggcgtgaacctgggaggcggagcttgcagtgagccgagattgtgccattgcactccagcctgggcgacagagcgagactctgtctcaaaaacaaaacaaaacaaaaaaaaaaaaaaccaggctgcacaggaagaagtgagcaagcattaccatctgagctctatctcctctcaggccagtggtggcattagattctcataggagcgtgtatgagttcgttctcacacttctgtaaagacatacctgagacatataaagaaaagaggtttaattggctcacagttctgcaggctgtacaggcttctgtttctgggaaggcctcaggaaacttgcagtcatggcagaaggtgaaggggaagtaggcacatcttcacatggcccacaggaaaaagagagaaggagagagagagagagacagagagagagagagaaaaagaaagattgagagggagagaggagggagaaaggagagtgcctgtagggggagttgctacacaaaggagcaccagggggatggtgctcaaccattagaaactacccccatgatccaatcacctcccaccaggccccacctccgacactggagattacaattcagcatgagatttgggtggggacacagagccaaaccatatcagagcatgaaccctattgtgaactgcacatttgagggatctaggttgcatgctccttatgagaatctaatgcctgatgatgatttgaggtggaacagtttcatcccgaaaccatcccccgccaaccctggtttgtggaaaaattgtcttccacagaaccggtccctggtgccaaaaagtttggggacctctgcacatatgcatgcacctgtacatggacacataatacatgtacatatgcatactttatattctctgccacttctggtccagactgatatactatctcatttggattactgcactagccttttgttttggaaacagcattttttaaaaaatttaatttaatttttttgagatagggtgtcattctgttgcccagcttggagtgcagtgtcatgatcatagctcactgcggcctcgatctcccaggctcaagtgatccttctgcctcagccttctcagtagttgggactacaggcatacccaccatgcccagctaattttttgatttttttttttttttgagacagagtctcagcctgtcgcccaggctggagtgggttggcgcgatctcagctcactgcaacttctgcctcccaggttcaagtgattctcctgcctcagcctcccgagtagttgggattacaggcgcctgccaccacacccagctaactttttgtatttttagtagagacggggtttcaccatgttggccaggctggtctcgaacttgtgacctcgtgattagcccgcctcggcctcccaaagtgctgggattacaggcgtgagctaccgctcccagccaggaaacagcattcttgagataattcatataattcacccatttaaagtatataattcattctctttagtatgcccacagagttgtacagccatcaccagaatcagttttagaacccataaaggaactctgtactctttacccaaaacctccatgcctccagctgcaggcagccactaacctgccttctgtctctgtgactctacgtcttctggacattactgtggatgggctcatacagtcagtgagcttgtgactggtgccttctaccaagcagggttttcagtgtagcagcctctctgtttttcttttttttttaaattgtgacggaacttctgcctcccgggttcaagcgattctcctgcctcagcctcccgagtggctgggactacaggcccatgtcaccatgcctggctaattttttttttttttttttttagtagagatgggtttcaacatgttagccagggtggtctcgatctcctgacttcatgatccgcctgcctcggcctcccaaagtgctgggattacaggcgtgagccaccatgcccggctaacctttcatttactgtctgcatttcttccctgatgccttccagtccatgcacccgattgtagccattcatcctattatggtttaaggtgactgtcttagtcagcatgggttgccataacaaaataccatagcctgggtggcttcaacaacagaatttacttctcacacttctggaggttgggaagtccaagatccaggactttcgccttgccctcatgtggtgagggggtgaggaagctctgtggggcctcttatatatggatgctaatctcattcatgaggggtctgccctcatgacccagtcacctcccaaaggccccacctcctaataccatcaccctggtaattaagtttcagtgtataaatttgggggactatagacattgaaaccataacaagcacttttctaagatcagggagtgagtaagtagcagagctaggacctcaattccacatgtcagtcatcttgccttcactctgctccatgatggctgcctcctagagcattgggagtctcgatgttctatatgctctcatgtgttgtgtattggagatagttgaggctttatgaatacatctggatttgttgacttctagctttgctggtaaccagctgtgaccttgaataagttacttcatctctgagcctgtttcctcttttagaaacaggagtttaaaatgctgctttgggttgggcacggtggctcatgcctgtaattccagcactttgggaggctgagatgggaggatcactggagcttggagttcgagaccagcctgggcatcatagtgtgagatcctgtctcctcaagaaattaaaaaattagctgggtgatgtggcgtgtgcctgtggtcccatctactctggaggctgaggtgggaggattgcttgagcccaggaggttgaggctacaatgaaatatgattgcaccccatcctgggtgacgagtgagaccctgtctcaaaaaagaaaaaaaaaatgctgctttgtacccctttcatgtcatggcgtcatggccaacatagaatgccctggttgtttgctgttggagggcatgggcctgggggctccctgagggctccttccatcttcaactcattctctgtgcacctgttaggaagttgtgggccagtccctaccatgtatcattgtgtgggtaaaagtaaataaaatgtgtacagtgtctgaactgtacatatcagggtccaagaacaaaatgagtgacatgggttagctctttttaataaatggtaaaaccaaatattctaattttcagttttgttatacttccatcacatgtttttgtttttttgttttttgtttttgtttttctattttaggcagccttgccttctctaacaaaccccccttctctaagtcccatccgacgaaaggggaaggagaaagaaccaggagaacaagcatctgtaccgttgagtcccaagaaaggcagtgaggccagtgcaggtaggaaacagcgtggggaagggagggacatgagtgcagcatctgtcatgtagaaacataggatttaagtaacttggtgttttagagaaataaatataatacacatcagtaaagtgagagaaagtttctccaggtgcggttcaagatattagaaactaatgactgatgtacacagaccaccttttggtctgaagcatttctaagtgccactggctgacatgcagcccctacagcctccaggcttccagccctagcatggagcatcactctcctatgcttccctggttgcaggtgatggctggagaggcctcctgattttcagtaagggaagtggtgtagatgcttaggaatagatgtagtgagtgaaaaaactgattctgatatgtcaaaaattctgattggaaatggaatatttacatttggaagagctaaaggcgagagaaagtggggataaagtcatctgagttggaggagcttaaaccattcacaagtttggaggacctttttttacccatgaaaaggtcagaacagaaggggctaggatttaggtgtgactgcagtttattgaattcccatccatactgctctcggtgggcagtggcaggggcaggagaggagcctggcaaagcatgaagtgactgctgctgcctctgctatctgggacgcctggccacctgtctgtacagtctccctccagacccattctcacgctgtctcttggcacccaggggccagtgatggttctcccatttgttttgtgtatatagcatttatatcaaggctatttatttatttatttattttatttatttatttttttgagacagagtctcactctgtcacccaggctggagtgcagtggtgcaatctcggctcagtgcaagctctgcctcctgggttcaagcaattctcctgcctcagcctcctgagtagctgggactacaggtgtgcaccaccacacctggctaattttttgtattttttattagtggagacggggtttcaccttgttggccaggatggtcttgatctcctgacctcgtgatccgtccacctcagcctctcaaagtgctgggattacaggcatgagtcactgtacccggcctatttatttatttttaattgacaaaattgtatatatctgtaatatacaacatgatgtttgaaatatgtgtacattggccaggcgtggtggctcacacctgtaatcccagcactttgggaggctgaggtgggcggatcacgaggtcgggagttcaagaccaaactggccagcatggtgaaatcctgtctctactaaaaataccacaaaaaaaaaaaaaaaaaaaaaaagccgggcatggtggctcgcgccagtcgtcccagctacttgggaggctgaggcaggagaattgcttgaatctggcaggtggaggttgcagtgagctgagttcatgccactgcactctagcctgggcgatagagcgagactccgtctcaaaaaaaaaaaaaaaagaagaaatacatatgcattgtggaatggctaattaacctgtgcatcacctcacgtatcattgttttgtggtgagaacacttaaaatctactctttcagtgattttcttgcatatggtacattgctattaactgcagtcaccatgctatacagtagatctcttgaactcattcctcctgtctataaatgaaattttgtatccttgaccaacacattcaaggttttttttgagatggagtcttcttcacccaggctggagtaccatggcacgatctcatctcactgcaacctccgcctcccaggttcaagcaattctcctgcctcagcctcctgagtagctgggattacaggcacatgctactgcacctggctaatttttgtatttttagtagaagtggagtttcaccatgttggccaggctggtctcgaactcctgacctcaagtgatccgcctgccttggcctgccaaagtgctgggattacaggtgtgagccactgcacccggcctcaagcgttttaaaagatgctcttttctaaggattgactgtagtacaggaggaagattgacctgttgaaaagcctcagcctttacaagtgtaaaattatcagtatattactatcatctttctgatgaattaaataaactaaggactccaagtcaaaagtcttcaaactgaagtagaatagttgtatatagtgcttggcactttaatatttagtatcggtttaatgataatgtttgtgcctttgccgtctttaaaacatttttacatcatccctgtttgattacttggtgtgctcatgaagttgttggccactaaggaatcttaggctcagagaggttctggaattggccagtggtccttgaatcagctgctcctatgattctctaactgatttctcacaaagcaaacaagcaatcataacaaaacaactgtgcacactgctcttcttattttgttatttaaaaagtacttaggctctacttatgtttgttagtcaatttctcattacttctagttaatcaaaaggtcagaggaaatacttgaatattttcatactagaatactttaaaaaatcatgatttccagtaatctctttaaaacttggcaagttattttgatctaaaagtttatcttttgtgtgcatatttttaaagcttctagacaatctgatacctcaggtcctgttacaacaagtaaatcctcatcactggggagtttctatcatcttccttcatacctcaaactgcatgatgtcctgaaagctacacacgctaactacaaggtatgggcctctgcatcttttaaaaatatatatgcacacatacttacgtctaatggatagttgatgtttttcttatgatttgtaggatgtataagccctttgagatatgagttacatttagttttttcaagtttgtttgtctttcagctttgtttatgatagcttctatcatacaggtgttttggattttcatattgtttgtactcacagctaagattgattacagtgacagagctaggatgtgcagccaggttatagggggaagtggccctggtggagtctggagggatccgtgtacaggcttccttccctcccgtgaggctcacacaaaaatacagcaacatgctggtcctgcaggtaccctctgcctaacatgagccacaattccagactcacagaagaaaagcaggtgttcggcataaaccatgtgtttcaaatagtctgggcatggtgagccacttgttatcagctagggaaagtttatgtcagcgtaagaaactgttcaccagatacccccaagagccagcctttctgtctagggatgttttagttttttagttcatttttttttttaactttaaaattttctgttcatctgcaatttgttagatatgaagtatgtgtctaatttaatttttgtttttggttgtccccaataatgtttacagaagaatttttctgcactaattggcttgagttacttacattctcatagttctctagtttcagtagtttcatttattattttgttatatcaatctatctgtctgctcatctattagaagcatccttgttttttttttttcttttttagacagagtcttgctctgtccccaggttggagtgcagtggtgcaaccatgcctccctgcagtctcagggctcaagtgatcctcccacctcagctcctgagtacctgggactaccggcatgtgccaccacacccagctaatttttacattttttgtagagacagggtctccctaagttgcctgggctggtctcaagctcctggcttaagtaatcctccctccttggcctcccaaagtgctgggattacaggtgtgagcaactgcacccggctacaagtatacttcttaattattgtagcttaatggtatttatgaggggatcagttcccctgttgttctttagaattttctggatattcttctttattgattttgggatgtgaacaatagaatcaacttctacttgtagattgatttagggagaacttatacctcagatgttaagtcaccctgtccagaatgtgggatgctttcctatttgttcagaactttttaaattacctcagaagcacatgaaatttaaaggattttaaaaaaaacttaaagattatttcacatagctcttgcacatttcttgataaatgaatcctcaggtattcctctgtttttgttactaatagttacttcttatgggttttttttcccctgaaaatcatttatcaaacgtatgtggcttattttctgaaggatgtttgataattttggaagatatgaaagtcttcatattttacaaggtttgaggtctctttaagctgcatggttctcatgtcagctcccaaagcagaagacggcatgttgaaaaatgccgtagagaagatacttcttttccacctgttttcaactcatatcatcttgaatttcagggcacctttccatgctcctagtgcttgctatctgtttattattttccttcctgaataccctgaactccagcatgttctgctgtaattctggcctccctggcatcttggactcctgtttcctttgctctgtcatccccgcggtcagctcctgctgcgcagcttctcagctgaagtgcgtttggagtgcctggcgtgtcttgctggatctttgagtattgcctctggtttccttggttccttctgctgagttgctcagcgtctccactccccatttcttgtgtggcccttcctgcactcctctgattccttttgtcttccctggtttcttgctttggtttcgagtctccacagaacttttgcagctcttctgaagacctggaagctttttcatcttaattctcatctcatgacctcttttcccttctttgagagctagaacttcccatggtgaacttctctttccagaattccatgccttcttttccctcccacttacctgttgtccaggagaggtcagattgctgtgcatattggaggagaaccctttcttccctgggctcttcatctcacatgacatcaccacatcacctcgttccttggaccctcagtggtgtcactgctggatttttctttcctttggctggccttagggcacacccaggttgactagcgtagtcatggtatttagatccactcacattttcagtttctgtgtctgtctcttgcctgcttctgacttcgcccagagaaagcttctctttcacaagggttcttagatttatgttcactgagcaccttcttttctgaggcagtgttttaccaatatttattttcctagtcagtctcgccttacctttcttgttatgcatgtctttggtcctgacccattctctgagtctgtaaaatagaattgctgtataatttaattacatgaaatcctttagaatcttaacacatcttacacctgatttaatattttattgtatccaaattgaaccaaccctatgtgaatttgacagtgatttctcccagggatcctagtgtataaggaataggacttagtattttctattttttgatataccacataccagatactgattatgatggacatttaacccttttttctcattatgaaagaaagttaggaattatttcttccagtagcgccagtgtaacctgaaagcctttgaaagagtagtttttgtatagctatctgaaaggaatttctttccaaaatatttttccagtgctgacaacaaacacgcagacacaccctgcaaggtgagtgtacggcgccgcacagtggaggcatctgctgcagccgtcgatgtttgtgtctttggttgtacattatgagatcgtgacagggccagtaaccgtgtgttctctccttcaccttcccaaggtcacgctggatcttcagaacagcacggaaaagtttggagggtttctccgctcagccttggatgttctttctcagatactagagctggccacactgcaggacattgggaaggtttgtgtcttgttttttctccttgggttgtggctggcacacttgatgtgcgtcttctgggctgagttcatctaggatggagcctggttctccagggtgcctccgggagactcctccctgccccacgtgcttgcgtcacaggacccaagtctgactctgccttagccatgaagtttagggggaagtttctatttgtattctatttttgtctgttatcatgtattagcttagacccagtttagtttggaaaatcagtgggtttcaaaatgtgtttgtagagtcctttatttcttaacttgaccttttcaagtggaaaggggcaaaacagacgggtaagggggcggggcgggaggtgtgacttgctcttttgtgcctgaggaagtaacagagctggggttgacagtcatattctctgacacagatagtctctgacttatctcacagaaagtcagcggcagagcctgagttaaaagtctcgtagattttctttttcttttttttggtggctaatttcagttttatttatatttgtttatttatttattatactttaagttctgggttacatgtgcagaatgtgcagttttgttacataggtatacacgtgccatgatggtttgctgcacccatcaacccatcacctacattaggtatttctcctaatgttatccctcccccagtcccctcactccccatgggccccggtgtgtgatgttctcctccctgtgcccatgtgttctcattgttcaatttccacttgtgagtgagaacatgcggtgtttggttttctgatcttgtgatagtttgctgagaatgatggtttccagcatcatccatgtgcctgcaaaggacatgaactcatccttttttatggctgtatagtattccatggtgtatatgtgccacattttcttaatccagtctatcattgatggacattcgggttggttccaagtctttgctattgtgactagtgccacaataaacatacatgtgcatgtgtctttatcgtagaatgatttataatcctttgggtatatgcccagtaatgggattgctgggtcaaatggtatttctagttctagacctttgaggaatcgccagactgtcttccacaatagttgaactaatttacactcccaccaacagtgtaaaagtgttcctatttttccacaacctctccagcatctgttgtttcgtgactttttaacgatcgccatcctaactggcgtgagatggtatctcattgtgattttgatctgcatttctctaatgaccagtggtgatgagcattttttcgtatgtctgttggctgcataaatgtcttcttttgcgaagtgtctgttcatatcctttgtccattttttgatggggttgtttgcttttttttcgtaaatttgtttaagttctttgtagattctggatgttaatcttttgtcagatgggtagattgcaaaaattttatcccattctgtaggttgcctgttcactctgatgatagtttcttttgctatgcagaagctctttagtttaattagatcccgtttgtcaattttggcttttgttgccattgcttttggtgttttagacatgaagtctttgcctatgcctatgtcctgaatgttatggcccaggttttcttctaggatttttatggtcctaggtcttatgtttaagtctttgatccatcttgagttgatttttgtgtaaggtataaggaaggggtccagtttcagttttctgcatgtggctagccagttttcccaacaccatttattaaatagggaatcttttccccattgcttatgtgtgtcaggtttgtcaaagatcagatgattgtagatgtgtggtggtatttctgaggcctctgttctgttccattggtctatatatctgttttggtaccagtaccatgcagttttggttactgtagtgttgtagtatagtttgaagtcaggtagtgtgatgcctccagctttgttcttctagcccaggattgtcttggctatgcaggctcttttttggttccatatgaagtttaaaatagttttttccaattctgtgaagaaagtcagtgatagcttgatggggggatagcattgaatctataaattactttgggcagcaaggccattttcacgatattgattcgtcctatccatgaacatggaatgtttttctatttgtttgtgtcctctcttatttccttgagcagtggtttgtagttctccttgaagaggtccttcacatcccttgtaagttgtcttcctaggtgtttcattcccttagtagcatttgtgaatgggagttcactcatgatttggctctctgtttgtctgttattggtgtataggaatgcttgtgatttttgcacattgattttgtatcctgagactttgctgaagttgctaatcagcttaaggagattttgagctgaaccaatagggttttctaaatatacaatcatgtcatctgcaaacagggacagttttacttcctctcttcctatttgaataccctttattgctttctcttgcctgattgcgctggccagaacttccaatactatgttgaataggagtggtgagagagggcatccttgtcttgtgccggttttcgaagggaatgcttccagtttttgcccattcagtatgatattagctgtgggtttgtcataaatagctcttactatgttgagatacgttccatcgatacctagtttattgagagtttttagcatgaaaggctgttgaattttgtcaaaggccttttctgcatctgttgagataatcatatggtttttgttgttggttctgtttatgtgatggattacgtttattgatttgcgtatgttgaaccagccttgcattccagggatgaagctgacttgattgtggtggataagctttttgatgtgctgctggattcagtttgccagtattttattgaggattttcacatcgatgttcatcagggatattggcctaaaattctctttttttgttgtgtctctgccaggctttggtatcaggatgatgctggcctcataaaatgagttagggaggattctctctttttctattgattggaatagtttcagaaggaatggtaccatctcctctttgtacctctggtagaattcggctgtgaatccatcctggactttttttggttagtaggctattaactattgcctcaagtttagaacctgttatcagtctattcagagattcagcttttttctggtttagtcttgggagggtgtatgtgtccaggaatttatccatttcttctagattttctagtttatttgggtagagatgtttatagtattctctgatggtagtttgtatttctgtgggatcggtggtgatatcccctttatcgtttttattgagtctatttgattcttctctcttttcttctttattagtcttgctagcggtctacctattttattgatcttttcaaaaaaccagcacctggattcattgattttttttggagggttttttttcgtgtctctatctccttcagttctgctctgatcttagttattttttgtcttctgctagcttttgaatttgtttgctcttgcttttctagttcttttaattgtgatgttagggtgttaattttagatcttttctgctttctcttgtgggcatttagtgctataaatttccctctacacactgctttaaatgtgtcccagagattctggtatgttgtgtcttcgttctcattggtttccaagaaaatttttatttctgccttcatttcgttatttacccagtagtcattcaagagcaggttgttcagtttccatgtagttgtgtggttttgagtgagattctcaatcctgagttctaatttgattgcactgtggtctgacagacagtttgttgtgatttctgttcttttacatttgctgaggagtgttttacttccaactatgtggtcagttttagaataagtgcaatgtggtgctgagaagaatgtatgttctgttgatttggggtgcagagttctgtagatgtctattaggtccgcttggtccagtgctgagttcaagtcctggatatccttgttaattttctggctcattgatctgcctaatattgacagtggggtgttaaagtctcccactattaccgggtgggagtctctttgtaggtctctaagaacttgcttcatgaatctgggtgctcctgtattgggggcgtgtatatttaggatagttagctcttcttgttgaattgatccctttaccattatgtaatggccttctttgtctcctttgaactttgttgatttaaagtctgttttatcagagactaggattgcaatccctgctttttttttgctttccatttgcttgttagatcttcctccatccctttattttgagccaatgagtgtctttgcatgtgagatgggtctcctgaatacagcacaccaatgggtcttgactctttatccaatttgccagtctgtgtcttttaattggggcatttagcccatttacatttaaggttaatattgctatgtgtgaatttgatcctgtcattatgatcctagttggttattttgcccgttaactgatgcagtttcttcatagcgtcagtagtctttacaatttggcatgtttttgcagtggctggtactggttgttcctttccatgtttagtgcttccttcaggagctcttgtaaggcaggcctggtggtgacaaaatctctgcatttgcttgtctgtaaaggattttatttctcgttcacttatgaagcttagtttggctggatatgaaattctgggttgaaaatactttttttaaagaatgttgaatattggctcccactcttttctggcttgtaggatttctgcagagagatctgctgttagtctgatgggcttccctttgtgggtaacccgacctttctctctggctgccctttccttcatttcaatcttggtggatctgatgattatgtgtcttggggttgctcttctcgaggagtatctttgtggtgttctctgtatttcctgaatttgaatgttggtctgccttgctaggttggggaagttctcctggataatatcctgaagagtgttttctaacttggttctattctccccatcactttcaggtacaccaatcaaacgtagatttggtcttttcacatagtcccatatttcttggaggcttggttcatttcttttcactcttttttctctaatcttgtcttctcgctttatttcattaatttgatcttcaatcactgatatcctttcttctgcttgattgaatcggctgtcgaagcttgtgtatacttcacaaaattctcgttctgtggtttttagctccatcaggtcatttaagctcttctctacactggttattctagccattagtctaacatttttttcaaggtttttagcttccttgtgatgggttagaacatgctcctttagctcggagaagtttgttattaccgaccttctgaagcctacttctgtcaattcatcaaactcattctccatccagttttgttcccttgctggtgaggagttgtgatcctttggaggagaagaggtgttctggtttttggaattttcagcctttctgctatggtttctccccatcattgtggttttatctacctttggtctttgatgttggtgacctacggatggggttttggtgtgggtgtcctttttgttgatgttgatgctattcctttctgtttgttagttttccttctaacagacaggcccctcagctgcaggtctgttggagtttgctggaggtccactccaggccctgtttgcctgggcatcaccagcagaggctgcagaacagcaaatattgctgcctgatccttcctctggaaacatcgtcccagagcacgaaggtgtctgcctgtatgaggtgtttgttggcccctactgggaggtgtctcccagtcaggctacatgggggtcagggacccacttgaggcagtctgttcattatcggagcttgaatgccgtaccgggagaaccactgctctcttcagagctgtcaggcacgtatgtttaaatctggagaagctgtctgctgccttttgttcagatgtgcccttcccccagaggtggaatctagagaggcagtaggccttgctgagctgcagtgggctctgcccagttcgagcttccctgctgctttgtttacactgtgagcatagaaccacctactctagcctcagcagtggtggacacccctcccccagccaagctcctgcatcccaggtcgatttcagagtgctgcgctagcagtgagcaaggccccatgggcgtgggacccgctgagccaggcacaggagagaatctcctggtctgctggttgtgaagactgtgggaaaagtgcagtatttgggcaggagtgtactgctccttcaggtacagtcactcatggcttcctttggcttggaaagggaagtcccccgaccccttgtgcttcccaggtgaggcaacaccccgccctgcttcggcttgccctccgtgggctgcacccactgtccagcaagtcccagtgagatgaactaggtacctcagttggaaatgcagaaatcacctgtcttctgtgtcgatctcactgggagctgtagactggagctgttcctattcggccattttggaagcatcccttgttttttgaggtggagtcttgctctgtcgcccaggctgacgtgcatcggcacaatctcggcccactgcaacctttgcctcctggtttcaagcgattctcctacctcagcctccggagtagctgggattacaggcacctgccaccatgcctggctaattttttgtatttttagtggagatggggtttcaccacattggccaggctagtctcgaactcctgaccttgtgatccacccacctcagcctcctagagtgctgggatcacaggtgtcagccaccacgcccagccatattttcagatctccctctctttgccctaaaccactgtgcttaataagtagtttttagtggccagcagtctccatgtataacacattttagcaaaatggaaaatactatatgttttaaatttgaacgtgagattatactgaaataaaaatcatctaactgggattctttaaatagtaagattttcttttttgtatgtgggtttttttttaaccttattattatgactgtcatatatagaaatggctgtttttcagttacagtcagtgaatgtatcaaatgctgccttatccaaataataaaagtaaattattaataagtcacaatttaatgaagattgatgttagttgatctttatattcttgaaatcagccatatggttgtgtgtgtatgtatatatttttaaaggtacataaagataataagctcatctctgaaaatttttacatttggcataagaataactggataattaagcatcttattctctggcctgtgtctttacagttaaaggtagatttactcacctctccttttttgtttttctaagttcatcttttttgctgtttcaagacagaggcccattttagctttctcgcatatccttttgtttgtactttggaagcctcacctgcttaattgttgagtttttatccgtggtcttttagagggggatatgtagggtagaagctttcacaggttcttgtttgcacttggcccctgactgttttgaggaatctccctcactgactcacagcatggcaaggtttcagatctctttctgccacacagcagttctgaggcagctggaaagatatccagatgcttagattgtcaggccaggcttgagatatacaaactattgagccttatctgtgaccttgcttaggtgaaggcatcagagcccctgcaccaacatgcataggcctctgcatgtgtgcggggctgggtgttgaggtctgagcacaagtgtagctggagaggtgagcttgatgtggcgacgggtatgagcaggttttcttcagacttctgtgagtttacctagttccaggatttaaaggcacagagactttagaattaaaatagaatcattttctttttctaaatagcaacactaggaataaaaaataataattccacattcttgacaggtaatgttttttcttgtcttctaatccttatttattccatactcatttttatacataattgaaatgtattatgcattggatttttcttttgcattatattatagacgatttttcatgtaactccttactgttccattttatatgttttgtctggtttaagactttatctgcaaaccgggaaactgtctctacaaaaagaaaaacaaaaatagttggccgcagtggcatgcgtctgtggtcccagctactcggggctgaggtgggaggattgcttgagccttgggaggttgaggctgcaaagagccatgatcatgccattgcactccagcatgggtgacagactttatactgtctgttttgggtgatttgataatgatatgccctgatgtagtttttttatatcttgtgtttcttgtgcctgggtttattgaggttgggtctgtggcttcatagtatttttaaagtttggaaaattttaggccattctttctttctttctttcttttttttttttttgagacagtgtctcgctctgtcgcctgcgttggagtgcagtgacactatcttggctcactgcaagctctgcctcctgggttcacgccattctcctgcctcagcctcctgagtagctgggactacaggcgcctgccaccacgcctggctaattttttgtatttttagtagagacgaggtttcactgtgttagccaggatggtctcaatctcctgacctcgtgatctgcccgcctgggcctcccaaagtgctgggattacaggcgtgagccactgcacccagctaggccattatttcttcaaagattttttttctgccctgcctccctccttttttccctctcttaaaggggctgtgatttcctgaatgattgcttagtgttgtcccatagcttactgatgctcttttcagtgtttgattgttttatgtgttttctgttttgtatagtttctattattgtgttttcaagttctctgatcttttcttctacagtgtctactctgttgttaatctgttaatctgttgttaatcctgtccagcgtatttttttttttgtttttgaaacagtctcactctgttgcccaggctggagtttagtggtgcgatatcagctcactgcaacctccacctcccaggctcaagcaattcttctgcctcagcctcccgagtagctgggactataggcacgtgccaccacacctggctaatttgtgtatttttattagagatggggtttcaccatgttggccaaactggccttgaactcctgacctcaggtgattcatccgcctcggtctcccaaagtgttgggattataggcatgagccaccgtgtctggcccctgttcagtgtatatcactaattttgtttttatctctagaagtttgatttaggtcttttaaaaatgtctccctgtgtttctgtttagctttgtgaacacaattgtaataactgttttaatatccttctctgctagttctaagatcttctaataacttcccagttcttggtgtttctcattggttgattgatactcctcgttttgggttgtattttcctgcctctttgtatggctgccaattttttattggatgcccaaccttgtgaattttactttgttggatgctatatatttttgtgttcccatagatcttcttgagctttgttctgaggttagttgagttacatatagatggtttactcttttgggtcttgctttataatttgtcagatgggttggagcagtgcttagtttaggactaattttttttttggactaattattcctctttaggaataattaggtaccatgcttaggaggcaagaccatcctgagtactctacctaatgaaccagaaagtttgggttttccagtccgcctgctgagaacagtgactttctagccctgtgtgagcgctgagctctgctccttctaatcctttccaatgcttctttccctggcctcagggagttttctcacacacatatctctgctgagtactcgagagggaccttccccagatctccagagctctctctgtcttgttttctcttctctggtgctctgtcttatgaactgtggctgtcttggtctccttagattctcagcacctcttcaattcagagggttgcctgtccctcctccttgtgccacagcctaggaactctctcaaagcagcgagttggggcagccatagggctgacttagtctctcgtctcccagggatcactgtccttcattgctcatgtccagtgtcttgaggactctgggttttgtctgttttgttttttggtttgctttggttgtctcaggcaggagggtaaacccagtccctcaccctcattgtgctcagtagtggaagtctcactctattacattagatattagtatttgtagcagagccctggttccctggtacttggggagctcttgaaaggccagaaacagcatgctttctcaccttttccagggcttcagtttctggtgcacatcaagcattccatacacatttgttaaagtcctttgttagacaagtagtgattcacaggttctatttgtaattttttcagttaacatgtattgggtatctgctgggagctagtaaaaacaaaaagtggtgtgtgacaaattcaattctgacaagaacaaccttaaacacttagaatatactttgagcatatcagaattttaaaaatgtgtggcccttgagtatttgaaaccaacaagaatctattgcttattagtagaggatattttgttaaacaagtggagagagaggcattttcagtctaattggtgttggcttttagcagctgatggaaaccagttcgtgattagccaggcagtggtgaaacaggctgtgcattctgaatgcctaggtatctaggcattcagaatggtggcgctctttgagttagcatcttcttctttcttgattcttttttttttttttttgagatggactttcgctcttgttgcccaggtaacaactccagtgcaatggcgccatctcggctcactgtaacctctgcctccctggttcaagcgattctcctgcctcagcctctcaagtagctgggattacaggtgtgcgccaccacgcctggctaattttgtatttttggtagagatggggtttcactatattggtcaggctggtcttgaactcctgacctcaagtgatgcacctgcctcgatctcccaaaatgctgggattacaggcgtgagccaccactcccagccccttcttgattcttgaaaaggacattgggtgctgtacatctcgttatagatgttgataaaaatgcttgtgagaagagtaacattaaggtagttatttggtcatttttgcagattattttaagacaattctaggactgatttgtggtaaatcacacattgctgtatcatagttgtgttcactgaacatattcaggggctctacagatgcagggctcttagctgctttgcacacttctgaattcctgccctgcgaacaggactggatacctaatagacaacaggtacttgataacagtttattgaattaatgagtgaatgaacagatacataaatgcatgaaagaatggttgtaatgtatataacttggatttcaagactttttactgactgttcaaaataagaaattgaaaactttcctctgattttcctctactatttacacaatttaaatggaagttatcttgtaccttcaatttctgtctaggattcgtacaataacgggtcatctctgagtcgcttaatgtctcacttgtctttctacagtgtgttgaagagatcctaggatacctgaaatcctgctttagtcgagaaccaatgatggcaactgtttgtgttcaacaagtaagagcttcattcttttcctcttctgttaagacgttcgggtatgacagcaaaacgctgctactccttaagaggcaggcgctgttggcataatcagctgggaggattgtggggtccagcgcagcactttttggctcagtccatgattgagccaagaggccatccttcccttcactccccaggaggacgaggtctgtcactgtggagggcagaggacaccagaagctcctctgcaacctcgctagttaacttccagtccctcggagtttctgtttagaatgctcaatctcatttagaattgcaaggaaacccaaaacgcctatttaaggtacaaacagcacttcatacaatatctcatgaggtattaatagtgattcacaggaagaatttcacgctgtgagtctttgctaacatatccagttatttacagatggatttgatatttgtgtgggagattcttaaaagtgttgttcacgccacattgttgatgcctcatttttttcactgtagttgttgaagactctctttggcacaaacttggcctcccagtttgatggcttatcttccaaccccagcaagtcacaaggccgagcacagcgccttggctcctccagtgtgaggccaggcttgtaccactactgcttcatggccccgtacacccacttcacccaggccctcgctgacgccagcctgaggaacatggtgcaggcggagcaggagaacgacacctcggggtaacagttgtggcaagaatgctgtcgttggtggaagcacgaaagagcaagcaggaaatactttgtaaaagaataaaaacgaaaaatgttagcgaacatcttctaatagtctgctgtattcagagaactctaggagatatatatggttgatgcaaagatgatttaaggcatagcccggccttccaagaagtgtgtggccagtgagtgagatgggcttgggacttacacatctcagaggtgggggtagaggaggaggaacactgagtgggctgagaagcagccagctctcattgccaaagtgtgtcagcaaaccagaatgcagttcataatgtccccacccattcaaagcacaggacctgtagagtggtgtggcatgtgttggtggcacttttcaggcctgtaacaaggatgaaagaacagcttcatagcagcacagtagtgctggtgttcagaggtgtgtgaaggccatagaagcatcttggatatattaccttgtgttttgtcagctttatgactagaagtctcttttcacttaaatttgttttttttttttttgagacggagtcttgctctgtcgcccaggctggagtgcagtggtgcaatctcagctcactgcaagctctgcatcctgggttcatgccattctcctgcctcagcctcccgagtagctgggactacaggcgcctgccatcacgcctggctaacttttttttgtatttttagtagagacggggtttcaccatgttagccaggatggtctcgatctcctgacctcgtgatctgcccgtcccggcctcccaaagtgctgggattacaggcgtgagccaccgcgcccggcctcttttcacttaaatttatgtttgtgtttttaatgcctagtatacaggacttcttaaattgccttaagtatgaacaggtatttgagttgctaatctgtatagtagcaataatagaatcccttgtttttccttttataaatttagcgattaaatagctacaattaaaacactagagtcaggagtcaaggaaaatacccatgttccaggctgtatgttagtgatgtacttactatatattggagtttcaggagtaagtctgtttcaatgctttctgtaaccatttggggtattaataagcatgtgagtgtgtgcatgtttgggttaatttcatatatgtttcttagaagggatatcattgatgtaaatattttaaaggcttgtcctccaaaaaaatcatgtaatttcttctaaattactgatcttttaaatgaccttcacctttctctcaaatctcacttaagactgggctgagtagtcagtttcctgtagcagaaaaaagctcagacttgagtagccttctgcgagtgaggagacttgatggctgtcaggcagctgtaaactctaaatagagtgtcattatctgaagagggcgatgctgccacactgagtggcctttcaagttgtttctcaatctgacacgttctgatcgtgtgaatgtgaaattggtttgagcaggagtatatctgagtgcagaggagattatttaaagatattctcattctctgcttcccttttattcccatttggcagatggtttgatgtcctccagaaagtgtctacccagttgaagacaaacctcacgagtgtcacaaagaaccgtgcagataaggtaaatggtgccgtttgtggcatgtgaactcaggcgtgtcagtgctagagaggaaactggagctgagactttccaggtattttgcttgaagcttttagttgaaggcttacttatggattctttctttctttttttcttttttatagaatgctattcataatcacattcgtttgtttgaacctcttgttataaaagctttaaaacagtacacgactacaacatgtgtgcagttacagaagcaggttttagatttgctggcgcagctggttcagttacgggttaattactgtcttctggattcagatcaggtttgtcacttttatctttcatccatcatacctgttcctaatttagtacaaattaccctaaaagacactgaaatctactttaaagaaatgtggtctgcatgtttccctcatcagttgctgctgcttatctttttcatgcacctagctggtgcagaaggcctggggcatagccagcctcagcaagtcagcatccttgccccagctccctggactcaaggctaacctggggttggctgttagggatttccaaaggtttgtcccatccacttgcctcccctccaaaataagtttgaatttaaattgtgagatacaattaagatttattgtttggggaacatttttgcaaaatctagagttagtttaaacagattatcaattattaccataattgatcatctgcagtttcaagctatctaacaggttcacttacctctttaaaaaggaatggaatttagcaggacagtaactgagacccgtgctcctggagtccatgtgggagctgtgtggctctgcacaagcatttgcacgcttcccctcttgactgcattaccttcctcctatagttgctgtgggcaccagattctggctagtcctgtcccttcatgatgcacattttcctcaagattcgtcccagttaaatcactgcagatgaaactgccttttcatcgtcaaaatttaactgtcatttttgagccgtgatcttgggctactttcttatgtggggtaggaatatttgtgagttagaaatattacacttctctatttccttctagacgtaaatctgttaatcctgtcagcactgttactcacctgaaagggtctgtttccctaggagaactgagggcactcggtcaacactgattttccacagtgggtattggggtggtatctgcttgttttttttgttgttgttgtttgtttttttttgttttttttttgagatggagtctcgctctgtcacccaggctggagtgcaggggtgcgatctcggctcactgccagctccgcctcagaggttcacgccattctcctgcctcagcctcccgagtagctgggactacaggcacccaccactacgccaggctaattttttgtatttttagtagagacgaggtttcactgtgttagccaggatggtctccatctcctgacctcgtgatctgcccgcctcggcctcccaaagtgctgggatgacaggcgtgagccaccgcgcccggcctggggtctgcttttaatgaaggaggcatcaaggggtgggctttgcgttggcctgatgctttcatctttctttcacaaaacctgtccgaagaaaatccgtctaaatgggccattgctctcctcaggaaatagtcattgggaacttcttttcctttcctttgacactaggaggctgactggggagaagccctggtctatggctgtgggcagcaggggctgagaggagcaggctctcaggggggcacgggtaccccaagggaagccagagccctgatttgttccattctagtaagaacaaagactgctctggtttcatgtttgttctgattgcctttcatcaaccggtcccctttctcccagttcttaagattcagtacagtgacagttttatgaacaagaatagaacactagaacagacaaaccattgaactctatgctgataaagatttattgagctcctgctgtatgtttgcattctgcccagaggctctgagaaaaccaggccatatgctccatgctttatccatggaagctccccgtcaggttgggaaagctgacagctgcagggaatacagtgtgacacaaaactggctcccatgcagcccttacgtgtcgcctctcagatggttgggggacgaaggtcgactcctttgggtatcttattactaaaccagtttcagggaatctgtgccaccctatctgccattaacgtgaacagatgagtccccaaggtgtaattttgggtattgtctgatgtctcttggaatttattatttgtttttccaatgagatttcacctcagggtatagtaaagttgttgaggggattcctggatgtgttctgcaattatctaggctgatttcagaatagagttatgcttatagtcaaatttatcagctgtcaagaattttatttaaaatttatgcagataagcaggaggaaaagaagcctggtttttacattttaatcctattattgatgtgaaattttattttccttcctgtaggtgtttattggctttgtattgaaacagtttgaatacattgaagtgggccagttcaggtaatagcattttattattttagatttttttcttcttcttgtgtacttacatgtaatttaggttattaagtgaatgtttaaactactgttaggcatttttgctgttttctttaaatggaaatctgactaacatactgtgcatttttgcttctcttaaaaattaatgtatatctcaagacttgtttggaagtagttatgtatctgaaaattccatatgttgtcagtattcattgcacatttcaaagcatttaattgtgttgacagatggtggaatgaaatcttgtggtggagcactagtttttaaatcttcttagagaaagcagttttatataatgttgtctttagtaattattatgcatttgtattctctgcagctttttcttgctagatgttgaggttttaatacttcttgctagtccattacaggtttataattattaaaagttaaaattcttttagtacctaaaatgcttaataaacattgtaattaggaaaatttagtgcagaaggaaagtgttcccagattccctggggtctggaaacatagtgtttattctaattacatgacacctccactgtgttttggggcaagttactgtttctcttttgagtttcaatttcttcaagagcaaagaggcagaggagagctaggaagatcgtagctgctgtgcccctgtgccgtcgggtgccttctacctgctgcctccgaacctttacacatgtccctgctctgcgcgagggcacagatgggatgcactgtggcaggggtggggttagagtagatcacggacacctgttagcttgatgtgtgcttgctgtcaaggttgaatcatgaattattttatgttgcttatattgatatgtatcttaattttaaaagaaaggtctaaatggatgtttttgtttttagggaatcagaggcaatcattccaaacatctttttcttcttggtattactatcttatgaacgctatcattcaaaacagatcattggaattcctaaaatcattcagctctgtgatggcatcatggccagtggaaggaaggctgtgacacatggtaacgggacacacctttcactgtcgtcttcggtgtcgtgatgtgcttggcagtgttcgttttcatatacccactttgaacgttgtcagtggcagccatgtgcttctcaggctctgcatgtgtgtctgtgtatgtgaaggtactggttagagacgtttcaaaagagaagagagcatattctttactctcagcaatttgtaatcttctcagggaaaaaaattcaagaaacagtaagataacctaaggtacagatagattctgaatataaagttcctgttcattcacatgaaacgctaaaagttcttcacttgatcttagccaaaaggccaagaagcgatgcaacactaaaaattcttaaatcgaacttgccgtgaattaaattttgatctctcatccagtggtattggagatatagtttgacttgggttcagggctttctgttttgcctgatgattttgctggagcttaaataaggaacccaggagatggccagctgtgcaagcccccagcctgtggaaggagctagtgtggttttatgaatgagttgcaaatctttctttgagctttttgaactgatcttccagcattgccctattgacccctccctgactcctttgctggaatctgtaggcttttgaactttgacagggacacatcctaagacccttgcaaactcccagatgtgagaatggcactactacttagagtcttttcgactcagcgtgtgtgcagaagagcatcaaccgggctgtgttgcgaggcagggccttggctgacctctcagtgtttacatagctaagccagttagtgtttgccacggcctcacaagggcttcagattcacacagccaaagtatagattattaaaggcataggtgtttggtttcctggacttggagggtctttggacagaaaatcagtaggcaaccacacccagtactttgtgctgggaagcttggtcatctgtgagagggtcagagagtatacccatgcgtgcatgccaccgaagggtcagtgagtattcctgtgtgtgcatgtctcagggccggagagagtatgtgtcactgagaggtcagagtgtttgtgtgtgtgtcaaagagggttgcattgtgcccttcactgaggggtcagagggtgcctcgcgtgtgtgtgtgtgtacgtgtgtgtgtgtcactgaggggtcagagtgtgcctgtgtgtgtgcttgtgtgtgcgtacatgtcactgaggggtcagagtgtgcctctgtgtgtgtgctcatgtgtgtgcatacgtgtcactgaggggtcagagtgtgcctctgtgtgtgctcatttgtgagcgtatgtgtcactgagggggtcagagtgtgcctctgtgtgtgtgctcatgtgtgagcgtatgtgtcactgagggggtcagagtgtgcctctgtgtgtgtgctcatgtgtgagcgtatgtgtcactgaggggtcagtgttcctatgtgctcatgacattgagggtcagagtgtgcctgtgtgccaatgaaaggcatttcttatatttttttatatgtggtcatagtagaccagttaatttattttgactcctgtgttagaccaaaataagacttgggggaaagtcccttatctatctaatgacagagtgagtttacttaaaaaagcataataatccagtggctttgactaaatgtattatgtggaagtctttattgtcttttcagatgaatcaagtagattattcttgagaccaggaatgttgctgttttggttatttggaaagttttatcattttcaaattgacttttgaatttgagtcaccttttttcagaagtggtgttaaattataggagccctaggttttttttctttttttagaagtcatcacaaaatgatcagtgttcagaggaagagctttgaccttccacatggtataatgattgataaccttaattcatctcttaccataaaccaagtatgtgtaagggttttctttatttcttgaaagcattttgtagatgttgagagcagttttccaaatgtaatttccatgaaatgcctgataagggtacccttttgtccccacagccataccggctctgcagcccatagtccacgacctctttgtattaagaggaacaaataaagctgatgcaggaaaagagcttgaaacccaaaaagaggtggtggtgtcaatgttactgagactcatccagtaccatcaggtaagaggaatgtatgttggaactgtcgtggatactttattgacccgtgcagatggaaggaagtgccatgtggtaacgctcactgttaactgtgttactttgaaccaggtttgggctttctggggcctgggtagatgccggtgcagggggatggggagggaggcggggggtgggggggtgtggtggagttggggaggtgcagtggcaggaggtgttgttggtgtgtatcctttttttttttttgagatggagtctctctccgtcgcccaggctggagtgtggtggcacgatcttggctcattgcaagctccacctcccgggtttaagcaattctcctgcctccacctcccgagtagctgggattacaggcatgcaccaccatgcccagcaaatttttttttttgtatttttagtagagatggggtttcaccatgatggccaagctgtttcgaactcctgacctcaagtgatcctcctgccttggcctcccaaagtgctaggattacaggcgtgagccaccatgcccagcctggtgtttatctttaaagtgggcacagccacaggagttcacctgactcctggtctgagagtcacgagatcgttcaagatagtgaggccctcttttccaaaacgaggaccaaaaatcaattgacagtgttggtcaagatggtagaaaccttaaaatgatagaaatctcaactctgaaataaaaactttatttgtatatttatttaccactattttgacatagggctaaggtctttttctttgagctgatttctggttttgttttcttaaagtggcataagaattcaaagacattttgaggaaggctgagtgcagaaatctctctttttaaatgacttctcctttcttttaacttgcactgttgtctagccctcacttattttgtcaattctttttagctgtttgtctttgaatcttcataaagccatagcttttctcataagaagcagcactttctttgttcattcatattttaatgaacccctgtagtatttaattaaatacttaatgcctaattaaatcacataattgcaatgcaaaagtacatgtatcataaagaggtctgaaaatgagcaactggcaagcaggtggtggcaggcagagctgcttgggtgggtgggtgtcatggagaggagttcatcagccacatgttcagtgagctctggatatgtctgtttagaaatgatcactaataaacttgtgctcaaccatgtatacctctgggaagcaggtgctcttcagtagattgcctctgcagagaacacagaattgaagtgaatgtccacaaaggcaatgagccacctgcagaatagtttagtcaaggctgtgtttgaagtttgccaaagattaatatacatttgattttcatgttgtgccttttctctgattgtgaaatattacaaattctatacaaataacaatgatggcaaatcctcctgagcaaagtgtgcaccttgtatgtgccctagaggaacttgtgtttcgttctgattcccctacatttctcatgtcatagagtgggggttgcattagtgtccccctgtcctcgctgggatcacatctgtttggatcctagagtcttccagctgaactgggacaagtataacagacggacacgtaggggtggaaaggcgtctcttggcagcagactttctaattgtgcacgctcttataggtgttggagatgttcattcttgtcctgcagcagtgccacaaggagaatgaagacaagtggaagcgactgtctcgacagatagctgacatcatcctcccaatgttagccaaacagcaggtttgtccccgcagccttggcttgttgttgcatagtgatggtagcttaaggtccttgtgaaaggtgggtggctggaatcagctcttccttcagtcctaatctgtgccttgatagcagttctccgtgctagtcatgggacagctgacttcatttcttctcacaatgccatctcaggttggtattgcccacctactttacaggggggatcccacagctccgagaggttatggaggtgatcaggcagcacacagctttagagtgctggggtgagggcgggccaaggctaactctaaagcccgaacccttacctcctacactgcctcctgcattctggtcaacccagtgttttatttggtggttagatttttgtttttgttaccttactgcttgtaatttagcagttttcctttcctttcccttcctttcctttccgacagggtctcactctgtcacccaggctagagtgcagtcgtgtaatctcactgcaacaacctctgcctcccaggttcaaccaattctcccacctcagcctcctgagtagcaaggaccacaggtgtgcaccactacgcctggctagttttttgtatttttagtagagatgaggtctcgctgtgttgcccaggctggttttaaactcctgggcgcaagtgatccaccaaccttggcctgccaaagtgctggcattacaggtgtgagccacctcgcctggcctattcatcactaatcagaatttctatgatcaaatgacatgaatcattgtttccacaactgcagtggaaggaaatggcctggcagtgccagtttcagaagcagcctgcccccagtcaggcacaggccactgtgcccccagtgtagcagcacctctgtagctcacagagaagggtggtggggacctccttgaggcagctctgccagaaaatctcatgagctgcctggcacagcttgaggttgccttttaagtggactcagcaaatacatgtttgttcatcttgattatacacaataaacaactactctgtatagtacgagtagtccgtggtttttggcatttgatttaaacttagaggcatgtgatattgatgttactgccttcatgactgcacccccattctgatttcataatggaatgttatcttgagaccagttagacaacaggacagggatcttggcttctggtgagattgacagcagttttagtgtggtcagggtctccctgcctacagatggttttagaatggtgccctggaagctttatcccattcttttctgtgcgtaatctgagtagagtggagatcgaaggcctgaatacatagtaaatacctgacttaatatctgccgcaatggaaattgtgtgatacaacatttatgaaacgcttagtgcagcacctgccaggtagctcaccacaggtgcatgttgcattcagaagtagtgctagatactatcctgttactggcagtgcatacatcagtgatcaaagcagattaaagaaagaccccctgccttcttggagtgaagattttgttgggatgcgggtaaggggacagacaatagaaaagcaagtgagtgaagtctataccatggcggctgatcaggaacaccgtacagaagaatccaggagggaagagagttaggtggtgtctgcggtgggagtggcattgttcagctggtgatgagaagaagctttggtgatctggtgacatttgagtgaatttgcagaaaggaaagatacaagcctaggagatacctggggaaggaacattccaggcagagcaaatagcagtgcaaaggccctggcggggggcggacatgctgttagggtacaagcaatgagggtggaggagtggggcagccatggggagggaagggagtgaggcctggtggggtgaggccagtgtggaggagccttgagagggtttgcgctgatgtggtgtaggttttagcaggatcattcttattcctgagttgagaatagccttgagggggaggtgagggcagagcagggccacccatgtgagacccggcactggagtggaatggcccaagtcagcatcccttggcagcatgaaagcaaaaccagcaaggtttgctggtggcttagatgtggcatgtgagagagagcagggctttgggggtgatttcagggtgaggacagggtggctgtggacaaggtagggcagacattgggggcagcaggaggtcagagcctgtctggatgtagcagttgagaccccataggtgcctaatgaggtgaggccagcatcaggtgtatgagcctggagttgtcgagagactgtggggcagggggtcagcatctgagatgtccactcacagtggacccagactggctggagaggaggaggagcttgaataccgagcctgctgagtcccagctccaaggtcaggtaggtgaggggagccagtgctggggcagggggagtaggcaggtgtggggttcctaaagccaagattttttttaaggcattttgtgcaggagggcgacatctgctgtcagcaccttgggaacttggcccaggtttggcagcaccgagggcactgatgagtgcttttggaggagcaaagggagccaaaccctaatgggaatgtgttcctgaaaggacaggagagagacttgggaaaaggttttacttgaagagggaacggagaaatagggcagtagccagaggaggagaggagtcggcaatgggttaagttggcagaaatgaaggcctgtttacgcactgagggcagaagcaacagggaggatcagttcatgacacaggagacacaaatcgccgttgtggtgttcacagacatgggttaggattggctgcatggatgacagagcactgtgggttctcccagagttgctggggaggaggcagagttggtgagcacaggcgagggtccaggatgcaggaatcctggagctcaagtcagttgttcccttgttgtaagatgtggccagtgttgtgagcttcacatctgtgccttgaaaaacaccacatctgtttgcagagttgtttactatgtatacacactcagtagaaacaaaaattggaaacagtcagtgcccaccatcaataagtaatggttgaacacactgtggtataagcttagactattttagcttgggctattttgcatgattaaaaatgttctggccaggtgtggtggctcatgcctgtaatcccagcactttgggaggccaaggcaggcagattgcttgagctcaggagtttgagaccagcctgggcaacatggtgaaaccctgtctctactagaaatacaaaaagtagctgggtgtggtggtgtgcgcctgtagtcctggctaactcaggaggctgaggtgggaggatcacttgagcccattcgtgcgccactgcactcctggggcacagagtgagactctgttagaaagagagagagagaaagaagagagagggagggaggaaggaaggaaggaaataaatggaagaaatggaagggaggaaggggagggaggaaggaagaaaggaagttcagccagttgccttgggagttctccattgcactgggttaagtgagaagagcagagacgtttatgatttttcaaaacaactaaaacaaaacctctgtgggtgagggggcaaggatatggctataggaacatggggcagattaagaaagggatatacacacaccacttagcatttgttacaactgttgtgggagggatggagtgcagaaaaagaaaaaaaaaagtgcacaccatcccatgtatgtgtatacaaagggacgcttggaagactggtccccaaaatgttggtaatgattgtgtcagggtgctgcagtgctagttgattttttttcacacttttgtatatttgagtcttttacagaaagcatttattatttatgtaataaaaatctaaatgacaagatttctgttatgggaaaaatgtagctatacagtgttgttgtaaaaatgtttgcttggttcaccactgaacttaaaatgcttttaaatgagggaaggtgacgatgagatgattatgatgatttgcccttgagttacatagctggtgtacaggaagctgtcgtttcttttggcttacgtagaaatgtttgtggtgtctaattccacagatgcacattgactctcatgaagcccttggagtgttaaatacattatttgagattttggccccttcctccctccgtccggtagacatgcttttacggagtatgttcgtcactccaaacacaatggtgagtctctcgcctggctcagcagatgaatctggacggcttgttcaggctctgattactgggaccacccccagaatgtctgagtcagtcagtttgggtagggcttcttgagagtttgcttttttttttttttttttttttggtgtgggggtggtgcggaacagagtctcactctgtcgcccaggctggagtacagtgtcatgatctcggctcactgcaagctctgccttccagcttcacaccattctcctgcctcagcctcccgagttgctgggactacaagcgcccaccaccacgcccggctaatttttttgtatttttagtagagatggggtttcaccgtgttagccaggatggtcttgatctcctgacctcgtgacccgcccatctcagcctcccaaagtgctgggattacaggcgtgagccaccgcacccggcctttttattttttttggagatggagccttgctctgtcacccaggctggagtacagtggcgctacctcgactcactgcaacctccgcctcccgggttcaagcaattttcctgcctcagcctcccgagtagctgggactacaggtgcgtgccactgtgcccggctaattttttgtatttttagtagagacggggtttcactgtgttagccaggatggtcgcgatctcctgaccttgtgatccgcccgcctcggcctcccaaagtgttgggattacaggtggctctcgcaccaagccaagagtttgcatttttagcaaattcccaggtgaaactaatgcctgcttttctgggagcacactttgggactcagtgatagagaggtttattggtaggatagtaaaataggagttattttctttcacaaaattggcaattgggggaaatttaatcttccttttttcttcagctgtgacttatgtattatgtttattttaggcgtccgtgagcactgttcaactgtggatatcgggaattctggccattttgagggttctgatttcccagtcaactgaagatattgttctttctcgtattcaggagctctccttctctccgtatttaatctcctgtacagtaattaataggttaagagatggggacagtacttcaacgctagaagaacacagtgaagggaaacaaataaagaatttgccagaagaaacattttcaaggtatgctttctatctgagcctataactaacccatgccttttgggaagtcacgtgatgtttcacagtcagtaagtctggaataatacctggtcttgcttcacttctgagttgggtaaagaagtctgtatcagtgtaattttctaatccgtcctgcattatctatggctcttggttcatacctgtcttgaagttctgtcatgttctgtctcttgtcctcagtagagatgctacagcagtggctcgcctcaggcagggcagggcagtggggtggctgtcctgggggcaggcagtaggggcacgctgacgtcagggaagttgaaacccaagagaagccagtaaaagtgagtctcagattgtcaccatgtgctggcagttttacacgctgtcagtaataaaagtcttctccctgcagggcagcctgcctccaataaatacgtgtagtatcaaatcctgtcttccctcataaattgtttggaagctccccaaggacagtgatgaggcactcgtaagtgcttgctgcctagatgggtccctctccacctttgctagattctgagcattcactgagttagagctgcttctgcaaatgtgctgcttctgctaagtggctgtgacttcatgcagccttcacttggtttgtcatcagtggagatgccctgtgttgtcgaaggagataagcccagtaagcctgctgggcaccttttggtttgcaggttcagcaggcagcccatggctttccctgtgtcgcattgaagcagctggctaaaattgatgatacattaaattcctgtgacagatgatcagcttgtatttgtgtaatggtgtacagttcacaaagcttaaaaaaatgctacctgccatttcatcctcagtgaggaaggtgatacacagagagaccaagtgactgtgtccacggcgacggcgctctgcatttcactttagcggttaatgtactctacctatatttttactttatatttaccatatatcttttcatgtatacttggcgtaagtgctttatagtagtcacctaattcactgtcatcttttttgtttcttggaaggtttctattacaactggttggtattcttttagaagacattgttacaaaacagctgaaggtggaaatgagtgagcagcaacatactttctattgccaggaactaggcacactgctaatgtgtctgatccacatcttcaagtctggtaggtgaatcacattagtcttcctggagtgtctcgttccccattctgcactatacactctcagagtgtaggagctgtgctgcccggtagaaactctgccttgcccagtgtgccagttgaaaatatttgttgctgtaagagtacacctgataccatgtgacccagcagttccactcttgggtatatacccaaaagaatggaaagcagggtggtgaaaagatatttgcatgccagcattcatagcagcattattcacgatagctaaaatgtggaaccaactgaagtgtccctcgatggatgaatggataagcaaaatctggtgtatatttacagtggaatattattcagccttaaaaaaaggacattctgacacatgctacaacatgggtgacccttaaggacattatgctaaatgaaataagccagtcacaaaaggacaaatactatgtgattccacttacatgagggacctggagtagttaattcatagatatagaaagtagaatggtggttgccaggggctgcaggggaggggagttatttttacaagatgaagagagttattctagaaatgaatggtggtgatggttgtataacattatgaatgtacttaatgctactgaactgtacagttaaaaatagttaagaggaccaggtgtcatggctcatgcctgaaatccaagcactttgagaggccaaggcaggaggattgcttgagccaaggagtttgagaccagcctcagcaacatggtaggaccccatctgtacaaacaaactagccggggatagtggtgtgcatgtggtcccagctactcaggagactgaggctggaggatcgcttgagcccaggaggttaagtctctagtgagatgtgttcatgccactgcactccagcctcggctatagagtaagaccctgcctcaaaaaaacaaaacaaaacaagacaagagccaaaaatggttaagatgggccaatcacagtggcttatgcctgtaatcccaacactttgggaggtcaaggtaaaaggatcacttgaagccaggagcttgggaccagcctgagcaacatatcgagacccctatctctacaaagaaaatcaaaaactagctagatatggtgggcacatgcctgtagtcccagctacttgggaggctgaggtgggaggatctcttgagctcaggagttcgaggctgcagggagctattattgcactccagcctgggctacagaatgataccctgcctcttattaaaaaaaaatccaaaaaaaaaaaaaagtaaacctgagagcttcctcctcctgtgttaaatttggaggccaagatgtttttgttacttttacaaatgatcaaggacggtgaaggttgggcatggtagctcacacctgaaatcccagcactttgggaggctgaggcggggtgatcgcttgagcttgagaccagcctggacaacatagcaagagaccccatctccacaaaaataaaaaaataaaaaaaaatagccaggagtagtggcatgagcctgagcccaggaggtcaagctgtagtgagccatgatcatgccactgcactccagcctgggcgagatcgagaccatgtctctagagaaagaaaatgacaaggacagtgaacccaagaaagtcataagatgccagctgtgcagcaagcatggaaagcagccagtccaaattaggacagtgtgttttccaagaagaacgatcgtttgtaatgagaatgctttgctttaaataaatgactaaatagctagaagcctagttctaggggataggcacgtctttcttctctcaagaaaatagaaaggcaattctaatttctagtaacagcaaacagcattaagtcatggtccaaatatgaggcaaaccaaaatgtggcttgattgttcagcagttgatctgttggaagcccttgatattaaaaaggttctcctttaagcggcttaggagtcacgatcaaagacctatagaaagagatgccatccttctaggatccttggctctcttgggaactagattcagatagtcataatgtaaatactgcttgagctttctttctttctttctttctttctttttttttttgagacagagtttcactcttgttgcccatcctggagtgcaatggtgccatctcggctcaccgcaacctctgcctcccaggttcaagcaattctcctgcctcagcctcccgagtagctgggattacgggcatgcaccaccacgcctggctaattttttgtatttttagtagagacagggtttctccatgttgaggctggtctcgaactcctgacctcaggtgatccacccgcctcggcctcccaaagtgctgggattacaggtgtgagccaccgcacccggcccgagctttcatttttgaaatcaatgtatgactgaaacactgaagacttactgacttaattatggtttcagaacagaatgaaaatgtcttcggttctgatgaatataaaaggaaaactaaccaagttaatttggcaagtagatggtagagatagaggtggggagtggaaggggaactaaaatcttcacctagcattgttgggattatatggttacatcatctgaagttgacagaccaaaatatagaggcttcagaggtctccaaatagaactaaacatgtaattcagattgttaggaggtagtataaatgagctaaatctcatctttattacggtagagttaatgggtgatgtctaaagttgtctgaagtctataaatcatgacaaattatgatgtggtgattgtattcaacagtctttcagttgcagggataaaaccccagtttaaactagagtaagagaaagaatgtgttggtttaagctcctggaaagtgcaggcaagggtagttggtaggactgcatctagtgttgtaattctgtggtctgcattgtatatttatgcatctcagctctgctttcttcttttcatttatataatttttaaattttattttaaagatagggtctcactttgtcgcctaggctgaagtgcagtggcatgaagtgcagtgcgaggctcactctagcctcgaactcctgggctctagagttcttcctgcctcagccttctaagtagctgagacaataggcatgtaccaacatgcctggataggttttaaaatttttttgtagaaatggaagtcttgctgtgttgcccaggcgggtctttaactcttagcttcaggcgatcctcctgcctctgcctcccaaaatgctgaggttataggtgtcacccaccacgcccagtctcatctctgcttcctgtgttagttttgttctctggtgggctgttttcacatgaccgaagatgacctctagcaggctgtgttctcagcccctcaagtaggcctatgtgattggccttgcatgagtaatatgggtgaccataaacccctgaatgctctggtccacatgggccaaatgggagactggacagcattccattgatgaggaggtggggctggtctccgggagtaagggagaggagcacatgcagtaactgatggtctgctgcaagggatagcagcacagcagttagaattttggaggtaactaccagaactgaaaacagaaatgataacaagtagttgccttaaaaagggatgggagcagggtgcttttgtgatcaaagctcctttctcttactggatttttgtacacattttgcatacatatcttagagtaaaagatagcattttcagccttggtccatttgaggatactcttggcgtggcccgcctccatgctagcaggctctggttgtgccaagttcagttgagcatcctggctcttgcctgcacggaacttccagtcagtgcgtcagtatcacaagtcttgatatttcctatgaagaagaacagtagtgcagtgacagacgaaatgggtgggcaggcagaggcaggatttctgagggagagaagtagctagctttttgcagagaagagttccggcacccaagagagcagctgagagtacaggcaggcaggcaggatgccggtagggcccggccgcacggcgccacagaatcctggagaaaggggcctcttcatggcctctgcattcagctgctgtcaccctccgcacaggccatggccaaaatttaattttcatagtggactctagtttttgagccttacttgctattattgaaataattttcttgtttctttttaaagatcttcggattatgcttcactgaccactgtaataagtttaaagttgagaaaatatggcttgttaatgaatgataggtcaattttagtatgttggtcattttaatattttgccaccagttggtttggatttgatgccaggaggagacagcctcatttctaaggactagtcttgcctttgtgggataagggtggtgtgttctgtgtccttctacatgtccgagcgatctctgtgcagctcaaatgtggtcactgtcttattgcgctgatttcctctccttccatctcacaattgaggcaaaatattgttactgttgaagtgttgtccaataggacttccagcagagacaggatgtctgcactgtctaatttagttgcctttagccacatgtggtgttctgtacctgaaatgtggctggtctgattggatagcttaatttataattttatttaattttaattaacttaaatttaaacagctctgtgtggatagtggctcctgtatgagacagtgcaggtctgttgagaagcagctttactggtgggagtggagggcttggagagggcacgtgggtttcctgctggtatcttttgaccttatttaatctgcccaacatttgcaagtaagttgtgtgtgtgtgtatatataaatgtgtgtttctgtcttcttgtttcctttgactgcatttatttgaaagacactaggtggcagaattactgtatttgattggtttcaagataagagttgaaataattcatctcgtgtttttatataagtaaggtgtgtttagcatgtaaaattggtaatatgtattcacgtactgcttaaacaaaggctatgaattccacccataaaccgaaaatgaagacctttaaatttgtccatttcaggcgtgggtacttcttaaataatacctggttcaggaactagtcagaatggcacccttgactttttgtttcctgcttttcctcttgttgggagaggagggtattcatcccaaagtggtttgcctatttcacattccatctaggataagcagaatagccaagaaagatagctgtcctcctgtttacaacatttggggtaaccagcatccctctcttttggtccaagatagactggtttagaaacagatgatggcaccagaggcccaggaggtggaaacatcagctttgtttgttgtccatgtggctgaattagagctgtctggccttgtagcctcaacacggccttccagctttgctcaccgtgattttcaaggacacatcttgtgctcttccctgcctgccatccagactatacccagtcagggtggcaggagctgctgccccttcctccctgagtcctggtcgtgggtggtggagatgtgccatgacgctcacggaggcatgctcaccccttcctctgtggcagaggggatggctgcacgacagctcttccctgtcctttccaaagcgtctgtggttccactttttggggcaaagcaggaatactggaagagagagaaagtggtcctttctatagtaataaagttgacattgattcaagttcatgcttggggaaaggacagggctactaacaattataatgctgggagcaatggaattttctcatgggtatgtggtaggtttaattttaattatcccagttaattcttagaactgctctgtgaagtatttcccgctttgtgcttaagttctaaaagatcctgtgccaaaaccaagaatgaaaacccaagcattctttcttgcccatcgatctttctctcatcaggccacttcttgggttgatagtggtgagtgtagccgctgccactttcagaatacccaccatgggccccagtcactgtgtggcgtggagaagagatggttctctctgtgtcatagctgaacaagcccagcccagagaggtttctgccctaggagctctcgatggtggaattgggatgcgatcccacatcctgcctgttttgaaaacagcattctttatttccaattcctgcttccattgttccttttaatatttctttgtttagctcacaaaaacacggcttgcggagctgctgcgtgcagctgtagctgtttctctgggtgcagcctgcatccgccttcctgcccgcctcctttcctgcactgccatcgtggtctccgggcacttggtccctttctcttcccctgagtccctttggctcccctgtgccacccttgtgatccacaggctctgccttctttctgtctcagactgctgctcatcactactcgggaccctaggaagggaggttccaccgagaagcatcttctcatctcagccacgttctcagtgccactgttgtctttgttaggtaatggtagctactgtaacaaataaaccaacatttccatggcttcacaccagagaaggttgtttcttggttttatgacaatgtattgagggtgttcttggttcacggatggttttcctccatgtgggaattcggggacccaggctcctttccttcttttggttctgttctccaggccttcacatcctctgtgtctggttggggacaaggagagggaaggtaaagaaggctttgtggccttggataagtgacaggcatgcctttgctggtgttctctcgtggtgacaggtcacagccccaccctgtaaaaggggactgagagacgtcgtcctgctgcttcccagcagcagcactgtggtctctgatgtgttttctgtgaggataaaaacaggtgattccaggatgaggaaagtcagggaaacccttggaaggaggggaccaggcgggtgtcaccatgggattagtggtggcttcagaatgagctgcagcgagtgccatgccttctaaagcttttgctattctgatatgcccacaccatgcccagcaggtgtctgccttgctctccgcagagagagtgatgaatccttctcatgagcctctgtccagttgttcctccctccacctggaagggaccctgggttcctcataacatcccagcggaacaggggaccttctatcctgtccccaagttcatcctcatcctcctgccggcttcctggcccctcttatgtctgcttcctgacgccacatccttctggattctctggaattgaattttgcctttgatgcttatttaaaaatatccattgcaggccaggtgtggtggctcacacctgtaatcctgtgcactttgggaagccaaggtgggcagattgcttgagcccaggagtttgagattagcctgagcaacatgttgaaatcctgtttctatagaaaatacaaaaattagctgggcatggtggcgcacacctatactcccagctactcaggaacctgagacaggaggatcaattgagccccggaggccaaagctacagtgggctgtgatcgtgccactgtactccagtctggtcaaacagagtgagaccctgtctgaaaaaaaaaaaaaaatccattgcatacttcaccgtagcgaaacatgtatgtcttacctttcctttcctgcctgtagctgctcttttacacttaacagccacactaagccagccttaaatgaaaaacaaaccagcacttcctgtgccctcctgcttccttcatgaggggtccctccctctgtgtacactccattctcattgcccatggtggtttgtttccctcttgtttctcaagccatggcagcctgcctcttgccctctttactaaaaaggcctttgcagaggctgcctgtgttctttctttctaggtctctctcatcctaggccctccagcttgattctgtggagctgccctcttgtcactcagtagcttgtggggtcttctctgtctagccacttaattgattgtgttcctcgagttgctgtccatggtctctcgttactgttttctctgtgtttctgcctctctccttggccttggtaggtccatcccctttgtgaccttggctgttgctctcatggacaactttctcttgctggtccttgtagtcctggcatccagcttctcgacacgggacttgtcctgccagtacctcagacttgcacttaaaattgaactagcaccactgtcactctccagggcctcttcttgttaattagatcattagggatgttcagaatcccagcatcatagtatgttcctcctcccgctaccccaggaaccctaaccttacctcctcctctctatctactaggaggtggccctcagagtccgtctcatcttccacctgaacttccctaataggctccagcagctgccaccccgggggctgagtacttcctccatgccttgtgcagtgctgagccctttacctgggttctcctgtttgctccttattacagccctgcgaacagatactgctcttaattccatcttacacctaaggaagctgaggccccaggtaaggtgcatccaaggtcacccaggtagtagacagtagagccacgatctgaaccaggcagtctgattcagagcctgtgttgacactcagccacctagaacacagcttggattgtgggtttctattacctgttcaaaacccctacatcccgggtctgtccctgcacgtgctctgtggcctggctgcatcttccttgaaggcagtgcatgcctcttcactcagggggcccatgcaggaacagagggccccacagaaggatgaggccagtgcagaatgggctggaggggacaatgctgaccaggaagcaagtgtagagaaatcccaggaaacctggaggagccagagacaaggcattagaactcctcgtcgtgacctggtctgcattctctgagtgtgctgcttctgttagctcgcttccttggtctcaggttatagtttaaggcattgtggagccctaaaaagcctgtactctgtttttacctgttttaggaccctttcactttggggatgtgttgattttttttttttttttttttttttttttgagatagagtctcgctccattgcccaggctagagtgcagtggcacgatcttggccactgctgcccctgcctcctgggttcaagcaattcttgtgctcccgcctcccaaatacctgggattacaggcacccgccaccacactcggccaatttttgtatttttagtggagacagggttttaccatgttggtcaggctggtctcgaactcctgacctcaagtgatctgcccaccttggcctcccaaagtgctgtgattataggcgtgagccaccacacccggcctgaaatttaaatcagaaataaaattttgatcccaacagtgatgccaggcagcccagatctgggggagagggtggccttggccagctgggcctttctctgtttcccaagtcttgctgcctctccctgctgggctttgcagcctgtgcatgtctctgtgcctttgaccttgtttatccaaaggagaggatagaatgaagtcatgattcctggagccctgagaaggatgctgtggagaaatttgccggtagaatctagctgagtgtgttgctgaggtgccagcattgtgtgtggggaggctgaccgcttggcctgcctaggcccaggatgctccatggccgggcacagaggccacttggctgtcaggtgtcaggagcctgcagagggcacacagagcctggaccgcaggggggtcctgctttctcacctggcctccttcagcatttctgtccctcagtccttagcaagcccaggagctgttgagtttggcaggtgccgagtgctgttcctgcctgtgtagctgtggctcagtcctgtgggggccccgctgtggcccgagtgcagtgattcgaggcgctgagtgttccctgactccttctccaggagctgtgttcagactttcgcagctcttggcttggagctcctggagggcttggcattgccgaccaatgtggaggtcgacagtgagagaggaggaatgctagctttcttgaccagtccattaaataagtgggatattggccaggcacggcggctcacgccttaatcccagcactttgggaggctgaggcgggtggatcacgagctcaggagttcaagaccagcctggccaacatggtgaaaccccctctatactaaaaatacaaatattagctgggcgtggtggcaggcgcctgtaatcctagctacttgggaggctgaggcaggagaacagcttgaaaccggaaggtggagtttgcagtgagccaagattgcgccactgcactccaacctgggcaacaagagcaaaactctatctcaaaaaaaaaaaaaaaagtaggatatctgtttctgcttagaaaaatcagaattttctaaatgccaggtgttctgaatacgtaagtatgggagacgactcagcctgtttcatttttatgtaaaatcttcgcgtagccatgtggcactggaccgagatgaaagcaaagacatttctccttaactttgtttctaggaatgttccggagaatcacagcagctgccactaggctgttccgcagtgatggctgtggcggcagtttctacaccctggacagcttgaacttgcgggctcgttccatgatcaccacccacccggccctggtgctgctctggtgtcagatactgctgcttgtcaaccacaccgactaccgctggtgggcagaagtgcagcagaccccgaagtaggttcataatgccccacagcccagggcgccagcccagcaccctgtcctgagactcccagtaacctgagctttggccaccgttaaagcattttcattttccattttttgtgagggcttgtgaaatttctgctgcatattaatattcctttcatggacagcatattattgggacaaacatgcggtccagctaaaggcattcaaaatagcagttgctttctaaatgcgattttctttggcaggttctttgacaccattgcatcttgtgggatatgcttgtcatgctctgtggctcctactaagttctagtccttaaattggttccatagccagacatgttgcaatgtcttaacctcattataaagtaaatgtggttctggttatccttagataatgaagtaacagtgtagcaaatttcaaaacctcttggaaatgttattttaccattcaaaaaggcttactaaggttctcgttatgggtggccctctttttgcaaaaggttttcaggcttaagctccatttctaggtgctccaacactccattatttgtatatgtatggaaataaaagctgtgaccacccccaaccctggcccccgcccagctgaatcctcagcacagtatttctggaaggctcaagatcccacgctggggaaaagaagttctggagacaaaagagggcaggtgctgccgtgcctctctgctcagtatggatactggaccttgtgctgccagggctcccagtagggccagttcatggcactcagctggaaagtccactgttgggaggcattcttaaccatccactctgtgccgtatgtagtggggtctggtcattctgttggaggagacagaccagtgacgacatttgaaatgcttggtggatgtcttaggcctgttacgatgactgagcactgtgggggcaggagacagaaagtcagtgtctcctagttctgtgctgctttaacgtgcatagaaatcagctgcggattcagcagatcactccttttctgacagatgggcctgcttactctgatgttatatcagaaagctctgaatctgggaattgtgtcccctgaattggagtaacagaaatgcttagatgatgagtgtttaaaagaaataaaccaaaggtaaatttagtttggaattcagcaagcgtcttcattcagccctctgagggcaaactacagctttttgtaaatgtaggtaaattctgtgactgtttcgtgaccccctctgatccagttttcctttataaccttctgtattgttccttctattatcctgaaataacattaatagattaggctgggcgtggtggctcatgcctataatcccagcaccttgggaagccaaggcgggcagatcacctgaggccaggacttcgagaccagcctggccaacatgatgaaatgctgtctctactgaaaataacaaaaattagccgagcatggtgacaggtgcctgtagtccctgctactcagaaggctgaggcgggagaatcgcttgaacctaggaggaaaaggttgcagtgagctgagatcgcgccactgcactctagcctgggtgacagagtgagactccatctcaaaaaaaaaaaaaaaaaaaaaaaattaatggatcaatggatttttaacctaataattaaatttcaaaaaatatcgttctttaatggtaatgtaaaggtaaaattaagataatatgtaacaagcatgtgagtgtctaaggtgtccccgtggtggaaggaaaaaataaatccccataagtgtccaagatgcccatagagagcagagctgttctggtttaaacccctgctcttagcactgtgtttttccagctgtgggtggtgggggatgagtatctttttatttccatgagatgagaaaaatgaattactagaagtgtgaaatacaaaacacagctgctctttttttagccatagactcagcagccataaaattgctgtatccagttgcagaaattcctgctgcttactcttgaccctctctcggtttgtgtgcatctcctctcaggctggctcccagatgggagctggctccaggcgacactgggtgctctgctccaggaggtccttatgtgggtcctgccctagcctagcccctctcttatggactctgtcactgtgggtttatgattcactctcaatctgtcttacctcttggtgaactgttagagtcctgcctatactttggcgcttgtgggtgtgttgtggtacacatgatgtgttggtcacttcccagctcatcttgttctgagtcaccctagatttgggacattcattcgccaccagtaccgggcggtgtatggcctgagatttgggggggcttgtgctgctacaaattggggctgaatttgagttgacagtggaccttctttatgtctactgctcatatttgaattgcaaatactgcctcttctctttcagaggctcattaccctatagctgtattattgcaaagtgcacaattacagcttgagtgtaagtcacactgcgctggcaggacggcccactgagaaagggcacgtttcctgttcgttagttttcacattgacacataatttacaatacagtaaaatgtacttttctatcaactgtagtcagtaacagcccccctcccccaaccacatcaagatatagaggagtgctgtcacttcaaacagttccctcttcctctgccacatcctgcccctccccaggtctaaccaccaatccgtgctctgtccctctgttcagcccattgcagaaggccatagaaatagaatctataggctaggtgtggtggctcatgcctgtaatcccagtattttgagaggctgaagtgggaggatgacttgaggctgggagttcaagactagcctgggctgcctagcaagaccccatctccagaaaaaaaaaatttaaaaattacaatcacgtccctgtagttcagctgcttgggaggctgaggcaggaggatcacttgagctcaggagttagaggttacagtgagctatgatcgtgccactgtgctccagcctaggtgacacagcaagacgttgtctctggggaaaaaagaaagaaacggaaccacgcggtgtgcagccttctgagtctggcccctttcggtgagcagtgtctaaagttctgtcgcgtgttgcccacgcgtcggtggctcgctccttgcaactgctgagcattgtatggctaggctgtagtttgttttcacttcaccagttgggaaacagagaaaaggcactttttaaaaagtttaaatctgtagaattttggtttttaccagttctcttctaaatcctgagggattacaggaaaagttgttgtatttcagaatattcttagcttgatgtgacctctgtccccgttaaggccctttgccgcaatgggaaggacgtcgctcggtcagaccctgaaggtcagaggggcagtttgggagtgtgtcaacattttaactgtatggactagagccaagagtctcaaggtttataattcccacgtattcaaaaagaaaaaaacaataaagtgagaagtcagtgtagagtgaaataacctgtgttagtggggaagaagtgtttttaaacaggatttccataacgtataacatcaacatgtttagagtggtgatgtttcattgggaaacgaacagtaaaacatgaaagcagggaggttttcattctggcagttggcaactttcacggcagatggagaatttcaaaagcaattgctcaattatcaaacatagccagtgtgagttctgaaataaaggtgctgattgaatgtgcagctttatggtggattttgctattcaggcaagcattttaattttctgcctgttaaattctgttttctttagtttttcatatgtggtttattgtagcttaggaatagataactgagagtatatattacacatacaacattctgatatggcaatatttaaaacaacttgtctgttttagaactagaattaaacataatcatcttcagtattttgcaaataagctcactgccatccagaaacattgtcaatgcatctgttgctccttctagaagacacagtctgtccagcacaaagttacttagtccccagatgtctggagaagaggaggattctgacttggcagccaaacttggaatgtgcaatagagaaatagtacgaagaggggctctcattctcttctgtgattatgtcgtaagtttgaaatgcctgtaaacggggttgagggaggtggggaccaggagaacatcctgtgtagatgacacttgcatggaccctctggaacccagaccgcccggtgtcctgccaagctccatcgaaactaaatctagaatgaatgtttacttctgctgtgacatataattggagaccaggcctggccttccagtcactggattctaagttggactgtgagagtttttgcagctgactcatttatcaaatgcccggctattggctcacgcctacatgatgctgggtatgtttgttaatttgagggaagcaatggaataataataactaatgatttaaaaaacaaagtaagtgcattgactgtagtggggttctgattttaaatttttttaaaaattaataccaggagcagtggcttatgcctaaattccagcaactcgagaggctgaggtaggaagatcacttgagcccaggagtttgagacaagcctgggctatggtgtgagacacccatctctaaaaaaataaaaaataaaaaattatccaagtgtggtggctcgtgcctgtaatcacagctctttgagaagctgagggcggaggatggcttgagcctgggagttcgagaccagcctggcaacacagagaaaccctgcctctaccaaaaaaagaaagagaggaagaaagaaaaattagcctggcgtggtggtgcatgcctgtggtcccagccacctgagagactgagaagggaggattgcttgagcccagaagtttgaggctgcagtgagctgtgactgtgtcactgcactccggcctgggtgacaaggcgagacccctgctctaaaataatttttttaagttaatttgtagaaaaggtgttagatgttctttgtcacattttatgatggattcctgtttaaatgccgttctctttaaagaaaaaaaaataacttgtgggagtttttaaccataaaactagcatcacatatttaccatggagaatttacaaaaaaacaaataaacggaggaaaataaaacctcctgtaatcatactactcagagataacttgctgttagattttggtctagatttaatactttttctatatttatattaaaaatatttaaaacatatgcatttctttgtcacaaacatggtatcttatagatactactgtcacatagcaaaacagtgttaaatattctgaatcagaaaaggaagccgactctccaactgaaagaggtgttatcctagagactttttctggtgatgacaatttattaatagtcactttttgctttactttctctattgaagtagtttttctattttgttctacttttaaggataatataatttataatgctgtttttcacagaaatataagaaaaaagatactaattttataagttaataaagtttgatcatcccaaatccaaaaatctgaaatccaaaatgctccaaattctgaagctttttgagtgctgacattatgttcaaaggaaatgttcattggaaggtttcagattttcggatttagggagctcaacaaataagtataatgcacatatttcaaaacctgaaaaaaatcctaaattcagaatacttctgatcccaaacatttcagataagggttattcaacctgtactgtcagatgatcccaaatgaaaaatattaatcgttaaccaaatatcaaggaattgatcacattttacagtttctgcctaggattatgaatcaagatgaaaaggctctgcatgtttaaaaatatatatttttattttcttataaatcttaaatatctacacttaagatttatttgatatgtgggatccattcatattttggattcaacagttctgtcaaaactgtggcagtgataggggattctttttttcccactgaactatcacaaaattggaaaaagagtaattggagaaccccactggcttagccggcccgaagcccgggagagggcaggcagtgctgtggatggggtcatcccagcgcaacgctgcccctgctacctgcggatctcgctgaggcctgcctttgtcctttgacccttggccatttgttagtgtctctgagagctggactgctgtaccctacttccccagggggcctaacttcacacagcctctgccgcagtgcgtggttggaggtgacggccttggtaaatcgagtttcctacctcctcaattatttgtgctcatacactgtatatttttagtgaggtttatatttgggatgtgttttctccttcttaccctttctggcctttctatggcattaatacctggtctcttcttgtgtacttgaaaatgaatctctcatcatatttttccttagtgtcagaacctccatgactccgagcacttaacgtggctcattgtaaatcacattcaagatctgatcagcctttcccacgagcctccagtacaggacttcatcagtgccgttcatcggaactctgctgccagcggcctgttcatccaggcaattcagtctcgttgtgaaaacctttcaactgtacgtcttcatcctgccgactattgccagttgcagttttccctgccttaaaaatggagtattgaaatttttaactttaatttctgatttgcaaaatagtcatcttttgttcttttccttcttgctgttagccaaccatgctgaagaaaactcttcagtgcttggaggggatccatctcagccagtcgggagctgtgctcacgctgtatgtggacaggcttctgtgcacccctttccgtgtgctggctcgcatggtcgacatccttgcttgtcgccgggtagaaatgcttctggctgcaaatttacaggtattgggaagagaaaccctgatattgatttatattgaaaatttagcaggccaagcaaaacaggtggctggctttttcctccgtaagtatggtcttgacatggtcaccgatagaaacatggaaacatctgcaaacttgccgttactcgtgtgtccgatctgactgtttcttgtatttttttctagtctgcccttactaggatgaactgtacacatcagttcatcctttttaaatgagcatgaggttattttgggttgttaggtgttacaaacacactaatgtgtttttgtctattagagcagcatggcccagttgccaatggaagaactcaacagaatccaggaataccttcagagcagcgggctcgctcagaggtaatgctggaaacacaggtcgtccttgtgttaggacaacccaggatataaaggatatagatttgtacgggaataaattcacaggacaagaaatcgatgtgccttataggtgggtttactgcagaagtgccataatagaaccttcctacttttaaaacaaccagatctcactttctaaagagtaaaggatgaccggcaggatcacgtctgtgacgtgagtggaggcagtttgcactcctggtggctgtttgagaggtagcatttagaatgcctgtattcactgtcctgtgatgagtgggaaaataggttatcaggtttatcttagcaaaatcaaagcatgtcatctaattgctaaacaagagttggcaaatctgagagacattactcaatccttggcatgcaggacttacatctgcatcctgttgccattttatgtcttcaaagcatttaatcatttagttgtgtttgcaaagtctttgagaagcctttgtcagaaatccctacatctcctatgtgagtgtatttccatgactgcagaataagttaaacttttacctttttccttcccttgcggggcggggtggggggcagggattgtgtgtgtgagagggagagagagacagcagagaaggagaatataattatcatgctgtgtactttgagctgaaactgcaaaaaaggaaaaacacacaaaaattattatgcttttcagtctttagagtaccttgtctattatgcttttcagtctttagagtaccttgttgatggtgtttttaaatgggattgggcacaattaggtggacagtttgggatgatttttcagtctgtagggccaagctcttttgtaatttgcattatgaagttgtcactctcatagcagatggcgggagataaactattattactttttgaccctagacttagtcttcagtccagatgagggagattaaaagattataaatatcttgtgccagatgaggtgattttattttgaaatgaccatgaattcctatcagttgtcttactgggatatttgatagtggaatttgtgcatttgagtcttagatgatctgttttacatttattaagaaagcctttattagcttttatactgtgtattgcctgttgcagtgtttgagtataaatgaaatttctggaaaatattaatggagtacaaactgtgatacttaaaagtaaactagggcctgcatttgtatcatgacctgtttgagtattgatgagaagatagctgtgaagaaaaaggtttaaacaagtgtattttcctttaagaagccactaatagtgcatctccttagagtgtatatttctagaatcctagtgtgcagagtttagactaagactaaaaaaaaaaaaaaacaaattatactgtaatttcatttttatttgtattttagacaccaaaggctctattccctgctggacaggtttcgtctctccaccatgcaagactcacttagtccctctcctccagtctcttcccacccgctggacggggatgggcacgtgtcactggaaacagtgagtccggacaaagtaagtgtccagcgtgtctgcatgggaggcacagggcgctgagtgcctctgtcacctgtggcagatacagagagtgcagaggaggtgccgtggacccaaggagttctggcgctcggctcggctcagtgaagctgtggttagagacgtggggggccatcaaggtctgagggagccaagcagtgctgatgtgggacccttttggtaggagtgtggggtgagtagttagtgggtgaatcaaggaatagtcggccgtggcctgcaggcccctgactgcacaggccttcaagcacatgtcaatgccgttagcctccctccatctcctcataccttctggccacctgtgagttgcactgccactgccagccattctggtatgttgtcagcacctccactgctcatacctcatggttagggaccacctggagccttggtagagccttggtagagccttggtactctactttcctggacaaagttcagcttatgaatatgaatttagatttcaaaaaccagcagcccaagtataagaaagcgaaggttcagtcctgccttcttaggctctattcgctaagcacctgccctgccctggttgctggggagagatgagtaaagcagacaacccaggagaggatggcaaaggggccgctaacccttagtggtttagctatatttggaaggcctattggaagttcaccaggtgaagggggaggctgtgagggtgcccaggcaggtaacagaagtccaaaggggaaaacctgtggtgtggtgagccgtatagccacagcctgccggccggcagccctctcagcctagtgcggtgttcccaagcactggcctaggcctgtagctccagggatgtgaagtccccttgaacgccgcccatcatgttccccttatccatttttttcttcccaggactggtacgttcatcttgtcaaatcccagtgttggaccaggtcagattctgcactgctggaaggtgcagagctggtgaatcggattcctgctgaagatatgaatgccttcatgatgaactcggtacggggggagcagtggaggcaaggaatcctcagcttttcttgtgacttccaagtgggatttgtctcatcatcatgtgacccacttgttgacaacacatgttggggactccagtctgggcagggacgggatgtcggagagactccactctgaatggggccgggaagtggggaggactccatttcagatggggtcgggacatgggggttatgctgatcgagacagaaaagcacattgtttcagccacattagaatccacggaggtgttgttttgaaatccagctggccccaaggctgggtgtatggtttgggatgagaactatctggcctccactggaggaacaaacacaggatgttatcatctaagctccatggccaagacagaatggaagtcaaggttgcgtatttgccgtagacttcaacacagtgtcgtaatgcgtgacgtcaataacttgtttctagtgtcttggaagttgatctttagtcgtaaaagagacccttggatgcagcgagatttcctctactcacacctctgttagatgtagtgaggttcttcaccccccaaccccagatgtcagagggcaccctgcgcagagctaggaggccatgcaaagccttggtgtccctgtccctcacccgtgggcaggtcctgtgagcagtgggggggccacctcttgggtatggtgcagccatggcccaagcagggcttcttctcagacctactaggacgggagaaacctcctggtgctttagccctgcgttgatatgcagcaaatgggagggaagtgggcacctgggaggacaaatgcctgtagaggccgggagtgacggcaggtgttcatgaaaagagaccttgtggggagggcaacacaacagtgtgttctgatgtactgaagagctcaactgaaaacaacaggagaattagcccaaaatccatttactaaaattgtttatctttttttttttttttgagacaaagtctcgctgttgtcccccaggctggagtgcaatggcgctatcttggctcactgcaacctccgcctcctgggttcatacgattctcctgcctcagcctcccaaatagctggtattaacaggcatgcaccaccacgcccggctaatttttgtatttttagtagagacgggatttcaccatgttggccaggctggtctcaaactcctgacctcaggtgatccgcccacctcggcctcccaaagtgctgggattataggcctgagccaccacgcccggcctaaaattgtttatcttaagattcatgcagtgaaagctaacttactgagtgataaatttgcttagtgatctgtttattaggttttccaaatttgctaattgggctttgaacagctgtaaaagttctgactgtaaaagaaagcttcaacttttggcattcatgatgcttttctgagtattaaactaagatagatgttttacctgaaggatcggccaccaatctttaaatggctaaacaaaagggttgctaaaacataatccaaattgacataagaaataccatttttccaaccaaaattttggcattcatatggctacttttacgtatttcagctgcatttgaacatctttttcaaactttagggtggttggtgtatcactgaggtcttggatgacactttagctttgattttgtttttatgaattaaaattgtcataccaaaatttttatttcaagcaaatccaagagcataaaaaattaaaatattacttaaaatactaagagagaacagatatatattttactaagcatatgttgaatgaaattgttcaaatatttataacaggcatagagtagaattttcttaaaaatatttttgatggtataccaatttgtattttctcagaaacatttgccttattcttttttctgttgtgtttttcttacctgattgaaagctcataatctgttgttattgtttgttaacctttaatgctctgatttcaggagttcaacctaagcctgctagctccatgcttaagcctagggatgagtgaaatttctggtggccagaagagtgccctttttgaagcagcccgtgaggtgactctggcccgtgtgagcggcaccgtgcagcagctccctgctgtccatcatgtcttccagcccgagctgcctgcagagccggcggcctactggagcaagttgaatgatctgtttggtaattaaaattaaaatttatcttatttttaaaaagcattccagggccagtatagtactttgcaccaagtaaatgtacaataaaggcagtggatctaatacattgaaagcgtttacagaggtagctaaagagcagcacgggtgtcctcggctcagaatttcttcctgtgtgtttgccactttgccattcattgacatggtcatggacatagggctctaagcccttgaggaaggctgggccagacctcaggggagatgcagccccaaaccacgtgcagtcctgtggacggatgtgtagatgtgccactgaggaacaatgtcttgagctttcatcagattctcagagaattgcttgactgcctttcgaagttgatgcatctgtgctcacgtttgcacccacccacgaggtccttctgtttcaggggatgctgcactgtatcagtccctgcccactctggcccgggccctggcacagtacctggtggtggtctccaaactgcccagtcatttgcaccttcctcctgagaaagagaaggacattgtgaaattcgtggtggcaacccttgaggtaagaggcagctcgggagctcagtgttgctgtggggagggggcatggggctgacactgaagagggtaaagcagttttatttgaaaagcaagatctctgaccagtccagtcacttttccatctcagcctggcagtaagtcttgtcaccgtcaagttattgtagccatccttcaccctcacctcgccactcctcatggtggcctgtgaggtcagccaggtccccttctcatctgcacctaccatgttaggtggatcctaattttagagacatgaaaaataatcatctggaagtactttatgtcttaagttggcctggacatgtcagccaaggaatacttacttggtttgtgttagtgcttgtaattcgcccccagaatgtgtacacgttctggatgcattaaagtctggcctgtatccttaaagggccatcgctgtgctgcctgccctcagcaaggacacactttgcagacccacagaggctccgcctccacctcacaccaaagaaagggaggagtccaaagggcatcagtgccattactcacaaaatgataaatacacccttattctgaaccacgtggagtcatatggtttgtgatccctgtccttcaggtttcagcttagtggggaagtgggaaagtcagcgtgtgatcacagcacagggtgattgctgctgattatattatgtgcctgctgtatgcaggatgaaatactttatatgcgtcatcttatttgactctcacaaccccctgtgagataggctctgttactcccatttgacaggtgaggaaagcaaggcttagagaatttcagtgacttgcccaggtcctctgagctaggaagtagccattctggcatttgaacccaaggcctgctatccctagaacccacgctctcaaattcaacctatgacagaggcaagccctggtgctgtgggagccccaaggaagagcctctggcctggtggccacgtagcccaggagagatttctacaggagcccacagcgctgaaggagagagaggcagcagagtaagggggctttgtggcagagaggggactggcactttggggaataggtgggtcaggactgaatgtaatggagccatgtcagagctgtccttctggaagggcaagggcacctggacgcgctgcccctcagtgctttggacggttccacaactgtgattcacacggcttccccaaacgaaggtacacgagtgggcattctgtgactcggtacttccctttaggccctgtcctggcatttgatccatgagcagatcccgctgagtctggatctccaggcagggctggactgctgctgcctggccctgcagctgcctggcctctggagcgtggtctcctccacagagtttgtgacccacgcctgctccctcatctactgtgtgcacttcatcctggaggccggtgagtccccgtccatgaacggtgggttcctatcatagttcctgtctgcttcaccatgtttttattttgtgctgcctgtttgccaggtactaagctaggaattggggatggagaggtagataaaatatgcatcaggaagggctgggccccatctcttactctccaatatattggagtctacactggaatttaactggaatttgcttttttagtcattttatttagattttgaagtttcagctttcatcaaaaatacctctaaactttatgtctctgtgatctttggtcttagctgttttatgtatttagtcttatatgatcataagattaataacattacattcagaagattatttgttttctgtcagagttaaaatgtttgtttttatactgcattgtaatattaacgtactgtaaaataaaagtggcttgttcttttcaaggaacagtatcctcaacaagggtcattagccacaatttttaaaaaattggacgtcatagtttacatgttagagggcgttttgaagctttgtatttttaaattaaatgttatagagtgatgttttcatgtttcataattgttttcatctgtgcatttgtagccaacttgaaaacaaagatccagggattactacttaaaagccagacttcttggaggttatagtgatgattttgatagtatcttgagccgtctcataataacctcagggtgagagatggccaacaggagacagtcgagggacttagaaatctgaatgaaatctgaagttcaaatcttcagacatataccactaaccaagagattggtacctcagtctagtattgtctgtttgtctaaaattggttctaaggaatctaggctagtctgtctatccctttcaacttttgtgaggctgcacaaatgtaaaatgttgaataaaaagcactgatggaagtgtgtagaaattcttctctttgttctgttgtaattttagttgcagtgcagcctggagagcagcttcttagtccagaaagaaggacaaataccccaaaagccatcagcgaggaggaggaggaagtagatccaaacacacagagtaagtctcaggacccatttttttcttacatgttgttcctccaggacttaaaaatcattcacagagacgtgcaccgcggtgagtgtggactcctggaagcgcaccgtagctccgctgtgtcctgctgctcctccctagctgtcagggaggctgtagtccattgctttgccagctcttttgtttccgagtgaacaccttatccgtacacatgcggctgtctctgaccctacagaccagctgggatgccactgggggagcgctcccttccccccgcacttcccacactctgcagttattctgagatccttgagggcagggaacaggtttgtcttctttgtgttctcagaaattaatgctcggcctctggtcagcaagcaacaaccttttgttgagtgataatgaataaataaatgtttcccacatgagtattcagtaacctcagtgtcaggttcagccatctgttttggtggatatttaaaagaaaattccgcttttcctacagaaaaaaaaaaaaatccaaatcccagtgatttaagccagttatagacttagacatatactacggcttttcatgcactttcctcccaattctagagtaggtattttactaggaaaatggtggcagtgcctgttgggaggaagattctttggccaagtgtcttttgttcttgccagggcccctaggctgctggggtgcttcagcttctttagcccagtgtctggtggggaatggcccctgttgcctgtcccacagaggtgggggtgcctcacctggagcctgtccacacattttacacagcacgcttacctggagcatcaggcatcttttccatgctctgtggctcaggaaacacgccttttcaatcatgagtgcaccagtgcttttgggctttttctccccgcttttgtgcaatcctggttgtggatggagttttcctgtctttagtcttctgcatagtacttttctcttctggttcccggttcaaggttttgtaattagagaatgacccagaagcaatggcattttaatgcacagccaaggacttctctgaatttgtatctcaaacctctgtgggtccttcaggcttcagtttgtgatttcatgatttcttgttgctacctaaggaatatgaaaacacccacctccctactctgcatcttccagccgagtggcacctcaggctgtggatcctgtgcttctgtggtgaggataagaatagtgccaaccgtgtggattgaaatcaatcagttaatccctccatgtaaagcacctggaacggatgacagtcttgttatgaatactcaacaaatgctatcatgatttttagttagatttccattgctttaaaacagttgagacatcttggcggtttgagttagagcaacgggccctgaagtgggttctgtttgggtgaagatgattatgcttattccccatggccctctttaggcaagagtgggaagctttctttgtttttttaatcacctcgataggacgttacttcttaaaggtcatccaataaatattaataggccgggcgcggtggctcacgcctgtaatcccagcactttgggaggccgaggcgggcggatcacgaggtcaggagatcgagaccatcccagctaaaacggtgaaaccccgtctctactaaaaatacaaaaaattagccgggcgtagtggcgggcgcctgtagtcccagctacttgggaggctgaggcaggagaatggcgtgaacccgggaggcggagcttgcagtgagccgagatcccgccactgcactccagcctgggcgacagagcaagactccgtctcaaaaaaaaaaaaaaatattaataaagccaactcgttagcgtggggcttaattgcttaagtccaatgagaagtccttctctatcctaggaagttgcccaaactgtagaatctcgtggcctgtgggtaatagccacgtaatacacactcactgcctcaacaaatcatattttagtaggtatgatattctagactcaagacaccattctgtggatcttcccaagggtgtgaagtgtccacagcgtctgccttgggagtttccatgcccaccagaaccatgccccaagcccctcaagcactctgacctaggaaagccagtgaagcaaggatgacaacatggccctttgatactagctgagggacagacacaggtcctgggagaccagagaaagacgaggggcagaggaggtgtcctaaaggaagtctgaggctgaggagccacaggatggcttccagctgtcacaggctgctgctggccttatcacagagagtgggccagagggctgggaaccaaggccagagctcaggttcaggaccattccagcaatcccagcagaaaatggggagaattgtatggtataggcggatatgaaggtagaatctgcaggccttcagtggccaactcagagtctaagtggattccacagttacagcttgagcagctggttgtaggtcatgctttctacactgggcatataggatgtgttttttaaaaagtcctctcttaaccgttgcttgtttagatcctaagtatatcactgcagcctgtgagatggtggcagaaatggtggagtctctgcagtcggtgttggccttgggtcataaaaggaatagcggcgtgccggcgtttctcacgccattgctaaggaacatcatcatcagcctggcccgcctgccccttgtcaacagctacacacgtgtgcccccactggtgagtctgctcgttccttgcagaagaccaagtacggtgaaaggcaccggtaggccctgggctgggcacacgtgagagggcgggacagaatccccgcagcccagaggctgcctgctgtggttctggtgcccactgtggttctggtgccaggctgctttcctcaggcaccacgtgtggaggtcgctagtagaaatactgggttttctaaaatgaactgaggccctacatccctaagagattagtgttagacctgattctagagcaactagaccactttgcttaatagcagaccagaaaccacaccccctcgagtgagtgagattttcctttggagataattcatgtttttctacacagttttgcagttgtcttcagaattggtttaaagtaggtgttattgccaggcgcagtagctcatgcctgtaatcccagcactttgggaagccaaggtgggcggatcacttgaggtcaggatttcgagaccagcctggccaacatggtgaaaccccatctctactaaaaatataaaaattagccaggtgtggtggtgtacgcctgtaatcccagctactcaggagactgagacaggagaatcgcttgaacccaggaggcgaaggttgcagtaagccgagatcgcgccactgcactctagcctgggcaacagagcaagactccgtctcaaaaaaaaaaaaggtaggtgttattgatcagaacccttgtttcagataacatgaggagcttagcttgaggagagtgagggttgatggagggggactgacttctgcccagtgaaatggcatcatctcccaccagcccgctgaaataagatgatggggcctgttccttagggcctgcagcatcctcaggcaggaaagaaaggccgacctggcagggtgtgagccagcaggtgtaggtcagggagaatggagccaggtcccagggaagaggcttgtggctgcctgagaagggtgcgtgcctgcctgtgtgtgtgtgtgcacgtgtgtgtatgtatgctggagagtctagggaggcttgctccaaggacgcagtattgtttgatcctgagagataaggattctgccgcagggaatgaaggtattccagatggcgggcttattccgaagaagaggccagtgcctggcggtgctggaagcagttgcagaacagggagttgtaggctttcctgggaagagagcagcaggggtgctggagaagcaggccacacttgctgcatggggttgctctcggccccactcttggtgcacagcgagtcactgtgggttcattagcatctggttatgagacagtaactgctcctttggaggggctcgtggagaccatgcaggagggcacggtcttgaggtcatgccgtccagagcacacctgaggataggccaggacgggctgcacgctgtaggtaaaattcctccagcaagctcttcactggcattgaggagttccctgagtgcggtcatctggaaggcagctgtaacaggcactgcagtctctccctgggtgggtaccagagaggagcataggggagcataaccgatttaaagagagggctttcctgtggtgaggtaagagattagctggtcattatcatagagccccctctgcctttgtgcagatgggctgtgggaatcctggggttccgttgggtcctttgtcacctcactgaaggcatgtaagctgagctggccagaccgtgagctgatcctgccacttgaacagcatcaagcctgcctctggattcttctgtgcatggcacttgtctgagcacctcacgcacagagaactggacttcagagtttacagaaataagctgtatggttcattttcatgcctgcttgccaataaacatatctgagctgaacctcattgaacgcctgcctttattctagcacagcacctgctgtttgtgggcgaggggtgctgtctctaactcctgcctgcttctcccagcactccctgagtggggtgtgccagcagcctcaggatgaggacaggaagtgggagggcagagcagatttgggagggccacttgatggggaaggaagtcccaggaagcagttggagctgttttctgggggagaaggtgccagctctgggacagtgttggggtagtgaggagggagcccagtggagagaagtcgggcttcctgcttcctcacagtatgtctgtcctgactcaactcggatgatgtcacttccttttcatcttctcaggtgtggaagcttggatggtcacccaaaccgggaggggattttggcacagcattccctgagatccccgtggagttcctccaggaaaaggaagtctttaaggagttcatctaccgcatcaacacactaggtactcttggggcctctccttcaggtcaccattgtcggacatctaccgggaggaaatccagagcccccagtactgggatcttctcatttgactccagaaaagatttaagcatgataataatacaaacctatgtgaatacattttgcagtgttggcaaaactccttttatactgagaaaatagatcccagttcctgtgttttgtggcttgaatcccagctttgtgtattccgggcttgtttgaagtcaggaaaggttcatgtgtagtggacaacgtgagaccaaattctgccttagattttgcatttaggctaaacagtggcagcacttgtctcagaatgttttcttgtgttcaccagtctgatcctgttgtgtctcagtggtccattttctcatatgggaacaagcagacgggagcagatggagtcaggtttcttggcactcgccttccccagagcctagaggcagcatggggagaaagcaggcttggggctcagacagtcctggtctgcttccagccctcctacctgagcagcgcagggcaagtccgtctaacctctagagaccctcagttttgtcatatgtaaaatgggggtcgtgtctatttcatagaattgttgcagatttagaaattacatttctaaacaaatgttaccccttatttctaaataagtgtctaaatgaataagtcaccacttttgcccctatttgatggcaagaggtgtgatcttgtggtgggactgtaatcagtcagttctcagtgactgtgccctgctgtggtgtttcctggaatgttcctgtcttgtcctagaaagtctggcaggggcaccctgactccactgtccagtcctctccccagtccctcgggcttctgcagatttgaggcttgtttggatcccagaaggttgtggcaggagacaccttgcctctactttcccctttataattcaatgtccaaagagagccctgagcaggtacctcacgccagctgcctcacggagctcctcctcttcctggctgtgaggatcggtatcagtggcctcctgctctctcccccttgcctaacacgagcacctttgcttacttgggtgcccttgctcttgaactgcccatcggacgtgcgtgacccaagactgtgccgcagtccttgccttgtctgtgctcattttctttgttcatttttttccctgtaacgtaaattgttatatttgtctgtatctgtgtctgaatcagtcctgcacgctctccttctctctgtctcttgttctttctttaccccgtttatcacggggaccccgatgtccattgctctagttctcctgtcctaagcaccccatcccgtctctctggccttaccacaagtggcgtggctgcctcagacatcatgatggggacatgaagcacagctgtcagaaacaactgttcgttagatacactcgaatgcagctcatcaatagggatggagggtctgtcggatgtattttcactgaatccccgttcctaccttgatacactctttttaatctattcttctagacaggtcagaggaaccattactttgacttttaaatttttagcagctttattgaggtagaattcacatactacagatttcacccactctaagcggacagcttggtggccattagttttatccacagagttgtgcagccagctgcacagtctcagggctggactccagggaagattttagcccatttagtgagtggggcagaagtggccctggccctgcacgaggttgcctgcatgggcgtccctgccctgtccctgtgtctgctccactgggggttgaccaggctgccagggccgacttgggcctgtgccacctgcctctcatgtgtctcggacagtgcagccgatgtctatacttcggtttcctcaatgatgaaatggaggggatagtgttccccgcatcatagaactgtgtgaggtttaagggactcactgcccttggcgtggagccttctccaggggccgtgctgtgtcggcgtagctgtcagctctccgttacaggcttgagaagggttgacactctctcatgtaacatttatatttctaggctggaccagtcgtactcagtttgaagaaacttgggccaccctccttggtgtcctggtgacgcagcccctcgtgatggagcaggaggagagcccaccagaagtaaggccacaccctgtgctggttggcacatgggcagttatggccgcttgcaggcctttggtggggaataaaataaggcagcaagctggtgttctttttttctcttaccttatttttgaaagagtagctgaatggtgtcttgactgatattccagagcagggacaaagcctgctgaggtctgggggctgcgattaccaatggctggaatgcattttattacggtgcattccatgttaaggatcaatacgattgtgccctttctggaaaatatcttttagtttatcaatattcagaggagtgtaggttgaattaaaatgaaaaggcactttataaaggccatgagtagtacctggtttcatttttctaatgtcttgcagagattttatcaggcttcttgaagtgttcacgtacattacgctaacacgatattaataataactgtgctctggtacagcggagccagcagaatgggaagttgtggaatgcaggcccttgattctgatagaaggtgtggtttgaactcacagaaatgacagtttggagggtagacatatgtcacaagtcatcaagattgtctttaaattcatgcatagaagctaacagggtgtcataagcaaggcctgtaaaatgtatgagggaattcaaagataatttattaaaaagtaattcatgtttggagttttgtgcccaaaggagtccttgatttgaaaaatgggcttttgcccatcagattgtttcagggcccgtgtgtgcggaggccctgccttgtgccccgtgagctcagcctgacagaaatcctttggtagcacttaaggctcctcttcctcccattgaggcagggaagactctgggttctgcaggcagaggtggttgtgggtgtcttgctgctcttgttgacatgtgggctctccttccaggaagacacagagaggacccagatcaacgtcctggccgtgcaggccatcacctcactggtgctcagtgcaatgactgtgcctgtggccggcaacccagctgtaagctgcttggagcagcagccccggaacaagcctctgaaagctctcgacaccaggtttgcttgagttcccacgtgtctctgggacatagcaggtgctggggacagtgggttccccgctgaagcgtccagcagcttcaaccaggccgttttccttcattgctagaattgaaaacaccgtccgtgtggcctgtgcaggagatgcagacccaaaggtggcctcctggtcagtgagaagctggaaacgtgacaggaactgacgtggggttattgagcatttaggggaagacgttagcagagcaggaatgagcaggcaactagtagaacacccacttaagggctcacggacaggtgctcacttaggaagtgagtttcatttggtattacaccaggttcctttaggcaaagcggagggaaagttctggtgtttttcacttgtaagattttgaaggaaacaaaacactctttaccttttttctaaaatgtaggtttgggaggaagctgagcattatcagagggattgtggagcaagagattcaagcaatggtttcaaagagagagaatattgccacccatcatttatatcaggcatgggatcctgtcccttctctgtctccggctactacaggtacctgagggaaagggtgcgggggagcggttgtacttgggctagaatgagagaagactggcatgctcaccacaccagtgatgcgggaagacctgagtgtggtctgagttggaggctgtggtgctaaatacgctgcccctttcataagcaggagtcttagtcaggcccagggaggaagtaaaatctggaaatgaatgagaagcattctctcctgccagtcaagaaatgagaagcgaaagaattctcacgggctgtaagaccagcaggatttaaaagttgaattagttgcttatgttaagaactcaaccaagttcatctacacaagctgaatctccagcttttcctaagaaaccatgtgtggcagtggctgcagggcagggcacagctgggcctgagcaccccgctccctgcacctctcccctccctgggccctgcctgtcactgcccactctcccaccaagccttccggttgtgtgcctgccctatcacaggcatcggagcttgtcacctggtttaaaagaagagagttgtgtggggatttgggatgcacgtttttcactcaaaagtattttagcgtagagctctgtgattccgtagctatttaggagtttaagcaccttgaaggctttaattgcagaaagttctatgtggacgtgcaatgtgttatacgcagtgtctatgagactcaaatgtttattagggcgttgaagtaaactgagcacttggagggccatggatccagccttcaaggagctcataagtcaggaggacccaggagcaatgacctgtcatagaaggcagaaaagaggggcacagaggtgggtgggaggcatacacaggcagctcctggagctccaaggggagcaagtgcttccagggaagggggcgtggaggcccctttggaggaggcaagttgatctggggtctggcagagggttagctggggacatttagcgggaggctggtgcccgggaattggggggatgcccagcagaaagacatgaggaggctggcctggggcgtgggggggtgtgaaaggttaagtgggggcattatcctgctcccgctcctgccggctgtatctggtcagcctgggcaccgaggtggggttctggaaggcactgttcaccaaaatgcttatctgggtcccccagagagcttgcctgcctggactgtcggctcgcctgcaactgctgactcctaagcttttgcagctcagcccacaaccagttcctattcacagaggtgggagctgaggggtgacaagtgactgctgcagtcttatttgtcatagagaaaaagtgacagagtccagcttgcccactggccctgccagcttaactggttataaagtgacaaatccccaagacccacagggctctgcacaacctgggccctcctgccagtggcggcgagggcaggtggctcacggctgggtgcctgtctgggcaggagctgggctggtatggggtgggcctgcggccctgcccccctgtgcagatcaagactcagggtgctggtgttcacaggtgccctcatcagccacgagaagctgctgctacagatcaaccccgagcgggagctggggagcatgagctacaaactcggccaggtcagtctcgcgcccccgccgcctggcctctgtccgtttctgtcctcagactttggcgcttgacacacccaggagaaaagctcagtgcactttttaaatgaaaggaagttttccttttttttaaaaaaaaatttaatgttcattgtttttatctgttttattcctaggtcccgcaagcagaggaagcattagttttgtttttatttatgttctgtattccagaaagtagttaagagacctcacatgtagcgatagagatgtgtgtaagagacagtgagagggcgtgacttggacttaagcaaggaccgtgagacacaaaaaggggggtgaggacagagtggagtcagctgaaatgctcaggaggaagtagacgccatgaagggccatggtatggggggccgcaggcgtggccgtgagtgtccctggggccagctcttggggggctccctgagtgtccctgtccctgtggccagttctgggtgggagccccgtgtgcaggcagacagctcggccacttcctagcaggtcacattggtctgtgcttctgtttcctcctcagataagtgaagggattcaagggtctgggtgtggtggctaacacctgtaatctataacattttaggaggctgaggcaggaggcttacctgagctcaggaggttgaggctgcagtgagccatgattgcaccactgcactccagcctgggcaacagaccagtactctgtcccttaaaaaaaaatgtaaacagaaacgtagggccatttgcatatgatggcacatggcgtggagccctacaggtgtatgctgggcggggcccggctgtgctggccgacttgcacctttccctccaccccggtgctgtgtctttcgctcaccgggttcctgatttagtgaaagcagttgtgcaggacagttctctttgtagcttttgtttctgtggaaatgggtcagaatatggtgtttagaaacacttatgagctctgagagtttcctcttctgagttcctggcctgcagccttcacagcagaaaccctgtgatgtcacaagcctgtttctgttccctgctctctgcctgtactgtcctgttttgtgcctgccggtttcagtgacaggaagcagggagctactggaccagcctgtatttttctagacatagttggaaaaagaagtcccactcttctgtcctttcacctttgacagatgtttccaccccaagataagtgaaaatgaccaataggatgcactgtatttttcatgaaagtgtttctgaagggcaggctgagagtgagaggcctggggctcactgggtgcctctggccttgtcctgggcccagggacactggtctgtgcccgaggtattccctatccccccaaccccgctgcatttggccacatccttcaatgtttgcgttgtgtccagcgtccgcaaaccaactgtcatgggatcatactggggctgaagtacggtcccacccctgccctgtctggggctgaagtacagtgccacccctgccctgtctggggctgaaggacagtgccacccctgccctgtctggggctgaagtacagtgccacccctgccctgtctggggctgaaggacagtgccaccccttccctgtctggggctgaaggacagtgccacccctgccctgtctggggctgaaggacagtgccacccctgccctgtctggggctgaaggacagtgccacccctgccctgtctggggctgaaggacagtgccacccctgccctgtctggggctgaaggacagtgccacccctgccctgtctggggctgaaggacagtgccacccctgccctgtctggggctgaaggacagtgccacccctgccctgtctggggctgaaggacagtgccacccctgccctgtctggggctgaaggacagtgccacccctgccctgtctggggctgaaggacagtgccacccctgccctgtctggggctgaaggacagtgccacccctgccctgtctggggctgaaggacagtgccacccctgccctgtctggggctgaaggacagtgccacccctgccctgtctggggctgaaggacagtgccacccctgccctgtctgggatgtttagcccctagatgccactggactgagccgctacttgcttttgggaaagaggggtgggggttaggggtctgggcgaggggagtgcaggggctcctccttggcctgagagctgttcatacagactcctcgcccactccctgcagggtgctgggtcccaggggggaaatggcccttggtgccaagaacgtgagttggggctagtgccagtgatgatggagaacagctttttatgggcacacagcccacagcactgtgccaagtgctcgaggcttcccgagaaccaggcagaaaggaggacagtcgaggtgtgctgactgcgtggtggctgcgtgatctagagcgcgggtcacaaaggcgcgagggagctctggccttgggtttaccgcaatgactgccagtgcgggagactggaaaaggaatctcacgtattggttccgtgttttggggactccattcagatgtcacttaggagtgaaagcatcccttcgtagagcctctttctgtgtcaccctcctcagctgctcctggggttgactggcccctgattcatgcctttagcatgtgctggagcttcccagcagctgtccagcccctgccccaccctctctgtgggctcccttgcccgtaacctggggtgtctgaacgacccttgctaaggggcagactgttagacggtaggcatgtgctgagtcccagtggccacacccacccaccaggagcctggcactgtggccgcagcactgagcagtgccccgtttctgtggcaggtgtccatacactccgtgtggctggggaacagcatcacacccctgagggaggaggaatgggacgaggaagaggaggaggaggccgacgcccctgcaccttcgtcaccacccacgtctccagtcaactccaggttttccaatggcctttttctttttaacagaaatttgaaatttcttatcagtcatttgatttgtttgaggtgcttcttgaaatgagcctctcatctcatgtacttggaaaatacccatctcgcatattccacaggaaacaccgggctggagttgacatccactcctgttcgcagtttttgcttgagttgtacagccgctggatcctgccgtccagctcagccaggaggaccccggccatcctgatcagtgaggtggtcagatccgtaagtgagccttcccattcccctcacacctgcacgtgccacacgcaccacacacgccacacaccccacacacacacaccgcccacacacatgccacttgcacacacacccctcatgcatgcaacacacacacaggccacacgcaccatagacaccacacacacatgccacatgcacacacatacacggcatgcaccatacacacaacacacacagcacacatgccacacacacacgccacaccacatgcaccacacacatgccacatgcacacacactccacatgcatgcaccacacacacacacacacaccacacacaccacatgcaccacaccacacaggttacatgcacacaacacacacatgccacgtgcacacaccccacacaccacatgtatgtgccacacacagcacacaaccacacacatgcaccacacacatgccacatgtgcatgcaccagacacatggcacacactacacacacgccacgtgcacacaccccacacacatgtacgcaccacacacatgccacacacacatgcaccacacacatgccacatgtacacacatgtatatacacaccccacaccacacacacaccacttgcacaccacgcacacacaccacatgcgcacacacacaccacatacgccacatgtacacaccatacacacaccatacatgcaccacgtgtaccacgcacccacacagacacagcacacgcatacaccacacacacacgcacacatgcgtcccgcacagtaatgtctcttgggtgtaagaacacgacttgccagtagtagcgttctggatgcgttgcctggattctaacagcgcgattctccccttgccctcctggttttccacatctccagcttctagtggtctcagacttgttcaccgagcgcaaccagtttgagctgatgtatgtgacgctgacagaactgcgaagggtgcacccttcagaagacgagatcctcgctcagtacctggtgcctgccacctgcaaggcagctgccgtccttgggatggtaagtgacaggtggcacagaggtttctgtgctgaagccacgggggcccatctgccttgggacctggtgttggccagaggtgccgggtgcggctgcctccttccaagagttgacccgaaccggactccacggcccacgtgagctgcagtgcttctcagatggagggggttcagcgacggtcagtgccattcacaggtcactgtgatgtgggttgtggcggccaagccatggtttggggtcccgtatccctgggcttatgacatcattgtagtagcccatccccacagaaccacggtgtgtggtggcgctgaggcatcgtagatggtggaaatgctactggcttccccatgctctgccctgaggcctgactgcctcactccccttctcagttatgttccaggccccccgagcttcctggctggacagcttctctcctgggggccgttttgtcacagtgaccctgtgtttctagtcccaaatctgggtgctatagtctctttttagcgtggtggttgtcttagtcttttttggctgctaccacaagttaccttagactgggtaatttataaacagtggaaatttacttctcaccgttctgggggctggaagttttcatggtcaaggtgccagcagatttggtgtgtgatgagggctgctctctgcttcatagatggcatcttctggctgggtcctcacggtggaaggagtgaacaagctccctcaggccttttagaagggccccaatccacaagggctctcccatcatgacctcatcacctcccaaggccccaccttcttgtactgtggcactgcaaattaggtgtcagtgtaggagtttcaggagggatagaaacattcagaccatcccagcggtcaagtgttcatcctcttgagttcctccttattctgcttctggtttatcaggattcagccagtgcagcatggtacctgtattctgtggcacatcaccacatggtatttgccaagtatccatcacctgcacacgtgaaatcattgcccgtgggtcccgacatctggcgaagcatattcaaggatggcagaactgtcagagctggcacctctggttccttgtcatgtggcattacctagtaatccattttatgatagcaatggaaactcatttcttcaacaaacacctgagtggctgccgtgtgccagccgtctggggcccttggtgagaatggcatggtggtgcccatcagggcctgcctagcccgtgctctggacgggctcctgtgtgtcaggaacgacaatgctgtcatgacggtgaatgatttttttttttgccatcactccagccgctaacatttgcggagctcttcctcccgcacccccacctgacaaggccaagggtgaccttggccccaccctaggcggccaaggtcagaggttagctggcttgtctgggtcacacaaaatgcagcagaggttgaggtgagcacatgtccgtgacctggagcctgactccctctctgcgagtcttgactgctcttgcctagactctgtcctccccgagcccaaacgccagtcatcttcccttgtgggtgtccttcagcctggtgccatgctggtgactcagcagccgtccagggagtggaaacaattgagtgtgtgggttccctgtgtgggcatctctcttcacggcgaacaccctctgggtgttgcccacacgatgtcaaagcggctcttggaaggggtccttctcctttgtgggaagtttcagctgctgggctaacttgaattgtaactgtggttttgtgctcaggcccagatccccctaggcaagtgttgtgccatcagtaatcaaatgagaaataatcattttgaaaagcagatcctaaggcaggatggtcatggacactcactcccagctctttgtgcactcatgctttctggaagatggccatcctctgtgaaggttttcagcgcgtcatgcttggtacccacgtatccagagcatgtcgttttgaggtatttgcccaccgttgtgaaatccgtgccacccgagagcaggtcctgatgtggggctttcagaagtgggacctggggccgtacgcagtccttagggaggggccgtgtggcgttgtgcgtgtgaggggatagcacagggtgaggtgggggcccaagaaggaagtgacccacaaagaacagcctcctcttttggtccttgttcctgggatggctgggagtggcttctgtgtcgtccggccatttcccctgcggagaggctcctaccactgccgagaacctcatcattccacaaaaacaagaggccgcctggccatccagcgctccatgggaattctgtgtccccatagtcttgggctgaaggagggtgacattccttgctgacttctgcaggggtctcctcactgttaaagagcagattgaaagtgaagaacgtgggctaagtgtttaggtcgatatttaaccctgctaggttttggatactaagtgaaattgaggccattttggttgaagttgacagaaaccactatcagggatccccaagactaccccaggcttttctagaaagactctcagctaagatgtgttatggtaaaagcacacaaaacaaaatcagcaaagaaaattagcaagggcagaggcccatggggcgatgtcccgaggacaccaggcttgagcttccagaatcctctcccagcggggtcgtgcaggacgcacttaactccccgcacagtgagccgtgacagcgcgtgtgcagtgtcgtcgccaggaaagcacactagagactcggtgccagggtttttactgggggctgggcacatgggcaccctctgcctgcctcgtgcccagactctggactcccggagggaaggcaagttctcagcaccaaccctggtgcccacacaagcagctgagcacagggagcccctcctcagtgaggatggtgggcaccgtcccaacaccagccaggggccagccttgcacacaggcctctcaggatggtctccggcctgctgtgtagtctcttctgcacacaagcgtgagggcagcgcccccgcctcggctgtggggaggagccactgggacgtgagctctggtggcatgcagcagcttttgtctgtgtgtgcctaggacaaggccgtggcggagcctgtcagccgcctgctggagagcacgctcaggagcagccacctgcccagcagggttggagccctgcacggcgtcctctatgtgctggagtgcgacctgctggacgacactgccaagcagctcatcccggtcatcagcgactatctcctctccaacctgaaagggatcgcccagtgagtgggagcctggctggggctggggcgggggtctcagaatgagctgtgaaggaagcagcatcaccctctccaagtgcccaggctcctggccagatggcaggccaggtatcagtgggaacccaggtgggtgccatggctgaggtcagtgagacgcaagagcacaggtgcgtcctagaggcttcctcgggcacctccagcgagctggagctctcgcctctgctgctgtctcatgtggcgcttagcacactctcccacgtgcccattcctgactctgctctcgaggccatcggctctcattctctgctcccagaaccctgttattacccaggctagcctcctctctgcaccttccccgccctggcccagtacctccctcttgtttccactgtgattccgacctcaccttatcttaaagctgctggacggcaggttctgtacacacgtgtccttgacaaagcacggctggtgccgcaacccctcagcgagcaagtcaagctcttcacagcgatgtcttacaagcgcagagggctctgtgacaccctggtctcaccgccactcttccaaagtcgcagaggctttagcagagatgggcccagcctctctgagtcataggcttctgcacacgggagctgtctttagagggagggtggaatttcatcagccacccacatgggggagttgagggcaagaattaggagcaaagatgggaaggggtctgggaggaatggccagtgatcccctttgacaagtgggcaggaaacgggggctaggtcaaagttgagtggaagacctggagggagacgggaaggtctctgtaggcacagttcagacaggagggaggtgtgagccagggcacatgccggtggccgtctggcaggatttgggacatgctggagcagggacagcggctcatcaggggccattgccctcatccaggccagagtgtcacaagcccgtggggaggcccttctcgcctgtcatccttgctgggcagtgggtgctgtgctagcaggacaggcggacggctggcaactgtctctgcatccctggagcctggcatagggccaagtcacacggggcacaggcctgcaaatcaggcacatatgttggtgcagtgacgtgattttggggggcagccccagaacaggccccagacacaggccaaagccctgcctgtgctggtgtgttgggctgttctatggctcttgctgtgggcatggaggactcagggaaggagagttgaggtggtccaggagttgcgtttgggatgcagagagcttgtggcatccaggtagaaatggtgcgtggggctgacctcagcaccatgggcagaggggccgtgtcacgtgcctccgaggtggaggtgggaccacgtggtgacagatatacgcatcactgggcacgtttttgtgggtgttggggggcatcgtattggctcctctgttcacagtggccactcattcagtccctggctaccaggtcctcactgtgccatggggaaggccggcgctgtcgggggatcacagaaggcagcacgtcatgatggcatgtgccatgaaggaaaagcacagggcactcaggaagtagaggggactggcctggggtgtgggaatctagggcctcgttgagggacagagagaggaagtgtgtggtggccagcatggaggtggccacaggggaggctgagttaggccgagagggcagggcgttggggaggtagacgggctcagccactcagggagtggtcaagcagaggctgaagggtcaggccaggttgcaggggcctgggggagccactcagggtaggcgctcccgggagcccgcctggcccatagctctacactcccgcgtggggccggacatgctgtgaagccctctccacgttggatgggggtggctgagcctggatgctgtctcccgttttcagctgcgtgaacattcacagccagcagcacgtactggtcatgtgtgccactgcgttttacctcattgagaactatcctctggacgtagggccggaattttcagcatcaataatacaggtgagtgggccctggctgtcttcctctgcacacggggagtgggcttcccttctcttttccttgcaggatcataccagtgggccagttttgacttggtcgggaggaggcatgaacacctgagactgtgcagcgattctttgacacagaggcctttctccctgtgcagatgtgtggggtgatgctgtctggaagtgaggagtccaccccctccatcatttaccactgtgccctcagaggcctggagcgcctcctgctctctgagcagctctcccgcctggatgcagaatcgctggtcaagctgagtgtggacagagtgaacgtgcacagcccgcaccgggccatggcggctctgggcctgatgctcacctgcatgtacacaggtgagcatgtacacggtgcccataaggccagcccaagtcctgttcaagggaggcaggagcatgctcactcaagggacctcgactaggtgccctctgatttcacacttctggtgttgccccaagccggccccatcaccttgcaagaaaggctctggagcccccagggctggagtacctggtcagggttgaccgtccctgtggtcactcatcccatgtggctgagctgggctgggtcctgggcaagcaaggggctgatatcacctgctttcagatctccagggactcactggacccctgtgtacaaagcactgtctacagagcctattgggttgtatagaggtaaccttcgtactgaacacttttgttacaggaaaggagaaagtcagtccgggtagaacttcagaccctaatcctgcagcccccgacagcgagtcagtgattgttgctatggagcgggtatctgttctttttgataggtaagaagcgaagccccatccctcagccgttagcttccctagaactttggcctgaagctgtgcttttgtgtgtgtctgctgatcccctggcgctgttgctggagtcctgccagtgattccccaccacagcctgaccatgggctgccttggctcagggttccactggcgagctggtggtccttggaccccagcactcaggtgtagcgttgaccagttccaaggttgtcccagtgcctgcccatctctcctgagggctcagggacagtacctggcagttgggggtgtggcagggggcaggaatgaccagcctctgggagggtggggcagaagcctgtacagtgaggaggagctggctcagcctggctgcctatcgtgagaggggagcccacggggctgtgggaggggggccgtggtgcctgtgagcagggtgaggagcagcggcaggaggatgaaggtggaacccacacatgcatctttgagacccgtgtggtcagtggcttctgccccccaccaccccccactgctgtgcgtgcatagaattggcttccctcacctgctctggaagtgggttaggagcttggtagggctttttctcaaggacaagggcccctgatttgctctcaggcctcagtcctggcgacatggtggatctggagccttgttgcactgccttgcctgtgctctccaatcagggtggccagtggggagccatttggcttttctcaagagcatactcaggtggaccttgctccactgtttgaccagatgaggcattctgaacagccaagcctgtgctggtctgttttcatgttgatttttttttttcttttctttttgagatggagtttttcccttgtcacccaggctggagtgcaatggtgtgatctcggctcactgcaacctccgcctcccgggttcaagtgattctcctgcctcagcctccctagtagctgggattacaggcacacaccaccatgcccagctaatttttgtgtttttagtagagacggggtttcaccgtgttggctgggctggtctcgaactcctgaactcaagtgatccaccctccttggcctcccaaagtgctgggattgcaggcgtgagccactgcgcccggcccccatgtcgatttttaaatgcacctctgcatcgttcttcagtccccatatgctcactgagcaccactgcgactggcagacgggcacagggaggcgccacgaccagtcctggccttcaaggggcttgtggtctagtgggcccaatgctaggtggcgagtgctccaaagagtgtggtgcacgccttccgcttgaccgctctccagacgccacagggaggcacctcgcagctgaccacagatttctctctgtggagcagtgtcttcagagcggctgccatgccactgctgggcgagggtctgcgggcgggtagagccaggagcacctgtgaggaagtgcactgccattttcgtagctgcttcccgtgtgtctcagttacacacggctggcatgtgtgcactgatgagacgggaacgtgatggttgcttttcagcactgaaagggatactgctcagggggcgtgtttcaggatctggttagggaagaagcagcgagagcacagatggggccctgtgtggtaacaagaaaaaagtcctggttgacaacagtgccacgaagcgttagaacacatagggatgtttgtggagcatttgcatgtggaaagcagcaaaaacataatgggaacgggttcttttgttatgatttttaaaaatctcttttgtaacatccttcccgctgcgccgtttctgcatattcctttatgtagctttcaaactcctcttaggagttctggtccctacagggcgtgggagcccaggctttacgtagctttcaaactcctcttaggagttctggtccctacagggtgtgggagcccagggcctgtgccgagcagcctgcctccacgagctagacagaggaagggctggggttttgcctttttagtctcaaaattcgtactccagttgcttaggctctgactttccccacttggaaagtccctcacggccgagggtccctcccagccctgatttcacatcggcattttccccagtattagagccaaggccctccgcgggcaggtggggcagctgtgggagctggtgccagtctctgacctgcgtccctcctcccaggatcaggaaaggctttccttgtgaagccagagtggtggccaggatcctgccccagtttctagacgacttcttcccaccccaggacatcatgaacaaagtcatcggagagtttctgtccaaccagcagccatacccccagttcatggccaccgtggtgtataaggtgaggttgcatgtgggatggggatggagtgggaaagcctggaggtggagttgcctccgacttcccagcagattcgccagcagagcccagctcctccgctttaaagcagcaatgcctctggcccccaccccacccccgccacccaggcgcagcaggtgcttcccgtccccccagccctgacactcaggcacctgcttgctccttgcaggtgtttcagactctgcacagcaccgggcagtcgtccatggtccgggactgggtcatgctgtccctctccaacttcacgcagagggccccggtcgccatggccacgtggagcctctcctgcttctttgtcagcgcgtccaccagcccgtgggtcgcggcgatgtatcctctctgggtccctggtgctggccccgtttcccttgtcaacaccgaggctcatgtttcatgataaggttttgaaacctaacctttgcaaaaaccccacagatgccagggtgacaggccctcagccccagggaagtaaaatgctgacaggggtacagaaaggagcacgtccagacatttgctgaccagggcctctcagaggggccggtgtatggcaggagggtcgcagctgaggggcctttctgtggagggcctgggtgaggggagcgagggtgggcggtggtctctgcagacgtcccgcccactcgcgggctctgtgtggctgggcttctcctgacactgcttctcattagctttggtcattgtgcctcgatcgccctctcggggaaaggcttaagtaaagatccagttcccacccccagatgctggctgccaggagtttccctttccacagcccttccccaagacagaccacaagagcctccaagcagcacagttgtcctggtgctgacagcacagccttgcccggcgtgcctggcacggctctgccctcactgcattggagcagggctagtggaggccagcggaagcaccggccaccagcgctgcacaggagccaggccaggtgagtgctgccgagtgggtgccctgcctgcagggcatccagccagccaagggttgcaggaatggaggtggaggcgctgatgcagctggaggcatccaggtggcccttccggggctctgctcgctctccaggctccctggacccctttgtagactgtttcaggagaggaactcccaggtgaggacagggaggcagcattcccctcatttgccggcctttttccttaactcctgcaccagcctcccacatgtcatcagcaggatgggcaagctggagcaggtggacgtgaaccttttctgcctggtcgccacagacttctacagacaccagatagaggaggagctcgaccgcagggccttccagtctgtgcttgaggtggttgcagccccaggaagcccatatcaccggctgctgacttgtttacgaaatgtccacaaggtcaccacctgctgagcgccatggtgggagagactgtgaggcggcagctggggccggagcctttggaagtctgcgcccttgtgccctgcctccaccgagccagcttggtccctatgggcttccgcacatgccgcgggcggccaggcaacgtgcgtgtctctgccatgtggcagaagtgctctttgtggcagtggccaggcagggagtgtctgcagtcctggtggggctgagcctgaggccttccagaaagcaggagcagctgtgctgcaccccatgtgggtgaccaggtcctttctcctgatagtcacctgctggttgttgccaggttgcagctgctcttgcatctgggccagaagtcctccctcctgcaggctggctgttggcccctctgctgtcctgcagtagaaggtgccgtgagcaggctttgggaacactggcctgggtctccctggtggggtgtgcatgccacgccccgtgtctggatgcacagatgccatggcctgtgctgggccagtggctgggggtgctagacacccggcaccattctcccttctctcttttcttctcaggatttaaaatttaattatatcagtaaagagattaattttaacgtaactctttctatgcccgtgtaaagtatgtgaatcgcaaggcctgtgctgcatgcgacagcgtccggggtggtggacagggcccccggccacgctccctctcctgtagccactggcatagccctcctgagcacccgctgacatttccgttgtacatgttcctgtttatgcattcacaaggtgactgggatgtagagaggcgttagtgggcaggtggccacagcaggactgaggacaggcccccattatcctaggggtgcgctcacctgcagcccctcctcctcgggcacagacgactgtcgttctccacccaccagtcagggacagcagcctccctgtcactcagctgagaaggccagccctccctggctgtgagcagcctccactgtgtccagagacatgggcctcccactcctgttccttgctagccctggggtggcgtctgcctaggagctggctggcaggtgttgggacctgctgctccatggatgcatgccctaagagtgtcactgagctgtgttttgtctgagcctctctcggtcaacagcaaagcttggtgtcttggcactgttagtgacagagcccagcatcccttctgcccccgttccagctgacatcttgcacggtgaccccttttagtcaggagagtgcagatctgtgctcatcggagactgccccacggccctgtcagagccgccactcctatccccaggccaggtccctggaccagcctcctgtttgcaggcccagaggagccaagtcattaaaatggaagtggattctggatggccgggctgctgctgatgtaggagctggatttgggagctctgcttgccgactggctgtgagacgaggcaggggctctgcttcctcagccctagaggcgagccaggcaaggttggcgactgtcatgtggcttggtttggtcatgcccgtcgatgttttgggtattgaatgtggtaagtggaggaaatgttggaactctgtgcaggtgctgccttgagacccccaagcttccacctgtccctctcctatgtggcagctggggagcagctgagatgtggacttgtatgctgcccacatacgtgagggggagctgaaagggagcccctcctctgagcagcctctgccaggcctgtatgaggcttttcccaccagctcccaacagaggcctcccccagccaggaccacctcgtcctcgtggcggggcagcaggagcggtagaaaggggtccgatgtttgaggaggcccttaagggaagctactgaattataacacgtaagaaaatcaccattccgtattggttgggggctcctgtttctcatcctagctttttcctggaaagcccgctagaaggtttgggaacgaggggaaagttctcagaactgttggctgctccccacccgcctcccgcctcccccgcaggttatgtcagcagctctgagacagcagtatcacaggccagatgttgttcctggctagatgtttacatttgtaagaaataacactgtgaatgtaaaacagagccattcccttggaatgcatatcgctgggctcaacatagagtttgtcttcctcttgtttacgacgtgatctaaaccagtccttagcaaggggctcagaacaccccgctctggcagtaggtgtcccccacccccaaagacctgcctgtgtgctccggagatgaatatgagctcattagtaaaaatgacttcacccacgcatatacataaagtatccatgcatgtgcatatagacacatctataattttacacacacacctctcaagacggagatgcatggcctctaagagtgcccgtgtcggttcttcctggaagttgactttccttagacccgccaggtcaagttagccgcgtgacggacatccaggcgtgggacgtggtcagggcagggctcattcattgcccactaggatcccactggcgaagatggtctccatatcagctctctgcagaagggaggaagactttatcatgttcctaaaaatctgtggcaagcacccatcgtattatccaaattttgttgcaaatgtgattaatttggttgtcaagttttgggggtgggctgtggggagattgcttttgttttcctgctggtaatatcgggaaagattttaatgaaaccagggtagaattgtttggcaatgcactgaagcgtgtttctttcccaaaatgtgcctcccttccgctgcgggcccagctgagtctatgtaggtgatgtttccagctgccaagtgctctttgttactgtccaccctcatttctgccagcgcatgtgtcctttcaaggggaaaatgtgaagctgaaccccctccagacacccagaatgtagcatctgagaaggccctgtgccctaaaggacacccctcgcccccatcttcatggagggggtcatttcagagccctcggagccaatgaacagctcctcctcttggagctgagatgagccccacgtggagctcgggacggatagtagacagcaataactcggtgtgtggccgcctggcaggtggaacttcctcccgttgcggggtggagtgaggttagttctgtgtgtctggtgggtggagtcaggcttctcttgctacctgtgagcatccttcccagcagacatcctcatcgggctttgtccctcccccgcttcctccctctgcggggaggacccgggaccacagctgctggccagggtagacttggagctgtcctccagaggggtcacgtgtaggagtgagaagaaggaagatcttgagagctgctgagggaccttggagagctcaggatggctcagacgaggacactcgcttgccgggcctgggcctcctgggaaggagggagctgctcagaatgccgcatgacaactgaaggcaacctggaaggttcaggggccgctcttcccccatgtgcctgtcacgctctggtgcagtcaaaggaacgccttcccctcagttgtttctaagagcagagtctcccgctgcaatctgggtggtaactgccagccttggaggatcgtggccaacgtggacctgcctacggagggtgggctctgacccaagtggggcctccttgtccaggtctcactgctttgcaccgtggtcagagggactgtcagctgagcttgagctcccctggagccagcagggctgtgatgggcgagtcccggagccccacccagacctgaatgcttctgagagcaaagggaaggactgacgagagatgtatatttaattttttaactgctgcaaacattgtacatccaaattaaaggaaaaaaatggaaaccatcagttgttgctgtgtgaggcttgctttgcttcatgagaacctagaccttgctgagctggagtcttaggaagcagtctcctaagtgcttctccagcaggggcagaaactgtcccaccagctaacatctggcattatggagggtcccccaggcagctgccagcagggacaggccccgtgttttctgtagccagggatgaggaagtggccccagggcatgggcctggctgggtgcttctgcaagggccttcccaaaccacagtacaggtggtcttcctgccctgcagatgggagctgtgggagctgctggagctgctggagccttcatggtcaagtgacatcataagcttatatgacatacacaagcctcaggacttggcccatggcactgaagcaggtcatcaggcccagcacagagactagagctgtgttctcacagggcccaccacccttccacctccttggccattgacacctgcgtccctggcccagctgctcccaggtaacccccaaagcagctggcacatcccacctctggtgtggccggggctgctgtgtgtccgcagggcctgccccgtctattctagcttgtttgtcctgtctgaaccagcgcctactccaagaagcctctgctcagcccagcggggatgcttctaagctccggacgagcctctcggaagccttggtgattggtggtgtagtcatcttgggatgcagatgtcttaccaacctgcaagaacaaaaaccctgtggcttcctctggtgcagggtatttagtcaatgtttgctgaggtcccgtctggttctggctaattggcaggggtcgtccacccattctttccctgctctgctgtctgtgccaggagagacgggggccagtcggccaaggggccagctcctgctgcctgctcctcttgggcacgtgcgggggccccctttctctgagcagggatagggatcagtctgccggagggatgtggtggacaggcctaaagcatttggggcggggcatgccacttgagctccctaaatctgtctcctcataggtgacaccgctccagggccccccagtggcctctcctttcagagctacctaaattctggtcacttcagagaaatggagcacccccttctccctggtccaggtgtggacagcctggcacactgagcacacctggcatggctggtaatttcagaaagaagaggggccggggtccagtgggaagcagcggtgaacccctcgtgagtgggctttgcagtccctccccatgccacggcagagctgccctcaacacagccttcctcttcctcatcggagagcacaccctgtccccttgccgagctgtgccctgtgccttcggtggtatttgattttggctgctactggctttgttgggatctggaagtcgcttcccctgcgtggtgcgtggagcactgtaagtcagatgagggaagtagccagggtgaggtgagtaccgggtggagccgccactgaagggactgggtaggggggccttgcctctacatgatgtgacacagccaaccgaggacagaggaagccccgttcctgggggtgtggggtgcacccctcagggaagcctgcagtggggcctgaggaaaggcatcctccgcgagcccacgagtctggtccatgagcaccgtgacagtgtctgtgggtagaggtggacccggccttgtgtcatcaccaggacctcttttgggaaaccatgtggacatcgcttgcgggtcccccaggctctgcagccccagcagcctggctgccttttgggcaagtggcttgagccacagaggacccagtcctgttgcagccacatcctctgggggggcccgccagtgtggccggctttctccaccctacaccaggcctccaggtgtcctggtcgggggtgtctgggccctgggtgggccctgtggacctgtgaggtcagggtcagggcatcactggaggcagagggctgaagttgtgggtctgggttccccttgtgtgcacaggcccctgccctccatgcttggtcaggcagctacccccaaaactgctaggacaggctggtcctgaggtggatcctggcccctgtaccctctggacagcccacccgcccaaccttctaccctgccccagcggcggcagtgttggccacatccttcccctcctggccccaattgctctggggaagtccaggctccggagcctgcccaggggccccccgtgatttgggcccaggactccacgtggttctctgccttcacccaagccctgaactcctcagctgccaaatccccacccatctgcacaggctgtgctcaccactgctgctcctggaaggtgcccctcagtgggacgcccacctcctctctgggcttctgtgtttgggagccctgctgcccccacccttggtcagtccccatgtcctgctggcctgtcaggcagggcagaaaatccacccagaaatgctgagcaggatgagagtctagttgggcccagcctcattatttagaagggatggaggcctagggagcatgcttctagcctgagcccagcagggccccgcccatgtcccaggtctgcaccagggacagctcctgccgaggcctgacctgccccttctccctcaggtgctgctggttgaccagcctctggccctaggagaccccgtagcgactgagggtcccagcaggccatgcagctttgccaaggtacgagcccctccccagcaggggacagatgtggggaccctcccaggcaggagcagctgggtgcctggtgctgccatctgctgcctgcctggttcttgtcctcacattggaggtcagtgtgagggctctgcctcgggaaaggccatggagcttgccctgtccagggcctcccatgtgcactgagcctgggaagagagggttggagttgagccttttaccctgggaatgctgcctggaggatggtgcgggtgtggggtggcaccctgccaggcagggccctgcctccctgcgcccactggaactcgggcaggcaggggtgtaggtgcctcctctagagccgtccggtgggggcccccggcagtggtggtggtgtccactggccagcagctgccccttcagccaggacagtaggcctgacgctgtccccagcagctccaaggtggatttgtggaagggggtagagggcacgtagaggccccatgacctccccagggttctgggagggctgtgcccccttagccagcaccatgctgggtgatatagtcagatcctgttacccctgttgtggaggtgaggaaacaggttagtggggaggacatgactaaggtccatgctgagtcgctagagctgcacccagaaccactgctgggaccccatgcctttctgcttaccccttgtgccgggagatgccaagagatgctgggagccagccccacctctgcccttggagtcatggctacggaaagggcattcggaccggtccctgacctcaccggggagggccgaaccctgttcctgaggagccagggcttcctagaggaggtaggccttctagtcactccttcatctgcaggcactccacagagctctctgtgccagcccccagcacggagggctgaccttagtcgagtggagatgccccagtgccaggcagtagggatgatgtctcctgaggcccagatggaagggactggactagtctcatggggctgatggtggggccaggccttgaccagggacccagtgtagggggtgcagagacccctctgagttcctcacacatccctggggccctccccatacacttcctatcctgactgcgggcaagagggagccccagttcgccttccctatgctgggcacccacagtggggctgggcacccccgccatgcccctgccctgtccttcccctgagagcctcggtcccacctccaaggtgcctcagaggacagcaggggcagcgggcagaggccgagatgcctcctcattccaggctcagctgcccttcttggggcagcccacacctgagagtctcctgcagttggtcaggcctgaggagggcaggggggtgcctgctgtccctctgctgaccacagtggcatttagcctgggcaccgcgcccagcacagtccatgctgcacaggtgccgtgggctccacagagccctgcctgacatgcatgtgttacgtttcgggtgccgatgcccttgggcggcacttctccgggcagaacccccaggccaccgctccggttccggttccgctgcatctggggctctcggcaggctgtggtcctccggccagcctgggggcatctcagtccctcagccccacaggggcctgccccgcagcctgggcctcgagccccgtctccgcacgctgtgccgaatctggctgcccatcagctccctgcgtacccagactgtgccctgccatgcccgtggctcttcccaggagtgccctgtggcctccccctggcttgctgggctgattccctcctgtgtctcaaacagagctcacctttgccatcactgctgtcctcaccggccggtgccagaggcccgtgtctgtgtaccctgtgtctgcacctctgggcagggcctggctctgaccaacccgggcttccagtgtccacagacctaaggcccagggcgcctgggggctggagcaagagaagcaaaaggagccaagggtgggggtttggggttcttgtgagggcccagccccaggaccccaggaccaggacacccaggagccccagggcccagccccagttcagaaggcaggggccttctgagggagcttaagggtcccacagcccaggacccccaccagggccagtggccagcgttgggggactcagcctcctcgtcgctcgtcctctctgtttctcccaccttttgccccctttctccttgcctgttcccacccgaggccccctcttggcctgcgtgagccggggcggcactgaactgggggccgatccgcctgggcggcggtgagaggcagggccgggagccgggccgctgggtttgggcctggcccgctcgccgcaatattgatggcccgtcagtgcagccctgattcctgtgctttcagttaaaaggtttctgttgttgtagcttatgcagttgctctgttgctatggaaacgtgacatcaaaatgacgtttcccgtttaaaagcttttaactaaattcctgcctgtcagatgtaggccccattttgagcgtggagctgccttcgagcgagcgtgagcggcgcctcccgcccatggtgcgtggggccgggccggggccctcgctgagcgcgctctctcaccccacaggcgcctccggcatggcggcggccgaggggcccggctacctcgtgtctccccaggcggagaagcaccggcgggcccgcaactggacggacgccgagatgcgcggcctcatgctggtctgggaggagttcttcgacgagctcaagcagaccaagcgcaacgccaaggtgtacgagaagatggccagcaagctcttcgagatgaccggcgagcgcaggctgggcgaggagatcaagatcaagatcaccaacatgaccttccagtacaggtgggcgagcgggcagtgtgggccccaccaggacgggcgggcccgggcgtggcgggccgctcctgactttcttggagctctgagtcgggacgatgtgtgggtcgtggcctgcctgtcggtctcctctggccgggtatgggcagaaccccacggggtgagacggggcccacggaaaccgtgtgtgcagccttccattggggaagtggggaaactgaggcccagcaagggcaggaaaccagtctaagagctgaggggtagcaggggtggggctggtgctgggcagaggccaggatggctcccaggacgtatgggcggtctgggcactgtccctcggaggcagcaacactcatggtggtgcccactgacctcacaccctgctcccccatagggaggcggcggctgccagtgccctccccaccaccaagctcccaagctcagcaggggtttcaggggcctactgcgtcattggggaaattgagactgcaagtgagaaggaggctcagtgctctgcgacttggagcatccactgagcctctgccatgagccggtgagccccactggggctggccctagggtcacggtggggtatttccagaaatcaccaggtgaggtgcaggaccagccagcgcatgggtggggcttacggtgcgaagaagaaagaggtggaggcctgccctggcccaggactcccagcgtgggggctcccggcctggccccacctctgctcctgctacatggcaggtgggcccttcctgccctggcaacctgcagggaaggccggaggggaccacccagccagggagatgttggcgtctaggaggggacaggtgtggtcccacacacccagcatcttaaagtgcgtgggtccccagcccattaggacagggtcccgggtgggcaggggtcatggtggggtgaaggtctcaggcacaggcaaggtcacaggtgcggtgagggtcttgcagggtgtgaaggtcataggtgtgcggtgaaggtcacaggtgtggggtgatggttttgggtgtggggagggtcttgcacggagcgagggtggcagcaagagctggaagctgcagggggagaatggcagcagagagcacccggccctgtgggcggcctggacagggctgggcctggggctgccggagagcctgtcagcttccaggatgggagtggcctcactcagctgctccacctccgggtcaggcaggtgagcctggggcagagaggctgagagcacctgagccacttgtgggagaggccacccccactgcccccctcaggcgaggagccggcctccagcacagcagaagggaacccccagtccccagccctagtgggagtggggaagaggcccagcaaggccccggacagaccgccagcctgtgaggtctccgctttcagttgcgttgatttgattttttctgagccttgaaggaggggtccggggcctggccctgcccaaaggcccctaggcaggccccaaagccgggacctagggtgctgagcatgacggatgttgggtttgagcggctggcttgcgacgtgagggctgaggtgtgagcctgggtatcttcagaggttcggtggacacaggcagctgcccgcggccccactgttcccgtggcctcctagtcctgctcaggcacctggtgaggaagggacgcagagggcagtgggaggtggccacgactgttccagcaggctcccctctgactcaggaattcacgggcaccacctccctggctggctctggttggtgtctggccaggttattcattatttatgctgaaagcctcttcagagtcccaggggagggtttctgtctccattcctggaggctgagagatgagggtgcagcagagtgggggcctccactccagaccctgcagtctgggctggccaagggctgcaccggtgcactgcacgtcatggctgatgaagcacttccacaccgcagcccctcagagctgccacagtcagccttagttcaccgagggggaagctgaggcccagagcatgagagggacttgcccagggccacatagtccttagcagaggaagctgtggctgggtgactcgatctttgtcctttttctttatacccgcagtctccccatagcagaggcttttcttttttttttctttttcttttttttttttttacaagaactctttatatattaaggctgttgggctgaagaagcctgagagggtggctggttctgtggagcatggtttgttgaagtacagtttgggggcctcctacactgagaataggccttttctcgtttctccaaagagtgggctggctcaagtagggcagagagagaagcctggggcagaggttagggatgggcacccagcgcctgccctcacacgctctgtgctggtgtcttcacagccacgtgccaccctgggcagcatcccctgctcaccatctggctgtgcctgtttgctgggggcacctcattcagaatccagcttattgtttccaacggccaatggccacaccctggcaggtagcaagagtaggagagaggagacacccactccgagcacaggttgggtttggagcccggccttggggcactctgtcactcaaaggcagagtggggagtgggcactgggccttaggaggtactgggtccagtgaggcagagatgcccctgccccacccccaccttgtggcttcttccctggcctggccagagctgtctggccgccatggggccctgtgtctcctgccttgacctcccagagggcagccgaggcccaggggaggcctggggacttagcctctcagggcaggacctgtctgcaggagtaggtgggtgctgggggtcccagtggtaatgaggcatcaggcagtgtgggaaggggcccatccggcccaccccagggcctctgggcaggttgcaggttgtagcgctggatctaggctcctgcccagactgtaggttcaaccaagaatggcatgggagcccagcctgctgtttgctttattaaatctgccctgtagctgggggaggggcttactttgatcatcactatgtcattgatataaaaatagaggctcagagaggtgaatgaacctgcccaaagtcacacagcaaagtgtggagatgagatactgactcagggctgtggacactgaagcctgtgctctaacgccagtggctgtcgctccctgaggcattctctcccgaacaacacagttattatattacaaaatattatcactatatttatatatcttataataccttattattacaataaaaccttattactctacctttcaaaatgaattatttaaaaagcagtatttgctcattgcagagagtctagaaactatagaaaagcaagggaaaagcaataggaccagccccaaggtcccagcatgcacagataaccttagtaatactgggacgtgtgcttcctttttaacatctgagcccgtgtaggtcctgaagcccagcttctttctaagtccattgtcatcttgaccctggagcctggccgattttgctggggaggcccttgccagccgagagcggctcctgcctgtgccggcgtggcgcgcccctctgctgaggctgggcaggacaggggctgggccagctctgtttctcacccttggctcttgtgtctctcgtttcaggaaattaaaatgcatgacagatagcgagtccgccccgcccgactggccctattacctagccattgatgggattctggccaaggtccccgagtcctgtgatggcaaactgccggacagccagccgccggggccctccacgtcccagaccgaggcgtccctgtcgccgcccgctaagtccacccctctgtacttcccgtataaccagtgctcctacgaaggccgcttcgaggatgatcgctccgacagctcctccagcttactgtcccttaagttcaggtagtgtgtctgcttgtccttcccctgccctggggtatctcagcccccaccatttagagaaagggactgggagtggcaaggccggcggcggcggccacagtggttgcagaggccgtggctgcgggcagcgcctccagggacaggcggcctcagaccagggagggctttagtgtccacaggcagaccgagtttgtctcccagctccatcacttttgagctgcacggaaagttccttgacttctctggcctcagtctccctcctataaaatgggggtaaatcagtacctttctcagagggtggctgggagcatcacaggagagaagacgcagcatggggcccggcacacggagggagaccaagccccagaccccagaatgcgccccctggcctcccttagcccacacagaccccaccctcacaggctagctgccctctcagcactggggagggtgtcgggctgcacctcatcacgtgttgccgtgggcatgacccgtcccctctgccatccatcccacacctcagacccgtcccgtgctggccacgtgactgtgcctgcaagatgctcacagggcagccgggagccaggcagcatgcaggacagacacctgcggggtgggcctggggagcccagagaaggtgcttttgaggaggggacatttggggtgggctttcaaggtaaaatagaagttggccatttggaggcaagaacaggaagattgtggatttgagtcacagcttctcccctgccctggtcttcaagtctttctgacaggaggtgtcagaaaagtatctttagtagagaaggcgtctccgaggagggtccctctcatgccgggggccgctgcttgactcaggatttctcattgaagacctgagacaaaaacgcttttgctggcagctagaaggaaccagcaggaggcctgagatttgtggctgttgttcccgtggactgagcccagttctcagactcagctgcctggggccttgcacaggactggggcgtgggggctgccctccctgatcaggcccaaagcgcggatctcacgcccctgaggttggctgtaccctctcagctcagagcagagtgtgggccagggatgagcaggcactggagcagggccctggggtctgtgggttttggcagctccctgcccttcagggaggtctgctgagaccacgggtggcccctaccccagcagcagagctctcaggaggcgcccacagggctggactgcctttactcaccacctctaccagagctctgaggtcctggggagagagcccaggcctcttgtgggccccacaccctctaggtgcctgtccttctgcctctctaccaaggtgtgccggccccatttctaggccgccgggagataagggggctcacatctcaggcccttccttctgggacctcagtttccccatctgcctaaggccgggtggggctggtggtcttggcttccctacaggggtcctgagtactctgcactacccagcaccccccacccctgccttcatctctccctgggggtggtctctccacccctggcccccaactggggctgagcccccacctgcccagtttggtgggtgaagggtgctccctggcaggatatgcccctctgcagcccagaacatcccaccctttccagaccgaaggggtgtggattgtcctgggaccctggtcattggggtcatccgctagtcgcaaaggacggcaatgcctgtggcctctctttctttctttttctttttttttttttttgagacggagtctcgctcttgtgcagagagcagtggcgcgatcttggctcactgcaacctccgcctcgtgggttcaagcgattctcctgcctcagcctcccgagtagctgggattacaggcacccgccacaacgcctggctaatttttgtatttttagtagagatggggtttcaccatgttggccaggctggtcttgaactcctgacctcaggtgatccacctgcctctgcctcccaaagtgctgggattacaggcataagcctccacacccggccacccctgttactttctgtcaaaggcggtgggttctggcccctcctttgcacatggaatatgagaccctgagtaagtgacctgactccctggggcctcagtttccccatttgcccagtaggattgtcgggagggtccggtgaggcccctggtgtgcccaggctctgtggccagcacgtccacagccggcactgtccttccaggtcggaggagcggccggtgaagaagcgcaaggtgcagagctgccacctgcagaagaagcagctgcggctgctggaggccatggtggaggagcagcgccggctgagccgcgccgtggaggagacctgccgcgaggtgcgccgcgtgctggaccagcagcacatcctgcaggtgcagagcctgcagctgcaggagcgcatgatgagtctgctggagaggatcatcaccaagtccagcgtctaggccagcaggcggcggcggcggcggggccgggcggctggtggtactgctcaggccacccagggcaggccactcaggccaggcgggcaagggggccgccccgcgagcggagaccgccttccacctggcctctggcaggatgtcccttctgaggggtattttgaggaacccccaggccctggggaccgtgaggctccagtctccagcatgaatgcccttcctcggacacaggccagggcctctggggttcactccgagtaagaacgtcctagagccactctccagtgtcgttactatcaatgatacttgacgtggctttgatattaaacgtatactttttcattcttgcctggaacgcacagtttgctgttgctggcttggtgaggatgccctgattgatggatcccgaaaatgaaagcagatggaaacgggttggggcaggctggagctgggggagctctctcctgaagggaaccctgtgtcctccctcaccaggacctctgcgtctctccttaaatggcctctgacgcctgatgaaaaccccagcgaccttccaggaggcttttattcagctctgtttggagcatcaggtgtttccactgcctccttagcaatgacactaataaaagtcgtaacacctgttcacatgcacagccctgttgagtgttctgggtgctggagatatcatggtggatgacacaaaggccctggcctcttggagcttatgctcccatgcggggaagacacatgggtcagtagagaaatggttgcaggttgtgataagtgctggaagggaggggttggcctgaggacacggaggcagacatacgtggagctgggaacagtggccacacagggaacggccagtgcgaaggcccagaggcagaggacactggagcaagcccaggagcagctaggaggctggtggccagcagccaggccacggaagcccgtgcagcccgtggggaggagtgttcatgcttttcaagcttagtgggagtcttttggccagtgcagctctgggtctgacatcggtgggggacagaggggtggtggagcggccacagctgcaagctcacctcactgccggcccttccaccagtttcaaactctttctagaagctccagctttcccaaagctgaattctctatgagcctccttggccgggactcgggcgtctggttgccctggctgcaaaggaggctggggccaggtgtgtttgagtcacctcctggaattaggcaagttgctgcccaaatagaaggttgttggcaggtgggtcagcaggtgaacagcatggtttgactcagggttcagaaaaatctccctctggctgccaagcgagcaggccgtggagacaggtgcagaggcaggtgtggcagcaggcatcctgccaggcagtgctgcagtcatcctgcgacaagcagcagcagctcatcctaccctctagggggtcttgaggtcagccaggcaagagagcagcttggactccactgggtgtgggaccagcctgtggaccatggtggtgtggagggtgccctcggcctgcctgtgtgaaggagaggccggcgtgttctgtggagcccaaaggggagctgggcaagcaggattcacttcactctgagggtcctggagctcccaccctcctcagccatctccccagagcctgtgtgccgaggactcggcccatgttgctgtgggatgagaggcagagtgtcgtgagggtgtaaggagcggcggcagtggtgggaggagggagcagcagccagcgctacggtgccagtttccagctgccagatgacgccgctgaccctgtggttgagaagagatgcacagagccagctcttgcaagccagtgtggctgccatagcacctgccgagaagcagaaggaagggtggccccaggaggacagaggatgcgggcacatctgatgcgggcctgagttttgggagcttttgctctagccagtttccagctccgggacccacccgcctcgtaggcaagacaccacccaagaaatcatttgcttaacaaacacactgggctccaactggacacctgtgccaccctagatgctgggaacccagccatgacacaggcacctgcccccagctgctgaccactgaggctggctagcagctcccatggggccagtgtggggttccccagcctcctaacagggagccagtcacaagccctcgagagggaagggtgcccgcggccctggcaggaaggttaggctggacgctcccacaagacataacagatggaggttctaaatgatgtagcaacttcttcaccctgaaactgctgtagagtcagccatgacgcaccggtacttcagtaactgccaggcatccgggacagcacaccgcgagtcgctgctgtgcttgggttagaagtggtttggtctgttttcttctcgccctctctaatcagagtcagtgattcatgcccttccatcaccttagagaaggggcaggcgctgcccgaccttctccaggctggagcagcatcgcctcatgtcagcagaactcagctgtagaatatcgtggggttggtgcctttcatcagcagcatgtccttaacaactttctgatttcttccttagttgttggtccattaaggagaaaaaaaatgatctcagccattgctaaaatatttgataagattcagcaaagcagcatgttaacattgaaaactagaatcaggagccaggcagatgtgcttgcttttcacctgtagtatttcatgttgttttgacgtttttagctaatgcattaagataaataaacaaaagccgggcacggtggttcacgcctgtaatcccagcactttgggaggctgaggcgggaggatcctctgaggtcaggagttcaagaccagcctgaccaacatggagaaacctcgtcattactaaaaatacaaaattagctgggcgtggtggtgcatgcctgtaatcccagctacttgggaggctgaggcaggagaatcgcttgaacccgggaggcggaggttgcagtgagctgagattgcaccactgcactccagcctgggtgacagtgaaactcggtctcaaaaaaaaaaaaaaattaaaaaaagataaataaaataagcaggataagaaatgaagaaagtagagttacctttgttttcagatttcatttttgtatacccagaaagccaaatgtacaaaagactgggagctctttaaaccagcttaaacttgttgaaaatgaggatgaagaaatatcccattcagagttggaatgaatttaacccagaaggaacaggacctctactgaagagaactatgcagtcttactgaaaaatctaaataatacctgagcgctggagaaacttcgcacactcctgaaagctccaaagtcaatgtcatcattttattaatgtcattccaaacatagtctcaataatatcacttcttggttttgacatggacgcgatgatgtttaaattcatatgaaaaaagaacggggccaaaagtccaaggccagtcagcgtgagaagaccgctcggcctccctcggagtcggggagttggaaccgcagactgagatcatgtggctgctggaggccaggacgaacgtcgggaaatggagactcctgcgttgctggtgggatgtggtgcagccgcttccaggagcaatttggtgtcccgtcctaaagctgaagaaacgcatttcctctggtcagtgccactcctagacaggccaccctgcggcagccgtcctcaaactggtctgaggacccctcaacgctcttaaaaatcattaaaagtgggccaggtgcggtggctcacacctgtaatcccagcactttgggaggccaagacaggcggatcacgaggtcaggacattgagatcatcctggctaacacggtgaaaccccgtctctactaaaaatacaaaaaattagccgggcgtggtggcgggcgcctgtagtcccagctacttgggaggctgagccaggagaatggcgtgaacccaggaggtggagcttgcagtgagctgagatcactccactgcactccagcctgggcagcagagcgagactctgtctcaaaaaaaaataataaataaataaataaaaataaaataaaataaaattcattaaaagtgccaaagaacttttgcttatgtgagttctaatgaccaatattaatacacattagaatatcttattagaaattaaacctgagacctttagaaaacatgtattcatttcaaaatagcaataaacccatgacatattaacataaataacaattgtatgaaaaatatattttccaaaacaaaaagttttcgggagaagtgtggcatagttttacatggtcgtaaatctctggcttaagagaagcccactggcctctcagcaggctctgggtccgtccactttgggggtgttttggttgtgaagtataggagtgaatggagaagctcattcttacccagatgtgtatttgaaaagaaaaggaacattttaataacctttgcaaataatcggtatattcttccgtgatcctattccaacactggacaggtggtggtttgttttttttttttggagacggagtcccgctctgtcactcaggctggagtgcagtggcgcgatttcagctcactgcaagctccgcctcc

SEQ ID NO: 2 - RNA, 13481 nt, Homo sapiens
  source 1..13481: mol_type = mRNA
gctgccgggacgggtccaagatggacggccgctcaggttctgcttttacctgcggcccagagccccattcattgccccggtgctgagcggcgccgcgagtcggcccgaggcctccggggactgccgtgccgggcgggagaccgccatggcgaccctggaaaagctgatgaaggccttcgagtccctcaagtccttccagcagcagcagcagcagcagcagcagcagcagcagcagcagcagcagcagcagcagcagcagcaacagccgccaccgccgccgccgccgccgccgcctcctcagcttcctcagccgccgccgcaggcacagccgctgctgcctcagccgcagccgcccccgccgccgcccccgccgccacccggcccggctgtggctgaggagccgctgcaccgaccaaagaaagaactttcagctaccaagaaagaccgtgtgaatcattgtctgacaatatgtgaaaacatagtggcacagtctgtcagaaattctccagaatttcagaaacttctgggcatcgctatggaactttttctgctgtgcagtgatgacgcagagtcagatgtcaggatggtggctgacgaatgcctcaacaaagttatcaaagctttgatggattctaatcttccaaggttacagctcgagctctataaggaaattaaaaagaatggtgcccctcggagtttgcgtgctgccctgtggaggtttgctgagctggctcacctggttcggcctcagaaatgcaggccttacctggtgaaccttctgccgtgcctgactcgaacaagcaagagacccgaagaatcagtccaggagaccttggctgcagctgttcccaaaattatggcttcttttggcaattttgcaaatgacaatgaaattaaggttttgttaaaggccttcatagcgaacctgaagtcaagctcccccaccattcggcggacagcggctggatcagcagtgagcatctgccagcactcaagaaggacacaatatttctatagttggctactaaatgtgctcttaggcttactcgttcctgtcgaggatgaacactccactctgctgattcttggcgtgctgctcaccctgaggtatttggtgcccttgctgcagcagcaggtcaaggacacaagcctgaaaggcagcttcggagtgacaaggaaagaaatggaagtctctccttctgcagagcagcttgtccaggtttatgaactgacgttacatcatacacagcaccaagaccacaatgttgtgaccggagccctggagctgttgcagcagctcttcagaacgcctccacccgagcttctgcaaaccctgaccgcagtcgggggcattgggcagctcaccgctgctaaggaggagtctggtggccgaagccgtagtgggagtattgtggaacttatagctggagggggttcctcatgcagccctgtcctttcaagaaaacaaaaaggcaaagtgctcttaggagaagaagaagccttggaggatgactctgaatcgagatcggatgtcagcagctctgccttaacagcctcagtgaaggatgagatcagtggagagctggctgcttcttcaggggtttccactccagggtcagcaggtcatgacatcatcacagaacagccacggtcacagcacacactgcaggcggactcagtggatctggccagctgtgacttgacaagctctgccactgatggggatgaggaggatatcttgagccacagctccagccaggtcagcgccgtcccatctgaccctgccatggacctgaatgatgggacccaggcctcgtcgcccatcagcgacagctcccagaccaccaccgaagggcctgattcagctgttaccccttcagacagttctgaaattgtgttagacggtaccgacaaccagtatttgggcctgcagattggacagccccaggatgaagatgaggaagccacaggtattcttcctgatgaagcctcggaggccttcaggaactcttccatggcccttcaacaggcacatttattgaaaaacatgagtcactgcaggcagccttctgacagcagtgttgataaatttgtgttgagagatgaagctactgaaccgggtgatcaagaaaacaagccttgccgcatcaaaggtgacattggacagtccactgatgatgactctgcacctcttgtccattgtgtccgccttttatctgcttcgtttttgctaacagggggaaaaaatgtgctggttccggacagggatgtgagggtcagcgtgaaggccctggccctcagctgtgtgggagcagctgtggccctccacccggaatctttcttcagcaaactctataaagttcctcttgacaccacggaataccctgaggaacagtatgtctcagacatcttgaactacatcgatcatggagacccacaggttcgaggagccactgccattctctgtgggaccctcatctgctccatcctcagcaggtcccgcttccacgtgggagattggatgggcaccattagaaccctcacaggaaatacattttctttggcggattgcattcctttgctgcggaaaacactgaaggatgagtcttctgttacttgcaagttagcttgtacagctgtgaggaactgtgtcatgagtctctgcagcagcagctacagtgagttaggactgcagctgatcatcgatgtgctgactctgaggaacagttcctattggctggtgaggacagagcttctggaaacccttgcagagattgacttcaggctggtgagctttttggaggcaaaagcagaaaacttacacagaggggctcatcattatacagggcttttaaaactgcaagaacgagtgctcaataatgttgtcatccatttgcttggagatgaagaccccagggtgcgacatgttgccgcagcatcactaattaggcttgtcccaaagctgttttataaatgtgaccaaggacaagctgatccagtagtggccgtggcaagagatcaaagcagtgtttacctgaaacttctcatgcatgagacgcagcctccatctcatttctccgtcagcacaataaccagaatatatagaggctataacctactaccaagcataacagacgtcactatggaaaataacctttcaagagttattgcagcagtttctcatgaactaatcacatcaaccaccagagcactcacatttggatgctgtgaagctttgtgtcttctttccactgccttcccagtttgcatttggagtttaggttggcactgtggagtgcctccactgagtgcctcagatgagtctaggaagagctgtaccgttgggatggccacaatgattctgaccctgctctcgtcagcttggttcccattggatctctcagcccatcaagatgctttgattttggccggaaacttgcttgcagccagtgctcccaaatctctgagaagttcatgggcctctgaagaagaagccaacccagcagccaccaagcaagaggaggtctggccagccctgggggaccgggccctggtgcccatggtggagcagctcttctctcacctgctgaaggtgattaacatttgtgcccacgtcctggatgacgtggctcctggacccgcaataaaggcagccttgccttctctaacaaaccccccttctctaagtcccatccgacgaaaggggaaggagaaagaaccaggagaacaagcatctgtaccgttgagtcccaagaaaggcagtgaggccagtgcagcttctagacaatctgatacctcaggtcctgttacaacaagtaaatcctcatcactggggagtttctatcatcttccttcatacctcaaactgcatgatgtcctgaaagctacacacgctaactacaaggtcacgctggatcttcagaacagcacggaaaagtttggagggtttctccgctcagccttggatgttctttctcagatactagagctggccacactgcaggacattgggaagtgtgttgaagagatcctaggatacctgaaatcctgctttagtcgagaaccaatgatggcaactgtttgtgttcaacaattgttgaagactctctttggcacaaacttggcctcccagtttgatggcttatcttccaaccccagcaagtcacaaggccgagcacagcgccttggctcctccagtgtgaggccaggcttgtaccactactgcttcatggccccgtacacccacttcacccaggccctcgctgacgccagcctgaggaacatggtgcaggcggagcaggagaacgacacctcgggatggtttgatgtcctccagaaagtgtctacccagttgaagacaaacctcacgagtgtcacaaagaaccgtgcagataagaatgctattcataatcacattcgtttgtttgaacctcttgttataaaagctttaaaacagtacacgactacaacatgtgtgcagttacagaagcaggttttagatttgctggcgcagctggttcagttacgggttaattactgtcttctggattcagatcaggtgtttattggctttgtattgaaacagtttgaatacattgaagtgggccagttcagggaatcagaggcaatcattccaaacatctttttcttcttggtattactatcttatgaacgctatcattcaaaacagatcattggaattcctaaaatcattcagctctgtgatggcatcatggccagtggaaggaaggctgtgacacatgccataccggctctgcagcccatagtccacgacctctttgtattaagaggaacaaataaagctgatgcaggaaaagagcttgaaacccaaaaagaggtggtggtgtcaatgttactgagactcatccagtaccatcaggtgttggagatgttcattcttgtcctgcagcagtgccacaaggagaatgaagacaagtggaagcgactgtctcgacagatagctgacatcatcctcccaatgttagccaaacagcagatgcacattgactctcatgaagcccttggagtgttaaatacattatttgagattttggccccttcctccctccgtccggtagacatgcttttacggagtatgttcgtcactccaaacacaatggcgtccgtgagcactgttcaactgtggatatcgggaattctggccattttgagggttctgatttcccagtcaactgaagatattgttctttctcgtattcaggagctctccttctctccgtatttaatctcctgtacagtaattaataggttaagagatggggacagtacttcaacgctagaagaacacagtgaagggaaacaaataaagaatttgccagaagaaacattttcaaggtttctattacaactggttggtattcttttagaagacattgttacaaaacagctgaaggtggaaatgagtgagcagcaacatactttctattgccaggaactaggcacactgctaatgtgtctgatccacatcttcaagtctggaatgttccggagaatcacagcagctgccactaggctgttccgcagtgatggctgtggcggcagtttctacaccctggacagcttgaacttgcgggctcgttccatgatcaccacccacccggccctggtgctgctctggtgtcagatactgctgcttgtcaaccacaccgactaccgctggtgggcagaagtgcagcagaccccgaaaagacacagtctgtccagcacaaagttacttagtccccagatgtctggagaagaggaggattctgacttggcagccaaacttggaatgtgcaatagagaaatagtacgaagaggggctctcattctcttctgtgattatgtctgtcagaacctccatgactccgagcacttaacgtggctcattgtaaatcacattcaagatctgatcagcctttcccacgagcctccagtacaggacttcatcagtgccgttcatcggaactctgctgccagcggcctgttcatccaggcaattcagtctcgttgtgaaaacctttcaactccaaccatgctgaagaaaactcttcagtgcttggaggggatccatctcagccagtcgggagctgtgctcacgctgtatgtggacaggcttctgtgcacccctttccgtgtgctggctcgcatggtcgacatccttgcttgtcgccgggtagaaatgcttctggctgcaaatttacagagcagcatggcccagttgccaatggaagaactcaacagaatccaggaataccttcagagcagcgggctcgctcagagacaccaaaggctctattccctgctggacaggtttcgtctctccaccatgcaagactcacttagtccctctcctccagtctcttcccacccgctggacggggatgggcacgtgtcactggaaacagtgagtccggacaaagactggtacgttcatcttgtcaaatcccagtgttggaccaggtcagattctgcactgctggaaggtgcagagctggtgaatcggattcctgctgaagatatgaatgccttcatgatgaactcggagttcaacctaagcctgctagctccatgcttaagcctagggatgagtgaaatttctggtggccagaagagtgccctttttgaagcagcccgtgaggtgactctggcccgtgtgagcggcaccgtgcagcagctccctgctgtccatcatgtcttccagcccgagctgcctgcagagccggcggcctactggagcaagttgaatgatctgtttggggatgctgcactgtatcagtccctgcccactctggcccgggccctggcacagtacctggtggtggtctccaaactgcccagtcatttgcaccttcctcctgagaaagagaaggacattgtgaaattcgtggtggcaacccttgaggccctgtcctggcatttgatccatgagcagatcccgctgagtctggatctccaggcagggctggactgctgctgcctggccctgcagctgcctggcctctggagcgtggtctcctccacagagtttgtgacccacgcctgctccctcatctactgtgtgcacttcatcctggaggccgttgcagtgcagcctggagagcagcttcttagtccagaaagaaggacaaataccccaaaagccatcagcgaggaggaggaggaagtagatccaaacacacagaatcctaagtatatcactgcagcctgtgagatggtggcagaaatggtggagtctctgcagtcggtgttggccttgggtcataaaaggaatagcggcgtgccggcgtttctcacgccattgctaaggaacatcatcatcagcctggcccgcctgccccttgtcaacagctacacacgtgtgcccccactggtgtggaagcttggatggtcacccaaaccgggaggggattttggcacagcattccctgagatccccgtggagttcctccaggaaaaggaagtctttaaggagttcatctaccgcatcaacacactaggctggaccagtcgtactcagtttgaagaaacttgggccaccctccttggtgtcctggtgacgcagcccctcgtgatggagcaggaggagagcccaccagaagaagacacagagaggacccagatcaacgtcctggccgtgcaggccatcacctcactggtgctcagtgcaatgactgtgcctgtggccggcaacccagctgtaagctgcttggagcagcagccccggaacaagcctctgaaagctctcgacaccaggtttgggaggaagctgagcattatcagagggattgtggagcaagagattcaagcaatggtttcaaagagagagaatattgccacccatcatttatatcaggcatgggatcctgtcccttctctgtctccggctactacaggtgccctcatcagccacgagaagctgctgctacagatcaaccccgagcgggagctggggagcatgagctacaaactcggccaggtgtccatacactccgtgtggctggggaacagcatcacacccctgagggaggaggaatgggacgaggaagaggaggaggaggccgacgcccctgcaccttcgtcaccacccacgtctccagtcaactccaggaaacaccgggctggagttgacatccactcctgttcgcagtttttgcttgagttgtacagccgctggatcctgccgtccagctcagccaggaggaccccggccatcctgatcagtgaggtggtcagatcccttctagtggtctcagacttgttcaccgagcgcaaccagtttgagctgatgtatgtgacgctgacagaactgcgaagggtgcacccttcagaagacgagatcctcgctcagtacctggtgcctgccacctgcaaggcagctgccgtccttgggatggacaaggccgtggcggagcctgtcagccgcctgctggagagcacgctcaggagcagccacctgcccagcagggttggagccctgcacggcgtcctctatgtgctggagtgcgacctgctggacgacactgccaagcagctcatcccggtcatcagcgactatctcctctccaacctgaaagggatcgcccactgcgtgaacattcacagccagcagcacgtactggtcatgtgtgccactgcgttttacctcattgagaactatcctctggacgtagggccggaattttcagcatcaataatacagatgtgtggggtgatgctgtctggaagtgaggagtccaccccctccatcatttaccactgtgccctcagaggcctggagcgcctcctgctctctgagcagctctcccgcctggatgcagaatcgctggtcaagctgagtgtggacagagtgaacgtgcacagcccgcaccgggccatggcggctctgggcctgatgctcacctgcatgtacacaggaaaggagaaagtcagtccgggtagaacttcagaccctaatcctgcagcccccgacagcgagtcagtgattgttgctatggagcgggtatctgttctttttgataggatcaggaaaggctttccttgtgaagccagagtggtggccaggatcctgccccagtttctagacgacttcttcccaccccaggacatcatgaacaaagtcatcggagagtttctgtccaaccagcagccatacccccagttcatggccaccgtggtgtataaggtgtttcagactctgcacagcaccgggcagtcgtccatggtccgggactgggtcatgctgtccctctccaacttcacgcagagggccccggtcgccatggccacgtggagcctctcctgcttctttgtcagcgcgtccaccagcccgtgggtcgcggcgatcctcccacatgtcatcagcaggatgggcaagctggagcaggtggacgtgaaccttttctgcctggtcgccacagacttctacagacaccagatagaggaggagctcgaccgcagggccttccagtctgtgcttgaggtggttgcagccccaggaagcccatatcaccggctgctgacttgtttacgaaatgtccacaaggtcaccacctgctgagcgccatggtgggagagactgtgaggcggcagctggggccggagcctttggaagtctgcgcccttgtgccctgcctccaccgagccagcttggtccctatgggcttccgcacatgccgcgggcggccaggcaacgtgcgtgtctctgccatgtggcagaagtgctctttgtggcagtggccaggcagggagtgtctgcagtcctggtggggctgagcctgaggccttccagaaagcaggagcagctgtgctgcaccccatgtgggtgaccaggtcctttctcctgatagtcacctgctggttgttgccaggttgcagctgctcttgcatctgggccagaagtcctccctcctgcaggctggctgttggcccctctgctgtcctgcagtagaaggtgccgtgagcaggctttgggaacactggcctgggtctccctggtggggtgtgcatgccacgccccgtgtctggatgcacagatgccatggcctgtgctgggccagtggctgggggtgctagacacccggcaccattctcccttctctcttttcttctcaggatttaaaatttaattatatcagtaaagagattaattttaacgtaactctttctatgcccgtgtaaagtatgtgaatcgcaaggcctgtgctgcatgcgacagcgtccggggtggtggacagggcccccggccacgctccctctcctgtagccactggcatagccctcctgagcacccgctgacatttccgttgtacatgttcctgtttatgcattcacaaggtgactgggatgtagagaggcgttagtgggcaggtggccacagcaggactgaggacaggcccccattatcctaggggtgcgctcacctgcagcccctcctcctcgggcacagacgactgtcgttctccacccaccagtcagggacagcagcctccctgtcactcagctgagaaggccagccctccctggctgtgagcagcctccactgtgtccagagacatgggcctcccactcctgttccttgctagccctggggtggcgtctgcctaggagctggctggcaggtgttgggacctgctgctccatggatgcatgccctaagagtgtcactgagctgtgttttgtctgagcctctctcggtcaacagcaaagcttggtgtcttggcactgttagtgacagagcccagcatcccttctgcccccgttccagctgacatcttgcacggtgaccccttttagtcaggagagtgcagatctgtgctcatcggagactgccccacggccctgtcagagccgccactcctatccccaggccaggtccctggaccagcctcctgtttgcaggcccagaggagccaagtcattaaaatggaagtggattctggatggccgggctgctgctgatgtaggagctggatttgggagctctgcttgccgactggctgtgagacgaggcaggggctctgcttcctcagccctagaggcgagccaggcaaggttggcgactgtcatgtggcttggtttggtcatgcccgtcgatgttttgggtattgaatgtggtaagtggaggaaatgttggaactctgtgcaggtgctgccttgagacccccaagcttccacctgtccctctcctatgtggcagctggggagcagctgagatgtggacttgtatgctgcccacatacgtgagggggagctgaaagggagcccctcctctgagcagcctctgccaggcctgtatgaggcttttcccaccagctcccaacagaggcctcccccagccaggaccacctcgtcctcgtggcggggcagcaggagcggtagaaaggggtccgatgtttgaggaggcccttaagggaagctactgaattataacacgtaagaaaatcaccattccgtattggttgggggctcctgtttctcatcctagctttttcctggaaagcccgctagaaggtttgggaacgaggggaaagttctcagaactgttggctgctccccacccgcctcccgcctcccccgcaggttatgtcagcagctctgagacagcagtatcacaggccagatgttgttcctggctagatgtttacatttgtaagaaataacactgtgaatgtaaaacagagccattcccttggaatgcatatcgctgggctcaacatagagtttgtcttcctcttgtttacgacgtgatctaaaccagtccttagcaaggggctcagaacaccccgctctggcagtaggtgtcccccacccccaaagacctgcctgtgtgctccggagatgaatatgagctcattagtaaaaatgacttcacccacgcatatacataaagtatccatgcatgtgcatatagacacatctataattttacacacacacctctcaagacggagatgcatggcctctaagagtgcccgtgtcggttcttcctggaagttgactttccttagacccgccaggtcaagttagccgcgtgacggacatccaggcgtgggacgtggtcagggcagggctcattcattgcccactaggatcccactggcgaagatggtctccatatcagctctctgcagaagggaggaagactttatcatgttcctaaaaatctgtggcaagcacccatcgtattatccaaattttgttgcaaatgtgattaatttggttgtcaagttttgggggtgggctgtggggagattgcttttgttttcctgctggtaatatcgggaaagattttaatgaaaccagggtagaattgtttggcaatgcactgaagcgtgtttctttcccaaaatgtgcctcccttccgctgcgggcccagctgagtctatgtaggtgatgtttccagctgccaagtgctctttgttactgtccaccctcatttctgccagcgcatgtgtcctttcaaggggaaaatgtgaagctgaaccccctccagacacccagaatgtagcatctgagaaggccctgtgccctaaaggacacccctcgcccccatcttcatggagggggtcatttcagagccctcggagccaatgaacagctcctcctcttggagctgagatgagccccacgtggagctcgggacggatagtagacagcaataactcggtgtgtggccgcctggcaggtggaacttcctcccgttgcggggtggagtgaggttagttctgtgtgtctggtgggtggagtcaggcttctcttgctacctgtgagcatccttcccagcagacatcctcatcgggctttgtccctcccccgcttcctccctctgcggggaggacccgggaccacagctgctggccagggtagacttggagctgtcctccagaggggtcacgtgtaggagtgagaagaaggaagatcttgagagctgctgagggaccttggagagctcaggatggctcagacgaggacactcgcttgccgggcctgggcctcctgggaaggagggagctgctcagaatgccgcatgacaactgaaggcaacctggaaggttcaggggccgctcttcccccatgtgcctgtcacgctctggtgcagtcaaaggaacgccttcccctcagttgtttctaagagcagagtctcccgctgcaatctgggtggtaactgccagccttggaggatcgtggccaacgtggacctgcctacggagggtgggctctgacccaagtggggcctccttgtccaggtctcactgctttgcaccgtggtcagagggactgtcagctgagcttgagctcccctggagccagcagggctgtgatgggcgagtcccggagccccacccagacctgaatgcttctgagagcaaagggaaggactgacgagagatgtatatttaattttttaactgctgcaaacattgtacatccaaattaaaggaaaaaaatggaaaccatca

SEQ ID NO: 3 - DNA, 20 bp, synthetic construct
  source 1..20: mol_type = other DNA
ctccgtccggtagacatgct

SEQ ID NO: 4 - DNA, 23 bp, synthetic construct
  source 1..23: mol_type = other DNA
ggaaatcagaaccctcaaaatgg

SEQ ID NO: 5 - DNA, 29 bp, synthetic construct
  source 1..29: mol_type = other DNA
tgagcactgttcaactgtggatatcggga

SEQ ID NO: 6 - DNA, 20 bp, synthetic construct
  source 1..20: mol_type = other DNA
tctctattgcacattccaag

SEQ ID NO: 7 - DNA, 20 bp, synthetic construct
  source 1..20: mol_type = other DNA
gccgtagcctgggacccgcc

SEQ ID NO: 8 - DNA, 19 bp, synthetic construct
  source 1..19: mol_type = other DNA
taacactcgattaaccctg

SEQ ID NO: 9 - DNA, 19 bp, synthetic construct
  source 1..19: mol_type = other DNA
taacacttgattaaccctg

SEQ ID NO: 10 - DNA, 19 bp, synthetic construct
  source 1..19: mol_type = other DNA
gttaacactcgattaaccc

SEQ ID NO: 11 - DNA, 19 bp, synthetic construct
  source 1..19: mol_type = other DNA
gttaacacttgattaaccc

SEQ ID NO: 12 - DNA, 19 bp, synthetic construct
  source 1..19: mol_type = other DNA
gctagttcatcccagtgag

SEQ ID NO: 13 - DNA, 19 bp, synthetic construct
  source 1..19: mol_type = other DNA
gctagttcaccccagtgag

SEQ ID NO: 14 - DNA, 19 bp, synthetic construct
  source 1..19: mol_type = other DNA
tggaaatgggtttttccac

SEQ ID NO: 15 - DNA, 19 bp, synthetic construct
  source 1..19: mol_type = other DNA
tggaaatggctttttccac

SEQ ID NO: 16 - DNA, 19 bp, synthetic construct
  source 1..19: mol_type = other DNA
tttaaccgtggcatgggca

SEQ ID NO: 17 - DNA, 19 bp, synthetic construct
  source 1..19: mol_type = other DNA
tttaaccgtagcatgggca

SEQ ID NO: 18 - DNA, 19 bp, synthetic construct
  source 1..19: mol_type = other DNA
ttcaagctagtaacgatgc

SEQ ID NO: 19 - DNA, 19 bp, synthetic construct
  source 1..19: mol_type = other DNA
ttcaagccagtaacgatgc

SEQ ID NO: 20 - DNA, 19 bp, synthetic construct
  source 1..19: mol_type = other DNA
acttcaagctagtaacgat

SEQ ID NO: 21 - DNA, 19 bp, synthetic construct
  source 1..19: mol_type = other DNA
acttcaagccagtaacgat

SEQ ID NO: 22 - DNA, 19 bp, synthetic construct
  source 1..19: mol_type = other DNA
gcagctaggttaaagagtc

SEQ ID NO: 23 - DNA, 19 bp, synthetic construct
  source 1..19: mol_type = other DNA
gcagctaggctaaagagtc

SEQ ID NO: 24 - DNA, 19 bp, synthetic construct
  source 1..19: mol_type = other DNA
aataagaaacacaatcaaa

SEQ ID NO: 25 - DNA, 19 bp, synthetic construct
  source 1..19: mol_type = other DNA
aataagaaatacaatcaaa

SEQ ID NO: 26 - DNA, 19 bp, synthetic construct
  source 1..19: mol_type = other DNA
cagaggaggcatactgtat

SEQ ID NO: 27 - DNA, 19 bp, synthetic construct
  source 1..19: mol_type = other DNA
cagaggaggtatactgtat

SEQ ID NO: 28 - DNA, 19 bp, synthetic construct
  source 1..19: mol_type = other DNA
cacagtgctacccaacctt

SEQ ID NO: 29 - DNA, 19 bp, synthetic construct
  source 1..19: mol_type = other DNA
cacagtgctccccaacctt

SEQ ID NO: 30 - DNA, 19 bp, synthetic construct
  source 1..19: mol_type = other DNA
taattttctagactttatg

SEQ ID NO: 31 - DNA, 19 bp, synthetic construct
  source 1..19: mol_type = other DNA
taattttctggactttatg

SEQ ID NO: 32 - DNA, 19 bp, synthetic construct
  source 1..19: mol_type = other DNA
gctacaacgcaggtcaaat

SEQ ID NO: 33 - DNA, 19 bp, synthetic construct
  source 1..19: mol_type = other DNA
gctacaatgcaggtcaaat

SEQ ID NO: 34 - DNA, 19 bp, synthetic construct
  source 1..19: mol_type = other DNA
gagctacaacgcaggtcaa

SEQ ID NO: 35 - DNA, 19 bp, synthetic construct
  source 1..19: mol_type = other DNA
gagctacaatgcaggtcaa

SEQ ID NO: 36 - DNA, 19 bp, synthetic construct
  source 1..19: mol_type = other DNA
agagagaacgagaaggctc

SEQ ID NO: 37 - DNA, 19 bp, synthetic construct
  source 1..19: mol_type = other DNA
agagagaacaagaaggctc

SEQ ID NO: 38 - DNA, 19 bp, synthetic construct
  source 1..19: mol_type = other DNA
agcccctctgtgtaagttt

SEQ ID NO: 39 - DNA, 19 bp, synthetic construct
  source 1..19: mol_type = other DNA
agcccttctgtgtaagttt

SEQ ID NO: 40 - DNA, 19 bp, synthetic construct
  source 1..19: mol_type = other DNA
gagcccctctgtgtaagtt

SEQ ID NO: 41 - DNA, 19 bp, synthetic construct
  source 1..19: mol_type = other DNA
gagcccttctgtgtaagtt

SEQ ID NO: 42 - DNA, 19 bp, synthetic construct
  source 1..19: mol_type = other DNA
tgagcccctctgtgtaagt

SEQ ID NO: 43 - DNA, 19 bp, synthetic construct
  source 1..19: mol_type = other DNA
tgagcccttctgtgtaagt

SEQ ID NO: 44 - DNA, 19 bp, synthetic construct
  source 1..19: mol_type = other DNA
atgagcccctctgtgtaag

SEQ ID NO: 45 - DNA, 19 bp, synthetic construct
  source 1..19: mol_type = other DNA
atgagcccttctgtgtaag

SEQ ID NO: 46 - DNA, 19 bp, synthetic construct
  source 1..19: mol_type = other DNA
gatgagcccctctgtgtaa

SEQ ID NO: 47 - DNA, 19 bp, synthetic construct
  source 1..19: mol_type = other DNA
gatgagcccttctgtgtaa

SEQ ID NO: 48 - DNA, 19 bp, synthetic construct
  source 1..19: mol_type = other DNA
tgatgagcccctctgtgta

SEQ ID NO: 49 - DNA, 19 bp, synthetic construct
  source 1..19: mol_type = other DNA
tgatgagcccttctgtgta

SEQ ID NO: 50 - DNA, 19 bp, synthetic construct
  source 1..19: mol_type = other DNA
atgatgagcccctctgtgt

SEQ ID NO: 51 - DNA, 19 bp, synthetic construct
  source 1..19: mol_type = other DNA
atgatgagcccttctgtgt

SEQ ID NO: 52 - DNA, 19 bp, synthetic construct
  source 1..19: mol_type = other DNA
taatgatgagcccctctgt

SEQ ID NO: 53 - DNA, 19 bp, synthetic construct
  source 1..19: mol_type = other DNA
taatgatgagcccttctgt

SEQ ID NO: 54 - DNA, 19 bp, synthetic construct
  source 1..19: mol_type = other DNA
agaatacgggtaacatttt

SEQ ID NO: 55 - DNA, 19 bp, synthetic construct
  source 1..19: mol_type = other DNA
agaatacaggtaacatttt

SEQ ID NO: 56 - DNA, 19 bp, synthetic construct
  source 1..19: mol_type = other DNA
ggagaatacgggtaacatt

SEQ ID NO: 57 - DNA, 19 bp, synthetic construct
  source 1..19: mol_type = other DNA
ggagaatacaggtaacatt

SEQ ID NO: 58 - DNA, 19 bp, synthetic construct
  source 1..19: mol_type = other DNA
ttagtaatcaattttaatg

SEQ ID NO: 59 - DNA, 19 bp, synthetic construct
  source 1..19: mol_type = other DNA
ttagtaaccaattttaatg

SEQ ID NO: 60 - DNA, 19 bp, synthetic construct
  source 1..19: mol_type = other DNA
agttagtaatcaattttaa

SEQ ID NO: 61 - DNA, 19 bp, synthetic construct
  source 1..19: mol_type = other DNA
agttagtaaccaattttaa

SEQ ID NO: 62 - DNA, 19 bp, synthetic construct
  source 1..19: mol_type = other DNA
gaaggaatgcttttactag

SEQ ID NO: 63 - DNA, 19 bp, synthetic construct
  source 1..19: mol_type = other DNA
gaaggaatgtttttactag

SEQ ID NO: 64 - DNA, 19 bp, synthetic construct
  source 1..19: mol_type = other DNA
ctaaaactaacttgagaat

SEQ ID NO: 65 - DNA, 19 bp, synthetic construct
  source 1..19: mol_type = other DNA
ctaaaaccaacttgagaat

SEQ ID NO: 66 - DNA, 19 bp, synthetic construct
  source 1..19: mol_type = other DNA
atctaaaactaacttgaga

SEQ ID NO: 67 - DNA, 19 bp, synthetic construct
  source 1..19: mol_type = other DNA
atctaaaaccaacttgaga

SEQ ID NO: 68 - DNA, 19 bp, synthetic construct
  source 1..19: mol_type = other DNA
ggtgggcaggaaggactga

SEQ ID NO: 69 - DNA, 19 bp, synthetic construct
  source 1..19: mol_type = other DNA
ggtgggcagaaaggactga

SEQ ID NO: 70 - DNA, 19 bp, synthetic construct
  source 1..19: mol_type = other DNA
cctaaatcaatctacaagt

SEQ ID NO: 71 - DNA, 19 bp, synthetic construct
  source 1..19: mol_type = other DNA
cctaaattaatctacaagt

SEQ ID NO: 72 - DNA, 19 bp, synthetic construct
  source 1..19: mol_type = other DNA
tccctaaatcaatctacaa

SEQ ID NO: 73 - DNA, 19 bp, synthetic construct
  source 1..19: mol_type = other DNA
tccctaaattaatctacaa

SEQ ID NO: 74 - DNA, 19 bp, synthetic construct
  source 1..19: mol_type = other DNA
gaaaatgtgagtggatcta

SEQ ID NO: 75 - DNA, 19 bp, synthetic construct
  source 1..19: mol_type = other DNA
gaaaatgtgcgtggatcta

SEQ ID NO: 76 - DNA, 19 bp, synthetic construct
  source 1..19: mol_type = other DNA
gtaaggcgagactgactag

SEQ ID NO: 77 - DNA, 19 bp, synthetic construct
  source 1..19: mol_type = other DNA
gtaaggcaagactgactag

SEQ ID NO: 78 - DNA, 19 bp, synthetic construct
  source 1..19: mol_type = other DNA
aggtaaggcgagactgact

SEQ ID NO: 79 - DNA, 19 bp, synthetic construct
  source 1..19: mol_type = other DNA
aggtaaggcaagactgact

SEQ ID NO: 80 - DNA, 19 bp, synthetic construct
  source 1..19: mol_type = other DNA
ctgagcggagaaaccctcc

SEQ ID NO: 81 - DNA, 19 bp, synthetic construct
  source 1..19: mol_type = other DNA
ctgagcgaagaaaccctcc

SEQ ID NO: 82 - DNA, 19 bp, synthetic construct
  source 1..19: mol_type = other DNA
ggctgagcggagaaaccct

SEQ ID NO: 83 - DNA, 19 bp, synthetic construct
  source 1..19: mol_type = other DNA
ggctgagcgaagaaaccct

SEQ ID NO: 84 - DNA, 19 bp, synthetic construct
  source 1..19: mol_type = other DNA
aaggctgagcggagaaacc

SEQ ID NO: 85 - DNA, 19 bp, synthetic construct
  source 1..19: mol_type = other DNA
ttccctaaaaacaaaaaca

SEQ ID NO: 86 - DNA, 19 bp, synthetic construct
  source 1..19: mol_type = other DNA
ttccctagaaacaaaaaca

SEQ ID NO: 87 - DNA, 19 bp, synthetic construct
  source 1..19: mol_type = other DNA
gattccctaaaaacaaaaa

SEQ ID NO: 88 - DNA, 19 bp, synthetic construct
  source 1..19: mol_type = other DNA
gattccctagaaacaaaaa

SEQ ID NO: 89 - DNA, 19 bp, synthetic construct
  source 1..19: mol_type = other DNA
cttttctattgtctgtccc

SEQ ID NO: 90 - DNA, 19 bp, synthetic construct
  source 1..19: mol_type = other DNA
cttttctgttgtctgtccc

SEQ ID NO: 91 - DNA, 19 bp, synthetic construct
  source 1..19: mol_type = other DNA
tgcttttctattgtctgtc

SEQ ID NO: 92 - DNA, 19 bp, synthetic construct
  source 1..19: mol_type = other DNA
tgcttttctgttgtctgtc

SEQ ID NO: 93 - DNA, 19 bp, synthetic construct
  source 1..19: mol_type = other DNA
aagggatgccgacttgggc

SEQ ID NO: 94 - DNA, 19 bp, synthetic construct
  source 1..19: mol_type = other DNA
aagggatgctgacttgggc

SEQ ID NO: 95 - DNA, 19 bp, synthetic construct
  source 1..19: mol_type = other DNA
accttcctcactgaggatg

SEQ ID NO: 96 - DNA, 19 bp, synthetic construct
  source 1..19: mol_type = other DNA
accttcctcgctgaggatg

SEQ ID NO: 97 - DNA, 19 bp, synthetic construct
  source 1..19: mol_type = other DNA
caaaccactgtgggatgaa

SEQ ID NO: 98 - DNA, 19 bp, synthetic construct
  source 1..19: mol_type = other DNA
caaaccactttgggatgaa

SEQ ID NO: 99 - DNA, 19 bp, synthetic construct
  source 1..19: mol_type = other DNA
aataaattgtcatcaccag

SEQ ID NO: 100 - DNA, 19 bp, synthetic construct
  source 1..19: mol_type = other DNA
aataaattgccatcaccag

SEQ ID NO: 101 - DNA, 19 bp, synthetic construct
  source 1..19: mol_type = other DNA
tcacagctatcttctcatc

SEQ ID NO: 102 - DNA, 19 bp, synthetic construct
  source 1..19: mol_type = other DNA
tcacagctaacttctcatc

SEQ ID NO: 103 - DNA, 19 bp, synthetic construct
  source 1..19: mol_type = other DNA
gcacacagtagatgaggga

SEQ ID NO: 104 - DNA, 19 bp, synthetic construct
  source 1..19: mol_type = other DNA
gcacacagtggatgaggga

SEQ ID NO: 105 - DNA, 19 bp, synthetic construct
  source 1..19: mol_type = other DNA
cagaacaaagagaagaatt

SEQ ID NO: 106 - DNA, 19 bp, synthetic construct
  source 1..19: mol_type = other DNA
cagaacaaacagaagaatt

SEQ ID NO: 107 - DNA, 19 bp, synthetic construct
  source 1..19: mol_type = other DNA
gcttacatgccttcagtga

SEQ ID NO: 108 - DNA, 19 bp, synthetic construct
  source 1..19: mol_type = other DNA
gcttacacgccttcagtga

SEQ ID NO: 109 - DNA, 19 bp, synthetic construct
  source 1..19: mol_type = other DNA
cagcttacatgccttcagt

SEQ ID NO: 110 - DNA, 19 bp, synthetic construct
  source 1..19: mol_type = other DNA
cagcttacacgccttcagt

SEQ ID NO: 111 - DNA, 19 bp, synthetic construct
  source 1..19: mol_type = other DNA
aagaagcctgataaaatct

SEQ ID NO: 112 - DNA, 19 bp, synthetic construct
  source 1..19: mol_type = other DNA
aagaagcctaataaaatct

SEQ ID NO: 113 - DNA, 19 bp, synthetic construct
  source 1..19: mol_type = other DNA
catacatcagctcaaactg

SEQ ID NO: 114 - DNA, 19 bp, synthetic construct
  source 1..19: mol_type = other DNA
catacattagctcaaactg

SEQ ID NO: 115 - DNA, 19 bp, synthetic construct
  source 1..19: mol_type = other DNA
cacatacatcagctcaaac

SEQ ID NO: 116 - DNA, 19 bp, synthetic construct
  source 1..19: mol_type = other DNA
cacatacattagctcaaac

SEQ ID NO: 117 - DNA, 19 bp, synthetic construct
  source 1..19: mol_type = other DNA
gtcacatacatcagctcaa

SEQ ID NO: 118 - DNA, 19 bp, synthetic construct
  source 1..19: mol_type = other DNA
gagactatagcacccagat

SEQ ID NO: 119 - DNA, 19 bp, synthetic construct
  source 1..19: mol_type = other DNA
gagactataacacccagat

SEQ ID NO: 120 - DNA, 19 bp, synthetic construct
  source 1..19: mol_type = other DNA
tagaggacgccgtgcaggg

SEQ ID NO: 121 - DNA, 19 bp, synthetic construct
  source 1..19: mol_type = other DNA
tagaggatgccgtgcaggg

SEQ ID NO: 122 - DNA, 19 bp, synthetic construct
  source 1..19: mol_type = other DNA
catagaggacgccgtgcag

SEQ ID NO: 123 - DNA, 19 bp, synthetic construct
  source 1..19: mol_type = other DNA
catagaggatgccgtgcag

SEQ ID NO: 124 - DNA, 19 bp, synthetic construct
  source 1..19: mol_type = other DNA
cacatagaggacgccgtgc

SEQ ID NO: 125 - DNA, 19 bp, synthetic construct
  source 1..19: mol_type = other DNA
acgtgtgtacagaacctgc

SEQ ID NO: 126 - DNA, 19 bp, synthetic construct
  source 1..19: mol_type = other DNA
acgtgtgtatagaacctgc

SEQ ID NO: 127 - DNA, 19 bp, synthetic construct
  source 1..19: mol_type = other DNA
tgttcagaatgcctcatct

SEQ ID NO: 128 - DNA, 19 bp, synthetic construct
  source 1..19: mol_type = other DNA
tgttcagaacgcctcatct

SEQ ID NO: 129 - DNA, 19 bp, synthetic construct
  source 1..19: mol_type = other DNA
aaacggcgcagcgggaagg

SEQ ID NO: 130 - DNA, 19 bp, synthetic construct
  source 1..19: mol_type = other DNA
aaacggcacagcgggaagg

SEQ ID NO: 131 - DNA, 19 bp, synthetic construct
  source 1..19: mol_type = other DNA
agaaacggcgcagcgggaa

SEQ ID NO: 132 - DNA, 19 bp, synthetic construct
  source 1..19: mol_type = other DNA
agaaacggcacagcgggaa

SEQ ID NO: 133 - DNA, 19 bp, synthetic construct
  source 1..19: mol_type = other DNA
agggcgcagacttccaaag

SEQ ID NO: 134 - DNA, 19 bp, synthetic construct
  source 1..19: mol_type = other DNA
agggcacagacttccaaag

SEQ ID NO: 135 - DNA, 19 bp, synthetic construct
  source 1..19: mol_type = other DNA
aagggcgcagacttccaaa

SEQ ID NO: 136 - DNA, 19 bp, synthetic construct
  source 1..19: mol_type = other DNA
aagggcacagacttccaaa

SEQ ID NO: 137 - DNA, 19 bp, synthetic construct
  source 1..19: mol_type = other DNA
caagggcgcagacttccaa

SEQ ID NO: 138 - DNA, 19 bp, synthetic construct
  source 1..19: mol_type = other DNA
caagggcacagacttccaa

SEQ ID NO: 139 - DNA, 19 bp, synthetic construct
  source 1..19: mol_type = other DNA
acaagggcgcagacttcca

SEQ ID NO: 140 - DNA, 19 bp, synthetic construct
  source 1..19: mol_type = other DNA
acaagggcacagacttcca

SEQ ID NO: 141 - DNA, 19 bp, synthetic construct
  source 1..19: mol_type = other DNA
cacaagggcgcagacttcc

SEQ ID NO: 142 - DNA, 19 bp, synthetic construct
  source 1..19: mol_type = other DNA
cacaagggcacagacttcc

SEQ ID NO: 143 - DNA, 19 bp, synthetic construct
  source 1..19: mol_type = other DNA
gcacaagggcgcagacttc

SEQ ID NO: 144 - DNA, 19 bp, synthetic construct
  source 1..19: mol_type = other DNA
gcacaagggcacagacttc

SEQ ID NO: 145 - DNA, 19 bp, synthetic construct
  source 1..19: mol_type = other DNA
ggcacaagggcgcagactt

SEQ ID NO: 146 - DNA, 19 bp, synthetic construct
  source 1..19: mol_type = other DNA
ggcacaagggcacagactt

SEQ ID NO: 147 - DNA, 19 bp, synthetic construct
  source 1..19: mol_type = other DNA
agggcacaagggcgcagac

SEQ ID NO: 148 - DNA, 19 bp, synthetic construct
  source 1..19: mol_type = other DNA
agggcacaagggcacagac

SEQ ID NO: 149 - DNA, 19 bp, synthetic construct
  source 1..19: mol_type = other DNA
gagcagctgcaacctggca

SEQ ID NO: 150 - DNA, 19 bp, synthetic construct
  source 1..19: mol_type = other DNA
gagcagctgtaacctggca

SEQ ID NO: 151 - DNA, 19 bp, synthetic construct
  source 1..19: mol_type = other DNA
tggtgccgggtgtctagca

SEQ ID NO: 152 - DNA, 19 bp, synthetic construct
  source 1..19: mol_type = other DNA
tggtgccaggtgtctagca

SEQ ID NO: 153 - DNA, 19 bp, synthetic construct
  source 1..19: mol_type = other DNA
aatggtgccgggtgtctag

SEQ ID NO: 154 - DNA, 19 bp, synthetic construct
  source 1..19: mol_type = other DNA
aatggtgccaggtgtctag

SEQ ID NO: 155 - DNA, 19 bp, synthetic construct
  source 1..19: mol_type = other DNA
ggggacagggtgtgctctc

SEQ ID NO: 156 - DNA, 19 bp, synthetic construct
  source 1..19: mol_type = other DNA
ggggacaggttgtgctctc

SEQ ID NO: 157 - DNA, 19 bp, synthetic construct
  source 1..19: mol_type = other DNA
gcttttcattgaaaagaaa

SEQ ID NO: 158 - DNA, 19 bp, synthetic construct
  source 1..19: mol_type = other DNA
gcttttcgttgaaaagaaa

SEQ ID NO: 159 - DNA, 19 bp, synthetic construct
  source 1..19: mol_type = other DNA
ctgcttttcattgaaaaga

SEQ ID NO: 160 - DNA, 19 bp, synthetic construct
  source 1..19: mol_type = other DNA
ctgcttttcgttgaaaaga

SEQ ID NO: 161 - DNA, 19 bp, synthetic construct
  source 1..19: mol_type = other DNA
actaggccgggcatgctgg

SEQ ID NO: 162 - DNA, 19 bp, synthetic construct
  source 1..19: mol_type = other DNA
actaggctgggcatgctgg

SEQ ID NO: 163 - DNA, 19 bp, synthetic construct
  source 1..19: mol_type = other DNA
agactaggccgggcatgct

SEQ ID NO: 164 - DNA, 19 bp, synthetic construct
  source 1..19: mol_type = other DNA
agactaggctgggcatgct

SEQ ID NO: 165 - DNA, 19 bp, synthetic construct
  source 1..19: mol_type = other DNA
aaacagctgttagttccca

SEQ ID NO: 166 - DNA, 19 bp, synthetic construct
  source 1..19: mol_type = other DNA
aaacagccgttagttccca

SEQ ID NO: 167 - DNA, 19 bp, synthetic construct
  source 1..19: mol_type = other DNA
agaaacagctgttagttcc

SEQ ID NO: 168 - DNA, 19 bp, synthetic construct
  source 1..19: mol_type = other DNA
agaaacagccgttagttcc

SEQ ID NO: 169 - DNA, 19 bp, synthetic construct
  source 1..19: mol_type = other DNA
gtgctacccaacctttctg

SEQ ID NO: 170 - DNA, 19 bp, synthetic construct
  source 1..19: mol_type = other DNA
agtgctacccaacctttct

SEQ ID NO: 171 - DNA, 19 bp, synthetic construct
  source 1..19: mol_type = other DNA
cagtgctacccaacctttc

SEQ ID NO: 172 - DNA, 19 bp, synthetic construct
  source 1..19: mol_type = other DNA
acagtgctacccaaccttt

SEQ ID NO: 173 - DNA, 18 bp, synthetic construct
  source 1..18: mol_type = other DNA
acagtgctacccaacctt

SEQ ID NO: 174 - DNA, 17 bp, synthetic construct
  source 1..17: mol_type = other DNA
acagtgctacccaacct

SEQ ID NO: 175 - DNA, 16 bp, synthetic construct
  source 1..16: mol_type = other DNA
cagtgctacccaacct

SEQ ID NO: 176 - DNA, 19 bp, synthetic construct
  source 1..19: mol_type = other DNA
tcacagtgctacccaacct

SEQ ID NO: 177 - DNA, 15 bp, synthetic construct
  source 1..15: mol_type = other DNA
cagtgctacccaacc

SEQ ID NO: 178 - DNA, 19 bp, synthetic construct
  source 1..19: mol_type = other DNA
atcacagtgctacccaacc

SEQ ID NO: 179 - DNA, 19 bp, synthetic construct
  source 1..19: mol_type = other DNA
tatcacagtgctacccaac

SEQ ID NO: 180 - DNA, 19 bp, synthetic construct
  source 1..19: mol_type = other DNA
atatcacagtgctacccaa

SEQ ID NO: 181 - DNA, 19 bp, synthetic construct
  source 1..19: mol_type = other DNA
atgctgacttgggccattc

SEQ ID NO: 182 - DNA, 19 bp, synthetic construct
  source 1..19: mol_type = other DNA
gatgctgacttgggccatt

SEQ ID NO: 183 - DNA, 19 bp, synthetic construct
  source 1..19: mol_type = other DNA
ggatgctgacttgggccat

SEQ ID NO: 184 - DNA, 19 bp, synthetic construct
  source 1..19: mol_type = other DNA
gggatgctgacttgggcca

SEQ ID NO: 185 - DNA, 19 bp, synthetic construct
  source 1..19: mol_type = other DNA
agggatgctgacttgggcc

SEQ ID NO: 186 - DNA, 18 bp, synthetic construct
  source 1..18: mol_type = other DNA
agggatgctgacttgggc

SEQ ID NO: 187 - DNA, 17 bp, synthetic construct
  source 1..17: mol_type = other DNA
agggatgctgacttggg

SEQ ID NO: 188 - DNA, 19 bp, synthetic construct
  source 1..19: mol_type = other DNA
caagggatgctgacttggg

SEQ ID NO: 189 - DNA, 15 bp, synthetic construct
  source 1..15: mol_type = other DNA
gggatgctgacttgg

SEQ ID NO: 190 - DNA, 19 bp, synthetic construct
  source 1..19: mol_type = other DNA
ccaagggatgctgacttgg

SEQ ID NO: 191 - DNA, 19 bp, synthetic construct
  source 1..19: mol_type = other DNA
gccaagggatgctgacttg

SEQ ID NO: 192 - DNA, 19 bp, synthetic construct
  source 1..19: mol_type = other DNA
tgccaagggatgctgactt

SEQ ID NO: 193 - DNA, 19 bp, synthetic construct
  source 1..19: mol_type = other DNA
ctgccaagggatgctgact

SEQ ID NO: 194 - DNA, 19 bp, synthetic construct
  source 1..19: mol_type = other DNA
attgtcatcaccagaaaaa

SEQ ID NO: 195 - DNA, 19 bp, synthetic construct
  source 1..19: mol_type = other DNA
aattgtcatcaccagaaaa

SEQ ID NO: 196 - DNA, 19 bp, synthetic construct
  source 1..19: mol_type = other DNA
aaattgtcatcaccagaaa

SEQ ID NO: 197 - DNA, 19 bp, synthetic construct
  source 1..19: mol_type = other DNA
taaattgtcatcaccagaa

SEQ ID NO: 198 - DNA, 19 bp, synthetic construct
  source 1..19: mol_type = other DNA
ataaattgtcatcaccaga

SEQ ID NO: 199 - DNA, 18 bp, synthetic construct
  source 1..18: mol_type = other DNA
ataaattgtcatcaccag

SEQ ID NO: 200 - DNA, 17 bp, synthetic construct
  source 1..17: mol_type = other DNA
ataaattgtcatcacca

SEQ ID NO: 201 - DNA, 16 bp, synthetic construct
  source 1..16: mol_type = other DNA
taaattgtcatcacca

SEQ ID NO: 202 - DNA, 19 bp, synthetic construct
  source 1..19: mol_type = other DNA
taataaattgtcatcacca

SEQ ID NO: 203 - DNA, 15 bp, synthetic construct
  source 1..15: mol_type = other DNA
taaattgtcatcacc

SEQ ID NO: 204 - DNA, 19 bp, synthetic construct
  source 1..19: mol_type = other DNA
ttaataaattgtcatcacc

SEQ ID NO: 205 - DNA, 19 bp, synthetic construct
  source 1..19: mol_type = other DNA
attaataaattgtcatcac

SEQ ID NO: 206 - DNA, 19 bp, synthetic construct
  source 1..19: mol_type = other DNA
tattaataaattgtcatca

SEQ ID NO: 207 - DNA, 19 bp, synthetic construct
  source 1..19: mol_type = other DNA
ctattaataaattgtcatc

SEQ ID NO: 208 - DNA, 19 bp, synthetic construct
  source 1..19: mol_type = other DNA
cagtagatgagggagcagg

SEQ ID NO: 209 - DNA, 19 bp, synthetic construct
  source 1..19: mol_type = other DNA
acagtagatgagggagcag

SEQ ID NO: 210 - DNA, 19 bp, synthetic construct
  source 1..19: mol_type = other DNA
cacagtagatgagggagca

SEQ ID NO: 211 - DNA, 19 bp, synthetic construct
  source 1..19: mol_type = other DNA
acacagtagatgagggagc

SEQ ID NO: 212 - DNA, 19 bp, synthetic construct
  source 1..19: mol_type = other DNA
cacacagtagatgagggag

SEQ ID NO: 213 - DNA, 18 bp, synthetic construct
  source 1..18: mol_type = other DNA
cacacagtagatgaggga

SEQ ID NO: 214 - DNA, 17 bp, synthetic construct
  source 1..17: mol_type = other DNA
cacacagtagatgaggg

SEQ ID NO: 215 - DNA, 16 bp, synthetic construct
  source 1..16: mol_type = other DNA
acacagtagatgaggg

SEQ ID NO: 216 - DNA, 19 bp, synthetic construct
  source 1..19: mol_type = other DNA
tgcacacagtagatgaggg

SEQ ID NO: 217 - DNA, 15 bp, synthetic construct
  source 1..15: mol_type = other DNA
acacagtagatgagg

SEQ ID NO: 218 - DNA, 19 bp, synthetic construct
  source 1..19: mol_type = other DNA
gtgcacacagtagatgagg

SEQ ID NO: 219 - DNA, 19 bp, synthetic construct
  source 1..19: mol_type = other DNA
agtgcacacagtagatgag

SEQ ID NO: 220 - DNA, 19 bp, synthetic construct
  source 1..19: mol_type = other DNA
aagtgcacacagtagatga

SEQ ID NO: 221 - DNA, 19 bp, synthetic construct
  source 1..19: mol_type = other DNA
gaagtgcacacagtagatg

SEQ ID NO: 222 - DNA, 19 bp, synthetic construct
  source 1..19: mol_type = other DNA
gctgcaacctggcaacaac

SEQ ID NO: 223 - DNA, 19 bp, synthetic construct
  source 1..19: mol_type = other DNA
agctgcaacctggcaacaa

SEQ ID NO: 224 - DNA, 19 bp, synthetic construct
  source 1..19: mol_type = other DNA
cagctgcaacctggcaaca

SEQ ID NO: 225 - DNA, 19 bp, synthetic construct
  source 1..19: mol_type = other DNA
gcagctgcaacctggcaac

SEQ ID NO: 226 - DNA, 19 bp, synthetic construct
  source 1..19: mol_type = other DNA
agcagctgcaacctggcaa

SEQ ID NO: 227 - DNA, 18 bp, synthetic construct
  source 1..18: mol_type = other DNA
agcagctgcaacctggca

SEQ ID NO: 228 - DNA, 17 bp, synthetic construct
  source 1..17: mol_type = other DNA
agcagctgcaacctggc

SEQ ID NO: 229 - DNA, 16 bp, synthetic construct
  source 1..16: mol_type = other DNA
gcagctgcaacctggc

SEQ ID NO: 230 - DNA, 19 bp, synthetic construct
  source 1..19: mol_type = other DNA
agagcagctgcaacctggc

SEQ ID NO: 231 - DNA, 15 bp, synthetic construct
  source 1..15: mol_type = other DNA
gcagctgcaacctgg

SEQ ID NO: 232 - DNA, 19 bp, synthetic construct
  source 1..19: mol_type = other DNA
aagagcagctgcaacctgg

SEQ ID NO: 233 - DNA, 19 bp, synthetic construct
  source 1..19: mol_type = other DNA
caagagcagctgcaacctg

SEQ ID NO: 234 - DNA, 19 bp, synthetic construct
  source 1..19: mol_type = other DNA
gcaagagcagctgcaacct

SEQ ID NO: 235 - DNA, 19 bp, synthetic construct
  source 1..19: mol_type = other DNA
tgcaagagcagctgcaacc

SEQ ID NO: 236 - DNA, 19 bp, synthetic construct
  source 1..19: mol_type = other DNA
accatgatatctccagcac

SEQ ID NO: 237 - DNA, 19 bp, synthetic construct
  source 1..19: mol_type = other DNA
accatgacatctccagcac

SEQ ID NO: 238 - DNA, 19 bp, synthetic construct
  source 1..19: mol_type = other DNA
ccaccatgatatctccagc

SEQ ID NO: 239 - DNA, 19 bp, synthetic construct
  source 1..19: mol_type = other DNA
ccaccatgacatctccagc

SEQ ID NO: 240 - DNA, 19 bp, synthetic construct
  source 1..19: mol_type = other DNA
ttaacactcgattaaccct

SEQ ID NO: 241 - DNA, 19 bp, synthetic construct
  source 1..19: mol_type = other DNA
tagttcatcccagtgagaa

SEQ ID NO: 242 - DNA, 19 bp, synthetic construct
  source 1..19: mol_type = other DNA
ctagttcatcccagtgaga

SEQ ID NO: 243 - DNA, 19 bp, synthetic construct
  source 1..19: mol_type = other DNA
gaaatgggtttttccacat

SEQ ID NO: 244 - DNA, 19 bp, synthetic construct
  source 1..19: mol_type = other DNA
ggaaatgggtttttccaca

SEQ ID NO: 245 - DNA, 19 bp, synthetic construct
  source 1..19: mol_type = other DNA
taaccgtggcatgggcagt

SEQ ID NO: 246 - DNA, 19 bp, synthetic construct
  source 1..19: mol_type = other DNA
ttaaccgtggcatgggcag

SEQ ID NO: 247 - DNA, 19 bp, synthetic construct
  source 1..19: mol_type = other DNA
cttcaagctagtaacgatg

SEQ ID NO: 248 - DNA, 19 bp, synthetic construct
  source 1..19: mol_type = other DNA
agctaggttaaagagtcac

SEQ ID NO: 249 - DNA, 19 bp, synthetic construct
  source 1..19: mol_type = other DNA
cagctaggttaaagagtca

SEQ ID NO: 250 - DNA, 19 bp, synthetic construct
  source 1..19: mol_type = other DNA
taagaaacacaatcaaaga

SEQ ID NO: 251 - DNA, 19 bp, synthetic construct
  source 1..19: mol_type = other DNA
ataagaaacacaatcaaag

SEQ ID NO: 252 - DNA, 19 bp, synthetic construct
  source 1..19: mol_type = other DNA
attttctagactttatgat

SEQ ID NO: 253 - DNA, 19 bp, synthetic construct
  source 1..19: mol_type = other DNA
aattttctagactttatga

SEQ ID NO: 254 - DNA, 19 bp, synthetic construct
  source 1..19: mol_type = other DNA
gagaatacgggtaacattt

SEQ ID NO: 255 - DNA, 19 bp, synthetic construct
  source 1..19: mol_type = other DNA
tgggcaggaaggactgaac

SEQ ID NO: 256 - DNA, 19 bp, synthetic construct
  source 1..19: mol_type = other DNA
gtgggcaggaaggactgaa

SEQ ID NO: 257 - DNA, 19 bp, synthetic construct
  source 1..19: mol_type = other DNA
ccctaaatcaatctacaag

SEQ ID NO: 258 - DNA, 19 bp, synthetic construct
  source 1..19: mol_type = other DNA
cttttccgtgctgttctga

SEQ ID NO: 259 - DNA, 19 bp, synthetic construct
  source 1..19: mol_type = other DNA
acttttccgtgctgttctg

SEQ ID NO: 260 - DNA, 19 bp, synthetic construct
  source 1..19: mol_type = other DNA
aacttttccgtgctgttct

SEQ ID NO: 261 - DNA, 19 bp, synthetic construct
  source 1..19: mol_type = other DNA
gctgagcggagaaaccctc

SEQ ID NO: 262 - DNA, 19 bp, synthetic construct
  source 1..19: mol_type = other DNA
attccctaaaaacaaaaac

SEQ ID NO: 263 - DNA, 19 bp, synthetic construct
  source 1..19: mol_type = other DNA
gcttttctattgtctgtcc

SEQ ID NO: 264 - DNA, 19 bp, synthetic construct
  source 1..19: mol_type = other DNA
cttcctcactgaggatgaa

SEQ ID NO: 265 - DNA, 19 bp, synthetic construct
  source 1..19: mol_type = other DNA
ccttcctcactgaggatga

SEQ ID NO: 266 - DNA, 19 bp, synthetic construct
  source 1..19: mol_type = other DNA
aaccactttgggatgaata

SEQ ID NO: 267 - DNA, 19 bp, synthetic construct
  source 1..19: mol_type = other DNA
aaaccactttgggatgaat

SEQ ID NO: 268 - DNA, 19 bp, synthetic construct
  source 1..19: mol_type = other DNA
acagctatcttctcatcaa

SEQ ID NO: 269 - DNA, 19 bp, synthetic construct
  source 1..19: mol_type = other DNA
cacagctatcttctcatca

SEQ ID NO: 270 - DNA, 19 bp, synthetic construct
  source 1..19: mol_type = other DNA
gaacaaagagaagaatttc

SEQ ID NO: 271 - DNA, 19 bp, synthetic construct
  source 1..19: mol_type = other DNA
agaacaaagagaagaattt

SEQ ID NO: 272 - DNA, 19 bp, synthetic construct
  source 1..19: mol_type = other DNA
gaagcctgataaaatctct

SEQ ID NO: 273 - DNA, 19 bp, synthetic construct
  source 1..19: mol_type = other DNA
agaagcctgataaaatctc

SEQ ID NO: 274 - DNA, 19 bp, synthetic construct
  source 1..19: mol_type = other DNA
tgatctgtagcagcagctt

SEQ ID NO: 275 - DNA, 19 bp, synthetic construct
  source 1..19: mol_type = other DNA
ttgatctgtagcagcagct

SEQ ID NO: 276 - DNA, 19 bp, synthetic construct
  source 1..19: mol_type = other DNA
gttgatctgtagcagcagc

SEQ ID NO: 277 - DNA, 19 bp, synthetic construct
  source 1..19: mol_type = other DNA
atagaggacgccgtgcagg

SEQ ID NO: 278 - DNA, 19 bp, synthetic construct
  source 1..19: mol_type = other DNA
gtgtgtacagaacctgccg

SEQ ID NO: 279 - DNA, 19 bp, synthetic construct
  source 1..19: mol_type = other DNA
cgtgtgtacagaacctgcc

SEQ ID NO: 280 - DNA, 19 bp, synthetic construct
  source 1..19: mol_type = other DNA
ttcagaatgcctcatctgg

SEQ ID NO: 281 - DNA, 19 bp, synthetic construct
  source 1..19: mol_type = other DNA
gttcagaatgcctcatctg

SEQ ID NO: 282 - DNA, 19 bp, synthetic construct
  source 1..19: mol_type = other DNA
ggacagggtgtgctctccg

SEQ ID NO: 283 - DNA, 19 bp, synthetic construct
  source 1..19: mol_type = other DNA
gggacagggtgtgctctcc

SEQ ID NO: 284 - DNA, 16 bp, synthetic construct
  source 1..16: mol_type = other DNA
gggatgctgacttggg

SEQ ID NO: 285 - DNA, 17 bp, synthetic construct
  source 1..17: mol_type = other DNA
acacagtagatgaggga

SEQ ID NO: 286 - RNA, 10081 nt, Mus musculus
  source 1..10081: mol_type = mRNA
gcactcgccgcgagggttgccgggacgggcccaagatggctgagcgccttggttccgcttctgcctgccgcgcagagccccattcattgccttgctgctaagtggcgccgcgtagtgccagtaggctccaagtcttcagggtctgtcccatcgggcaggaagccgtcatggcaaccctggaaaagctgatgaaggctttcgagtcgctcaagtcgtttcagcagcaacagcagcagcagccaccgccgcaggcgccgccgccaccgccgccgccgcctccgcctcaaccccctcagccgccgcctcaggggcagccgccgccgccaccaccgccgctgccaggtccggcagaggaaccgctgcaccgaccaaagaaggaactctcagccaccaagaaagaccgtgtgaatcattgtctaacaatatgtgaaaacattgtggcacagtctctcagaaattctccagaatttcagaaactcttgggcatcgctatggaactgtttctgctgtgcagtgacgatgcggagtcagatgtcagaatggtggctgatgagtgcctcaacaaagtcatcaaagctttgatggattctaatcttccaaggctacagttagaactctataaggaaattaaaaagaatggtgctcctcgaagtttgcgtgctgccctgtggaggtttgctgagctggctcacctggttcgacctcagaagtgcaggccttacctggtgaatcttcttccatgcctgacccgaacaagcaaaagaccggaggaatcagttcaggagaccttggctgcagctgttcctaaaattatggcttcttttggcaatttcgcaaatgacaatgaaattaaggttctgttgaaagctttcatagcaaatctgaagtcaagctctcccaccgtgcggcggacagcagccggctcagccgtgagcatctgccaacattctaggaggacacagtacttctacaactggctccttaatgtcctcctaggtctgctggttcccatggaagaagagcactccactctcctgatcctcggtgtgttgctcacattgaggtgtctagtgcccttgctccagcagcaggtcaaggacacaagtctaaaaggcagctttggggtgacacggaaagaaatggaagtctctccttctacagagcagcttgtccaggtttatgaactgactttgcatcatactcagcaccaagaccacaatgtggtgacaggggcactggagctcctgcagcagctcttccgtacccctccacctgaactcctgcaagcactgaccacaccaggagggcttgggcagctcactctggttcaagaagaggcccggggccgaggccgcagcgggagcatcgtggagcttttagctggagggggttcctcgtgcagccctgtcctctcaagaaagcagaaaggcaaagtgctcttaggagaggaagaagccttggaagatgactcggagtccaggtcagatgtcagcagctcagcctttgcagcctctgtgaagagtgagattggtggagagctcgctgcttcttcaggtgtttccactcctggttctgttggtcacgacatcatcactgagcagcctagatcccagcacacacttcaagcagactctgtggatttgtccggctgtgacctgaccagtgctgctactgatggggatgaggaggacatcttgagccacagctccagccagttcagtgctgtcccatccgaccctgccatggacctgaatgatgggacccaggcctcctcacccatcagtgacagttctcagaccaccactgaaggacctgattcagctgtgactccttcggacagttctgaaattgtgttagatggtgccgatagccagtatttaggcatgcagataggacagccacaggaggacgatgaggagggagctgcaggtgttctttctggtgaagtctcagatgttttcagaaactcttctctggcccttcaacaggcacacttgttggaaagaatgggccatagcaggcagccttccgacagcagtatagataagtatgtaacaagagatgaggttgctgaagccagtgatccagaaagcaagccttgccgaatcaaaggtgacataggacagcctaatgatgatgattctgctcctctggtacattgtgtccgtcttttatctgcttcctttttgttaactggtgaaaagaaagcactggttccagacagagacgtgagagtcagtgtgaaggccctggccctcagctgcattggtgcggctgtggcccttcatccagagtcgttcttcagcagactgtacaaagtacctcttaataccacggaaagtactgaggaacagtatgtttctgacatcttgaactacatcgatcatggagacccacaggtccgaggagctactgccattctctgtgggacccttgtctactccatcctcagtaggtcccgtctccgtgttggtgactggctgggcaacatcagaaccctgacaggaaatacattttctctggtggactgcattcctttactgcagaaaacgttgaaggatgaatcttctgttacttgcaagttggcttgtacagctgtgaggcactgtgtcctgagtctttgcagcagcagctacagtgacttgggattacaactgcttattgatatgctgcctctgaagaacagctcctactggctggtgaggaccgaactgctggacactctggcagagattgacttcaggctcgtgagttttttggaggcaaaagcagaaagtttacaccgaggggctcatcattatacagggtttctaaaactacaagaacgagtactcaataatgtggtcatttatttgcttggagatgaagaccccagggttcgacatgttgctgcaacatcattaacaaggcttgtcccaaagctgttttacaagtgtgaccaaggacaagctgatccagttgtggctgtagcgagggatcagagcagtgtctacctgaagctcctcatgcatgagacccagccaccatcacacttttctgtcagcaccatcaccagaatctatagaggctatagcttactgccaagtataacagatgtcaccatggaaaacaatctctcaagagttgttgccgcagtttctcatgaactcattacgtcaacaacacgggcactcacatttggatgctgtgaagccttgtgtcttctctcagcagcctttccagtttgcacttggagtttaggatggcactgtggagtgcccccactgagtgcctctgatgagtccaggaagagctgcactgttgggatggcctccatgattctcaccttgctttcatcagcttggttcccactggatctctcagcccatcaggatgccttgattttggctggaaacttgctagcagcgagtgcccccaagtctctgagaagttcatggacctctgaagaagaagccaactcagcagccaccagacaggaggaaatctggcctgctctgggggatcggactctagtgcccttggtggagcagcttttctcccacctgctgaaggtgatcaatatctgtgctcatgtcttggacgatgtgactcctggaccagcaatcaaggcagccttgccttctctaacaaaccccccttctctaagtcctattcgacggaaagggaaggagaaagaacctggagaacaagcttctactccaatgagtcccaagaaagttggtgaggccagtgcagcctctcgacaatcagacacctcaggacctgtcacagcaagtaaatcatcctcactggggagtttctaccatctcccctcctacctcaaactgcatgatgtcctgaaagccactcacgccaactataaggtcaccttagatcttcagaacagcactgaaaagtttggggggttcctgcgctctgccttggacgtcctttctcagattctagagctggcgacactgcaggacattggaaagtgtgttgaagaggtccttggatacctgaaatcctgctttagtcgagaaccaatgatggcaactgtctgtgtgcagcagctattgaagactctctttgggacaaacttagcctcacagtttgatggcttatcttccaaccccagcaagtctcagtgccgagctcagcgccttggctcttcaagtgtgaggcccggcttatatcactactgcttcatggcaccatacacgcacttcacacaggccttggctgacgcaagcctgaggaacatggtgcaggcggagcaggagcgtgatgcctcggggtggtttgatgtactccagaaagtgtctgcccaattgaagacgaacctaacaagcgtcacaaagaaccgtgcagataagaatgctattcataatcacattaggttatttgagcctcttgttataaaagcattgaagcagtacaccacgacaacatctgtacaattgcagaagcaggttttggatttgctggcacagctggttcagctacgggtcaattactgtctactggattcagaccaggtgttcatcgggtttgtgctgaagcagtttgagtacattgaagtgggccagttcagggaatcagaggcaattattccaaatatatttttcttcctggtattactgtcttatgagcgctaccattcaaaacagatcattggaattcctaaaatcatccagctgtgtgatggcatcatggccagtggaaggaaggccgttacacatgctatacctgctctgcagcccattgtccatgacctctttgtgttacgaggaacaaataaagctgatgcagggaaagagcttgagacacagaaggaggtggtggtctccatgctgttacgactcatccagtaccatcaggtgctggagatgttcatccttgtcctgcagcagtgccacaaggagaatgaggacaagtggaaacggctctctcggcaggtcgcagacatcatcctgcccatgttggccaagcagcagatgcatattgactctcatgaagcccttggagtgttaaataccttgtttgagattttggctccttcctccctacgtcctgtggacatgcttttgcggagtatgttcatcactccaagcacaatggcatctgtaagcactgtgcagctgtggatatctggaatcctcgccattctgagggttctcatttcccagtcaaccgaggacattgttctttgtcgtattcaggagctctccttctctccacacttgctctcctgtccagtgattaacaggttaaggggtggaggcggtaatgtaacactaggagaatgcagcgaagggaaacaaaagagtttgccagaagatacattctcaaggtttcttttacagctggttggtattcttctagaagacatcgttacaaaacagctcaaagtggacatgagtgaacagcagcatacgttctactgccaagagctaggcacactgctcatgtgtctgatccacatattcaaatctggaatgttccggagaatcacagcagctgccactagactcttcaccagtgatggctgtgaaggcagcttctatactctagagagcctgaatgcacgggtccgatccatggtgcccacgcacccagccctggtactgctctggtgtcagatcctacttctcatcaaccacactgaccaccggtggtgggcagaggtgcagcagacacccaagagacacagtctgtcctgcacgaagtcacttaacccccagaagtctggcgaagaggaggattctggctcggcagctcagctgggaatgtgcaatagagaaatagtgcgaagaggggcccttattctcttctgtgattatgtctgtcagaatctccatgactcagaacacttaacatggctcattgtgaatcacattcaagatctgatcagcttgtctcatgagcctccagtacaagactttattagtgccattcatcgtaattctgcagctagtggtctttttatccaggcaattcagtctcgctgtgaaaatctttcaacgccaaccactctgaagaaaacacttcagtgcttggaaggcatccatctcagccagtctggtgctgtgctcacactatatgtggacaggctcctgggcacccccttccgtgcgctggctcgcatggtcgacaccctggcctgtcgccgggtagaaatgcttttggctgcaaatttacagagcagcatggcccagttgccagaggaggaactaaacagaatccaagaacacctccagaacagtgggcttgcacaaagacaccaaaggctctattcactgctggacagattccgactctctactgtgcaggactcacttagccccttgcccccagtcacttcccacccactggatggggatgggcacacatctctggaaacagtgagtccagacaaagactggtacctccagcttgtcagatcccagtgttggaccagatcagattctgcactgctggaaggtgcagagctggtcaaccgtatccctgctgaagatatgaatgacttcatgatgagctcggagttcaacctaagccttttggctccctgtttaagccttggcatgagcgagattgctaatggccaaaagagtcccctctttgaagcagcccgtggggtgattctgaaccgggtgaccagtgttgttcagcagcttcctgctgtccatcaagtcttccagcccttcctgcctatagagcccacggcctactggaacaagttgaatgatctgcttggtgataccacatcataccagtctctgaccatacttgcccgtgccctggcacagtacctggtggtgctctccaaagtgcctgctcatttgcaccttcctcctgagaaggagggggacacggtgaagtttgtggtaatgacagttgaggccctgtcatggcatttgatccatgagcagatcccactgagtctggacctccaagccgggctagactgctgctgcctggcactacaggtgcctggcctctggggggtgctgtcctccccagagtacgtgactcatgcctgctccctcatccattgtgtgcgattcatcctggaagccattgcagtacaacctggagaccagcttctcggtcctgaaagcaggtcacatactccaagagctgtcagaaaggaggaagtagactcagatatacaaaacctcagtcatgtcacttcggcctgcgagatggtggcagacatggtggaatccctgcagtcagtgctggccttgggccacaagaggaacagcaccctgccttcatttctcacagctgtgctgaagaacattgttatcagtctggcccgactccccctagttaacagctatactcgtgtgcctcctctggtatggaaactcgggtggtcacccaagcctggaggggattttggcacagtgtttcctgagatccctgtagagttcctccaggagaaggagatcctcaaggagttcatctaccgcatcaacaccctagggtggaccaatcgtacccagttcgaagaaacttgggccaccctccttggtgtcctggtgactcagcccctggtgatggaacaggaagagagcccaccagaggaagacacagaaagaacccagatccatgtcctggctgtgcaggccatcacctctctagtgctcagtgcaatgaccgtgcctgtggctggcaatccagctgtaagctgcttggagcaacagccccggaacaagccactgaaggctctcgataccagatttggaagaaagctgagcatgatcagagggattgtagaacaagaaatccaagagatggtttcccagagagagaatactgccactcaccattctcaccaggcgtgggatcctgtcccttctctgttaccagctactacaggtgctcttatcagccatgacaagctgctgctgcagatcaacccagagcgggagccaggcaacatgagctacaagctgggccaggtgtccatacactccgtgtggctgggaaataacatcacacccctgagagaggaggaatgggatgaggaagaagaggaagaaagtgatgtccctgcaccaacgtcaccacctgtgtctccagtcaattccagaaaacaccgtgccggggttgatattcactcctgttcgcagtttctgcttgaattgtacagccgatggatcctgccatccagtgcagccagaaggacccccgtcatcctgatcagtgaagtggttcgatctcttcttgtagtgtcagacttattcaccgaacgtacccagtttgaaatgatgtatctgacgctgacagaactacggagagtgcacccttcagaagatgagatcctcattcagtacctggtgcctgccacctgtaaggcagctgctgtccttggaatggacaaaactgtggcagagccagtcagccgcctactggagagcacactgaggagcagccacctgcccagccagatcggagccctgcacggcatcctctatgtgttggagtgtgacctcttggatgacactgcaaagcagctcattccagttgttagtgactatctgctgtccaacctcaaaggaatagcccactgcgtgaacattcacagccagcagcatgtgctggtaatgtgtgccactgctttctacctgatggaaaactaccctctggatgtgggaccagaattttcagcatctgtgatacagatgtgtggagtaatgctgtctggaagtgaggagtccaccccctccatcatttaccactgtgccctccggggtctggagcggctcctgctgtctgagcagctatctcggctagacacagagtccttggtcaagctaagtgtggacagagtgaatgtacaaagcccacacagggccatggcagccctaggcctgatgctcacctgcatgtacacaggaaaggaaaaagccagtccaggcagagcttctgaccccagccctgctacacctgacagcgagtctgtgattgtagctatggagcgagtgtctgttctctttgataggatccgcaagggatttccctgtgaagccagggttgtggcaaggatcctgcctcagttcctagatgacttctttccacctcaagatgtcatgaacaaagtcattggagagttcctgtccaatcagcagccatacccacagttcatggccactgtagtttacaaggtttttcagactctgcacagtgctgggcagtcatccatggtccgggactgggtcatgctgtccctgtccaacttcacacaaagaactccagttgccatggccatgtggagcctctcctgcttccttgttagcgcatctaccagcccatgggtttctgcgatccttccacatgtcatcagcaggatgggcaaactggaacaggtggatgtgaaccttttctgcctggttgccacagacttctacagacaccagatagaggaggaattcgaccgcagggctttccagtctgtgtttgaggtggtggctgcaccaggaagtccataccacaggctgcttgcttgtttgcaaaatgttcacaaggtcaccacctgctgagtagtgcctgtgggacaaaaggctgaaagaaggcagctgctggggcctgagcctccaggagcctgctccaagcttctgctggggctgccttggccgtgcaggcttccacttgtgtcaagtggacagccaggcaatggcaggagtgctttgcaatgagggctatgcagggaacatgcactatgttggggttgagcctgagtcctgggtcctggcctcgctgcagctggtgacagtgctaggttgaccaggtgtttgtctttttcctagtgttcccctggccatagtcgccaggttgcagctgccctggtatgtggatcagaagtcctagctcttgccagatggttctgagcccgcctgctccactgggctggagagctccctcccacatttacccagtaggcatacctgccacaccagtgtctggacacaaaatgaatggtgtgtggggctgggaactggggctgccaggtgtccagcaccattttcctttctgtgttttcttctcaggagttaaaatttaattatatcagtaaagagattaattttaatgt

SEQ ID NO: 287 - DNA, 20 bp, synthetic construct
  source 1..20: mol_type = other DNA
attacagtctcaccacgccc

SEQ ID NO: 288 - DNA, 20 bp, synthetic construct
  source 1..20: mol_type = other DNA
gacaagggaagacccaagtg